European Patent Specification EP 3 617 312 B1, published February 18, 2026. Title: Antigen of Allergy or Epitope. Applicant: FUJITA ACADEMY HOYU CO., LTD. The sequence listing filed with the application follows.

SEQUENCE LISTING (984 sequences)

SEQ ID NO: 1 - DNA, 3219 bp, Litopenaeus vannamei
gccactcgtggtgaagaggagctggagaaactggaagctactgctgttaaggctgaagaagagtttgagaaggtacttaaggttcgcgaagaacttgaagcccagaatgcacttcttttggcagagaaaaatgaacttttggcagctgtcgaatcatctaaaggtggcgtatcggaatacttggataagcaagctaaacttctggcccaaaaggccgagctcgaaggacagcttaatgaaactttggaacgcctgagaaaggaggaagacgcacgcaaccagatttctaatggcaagaagaaatgtgaacaagaagtttccaacctgaagaaggagcttgaggaactcgaactctctgtccagcagggtgagcaggataaacaaaccaaggatcagcagcttacaaacctgaacgaggagatctctcatcaagaagaactcatttctaaagttaacaaggaaaagaagcatcttcaggaatgcaaccagaagactgctgaagaccttcagggcattgaagacaaatgcaacaatctcaacaaggttaagacaaagttagaatccggccttgatgaacttgaagatactctggagcgtgagaagaagcttcgtgctgaggttgagaagtcaaagaggaaggttgagggtgaccttaggctaactcaggaagctgtttctgatctggaacgcaatctcaaggaacttgaagttgcggctgagcgcaaggaaaaggaaattgctgccatgactgccaagatcgatgatgaacaggctcttgtgtacagggaccagaggcagattaaggaactgcaagctcgtcttgaggagctcgaggaggaagttgagcatgagcgtcaggcccgtagcaaggccgagaaagccaagaatcttctgtctcgtgaactgtcagaacttggagagcgactggatgaggctggtggcgcaaccgcggctcaaatcgaaatcaataagaagcgtgaaggtgaactggctaaggtccgccgcgacattgaggagtccaaccttcagcatgaggctgctcttgctactctccgcaagaagcacaacgacgccgttgccgagatgtctgagcaagtcgattacctcaataagatgaaggccagaactgaaaaggacaaagaagccatgaagcgagatgccgatgatgctaaggcttccatggatacacttgctcgtgacaagactaccgctgagaagaccaccaagcagcttcagcatcagtacggcgagatctgcgccaagttagacgaggtcaaccgcaccctgagtgacttcgatgccaccaagaagaagcttgcctgcgagaatgcagaccttgtccgccagctggaagaggccgaaaaccaggtcagccagctgtcaagggtcaagctctctctcaccaaccagctcgacgacaccaggaagatgtgcgatgaagagagcaggggccgtgccactctcctgggcaagttccgcaacctggagcacgatattcaagccctccgtgatcaactggatgaggagagcgatgccaagggagatgttctccgaatgctctccaaggctaacgctgaggctctcatgtggcgctccaagtacgagtctgagggtgttgcccgtgcagaggaactcgaggctgctcgtatgaagctcgccgctcgtcttgaggaggccgaaatgcaaatcgagtctctcaatgttaggaacctgcatctcgaaaagactaaaatgcgtgctgctgctgagctggacgatctccatgcttctgctgagcgtgcacaggccctggctagtgctgctgaaaagaagcagaagaacttcgacaagatcatttccgaatggaaactgaaggttgatgacttggccgctgaggtagatgcctcgcagaaggaatgccgcaactactccaccgagcacttccgcctgaaggccgccaatgatgagaacattgaacagcttgacagcattcgccgagagaacaagaacctgagcgacgagatcagggatctgatggaccagcttggtgagggtggccgagcataccatgaagttcagaagaatgccagacgtcttgagctcgagaaggaagaactccaggctgctcttgaggaggccgaggccgctctcgaacaagaggagaacaaggtcctccgcactcaacttgaactcagccagatcagacaagagattgacaggcgtcttcaggagaaggaggaagagttcgacaacacacgcaagtgtcaccagagggccatcgactccatgcaagcttctcttgaggttgaagccaagggtaaggccgaggctcttcgcataaagaagaagctcgagtccgacatcaacgagctcgagatcgcccttgaccacgccaataaggccaactctgaccttcacaaacatctgaggaaggttcacgatgaaatcaaggatgcggaaacccgtgttaaggaagagcaacgccatgcctccgagttccgtgaacagtatggcattgctgaacgccgcttcaacgcccttcacggagagctggaagaatcccgcactctcctggaacagtctgaccgcggccgtcgccacgctgagactgagctcaatgatgcacgcgaacagatcaacaacttcaccaaccagaacactgctctcactgcctcaaagaggaagcttgaaggtgaaatgtcaaccctccaggctgaccttgaggagatgctcaacgaggcaaggaactctgaggagaaggcgaagaaggcaatgcttgacgctgcccgcctggccgacgaactccgctctgagcaggaacacgctcaggcccaagagaagatgcgtaaggccttggaaattaccgtcaaggatctccagacccgtcttgatgagagtgagagtgctgccatgaaggctggcaagaaggccgtcagcaacatggaagctcgcattcgtgatctcgagtctgcgctggatgaagaggtccgtcgtcacgccgattcgcagaagaacctgaggaagtgcgagaggcgcatcaaggagctcgccttccagactgaagaggacaagaagaaccacgacaggatgcaggacctcgtcgataagctccagcagaagatcaagacctacaagcgacagatcgaggaggctgaggagatcgccgccctcaacttggccaagttccgcaagactcagcaggagcttgaagaatctgagggagtaactatcatccactat

SEQ ID NO: 2 - protein, 1073 aa, Litopenaeus vannamei
ATRGEEELEKLEATAVKAEEEFEKVLKVREELEAQNALLLAEKNELLAAVESSKGGVSEYLDKQAKLLAQKAELEGQLNETLERLRKEEDARNQISNGKKKCEQEVSNLKKELEELELSVQQGEQDKQTKDQQLTNLNEEISHQEELISKVNKEKKHLQECNQKTAEDLQGIEDKCNNLNKVKTKLESGLDELEDTLEREKKLRAEVEKSKRKVEGDLRLTQEAVSDLERNLKELEVAAERKEKEIAAMTAKIDDEQALVYRDQRQIKELQARLEELEEEVEHERQARSKAEKAKNLLSRELSELGERLDEAGGATAAQIEINKKREGELAKVRRDIEESNLQHEAALATLRKKHNDAVAEMSEQVDYLNKMKARTEKDKEAMKRDADDAKASMDTLARDKTTAEKTTKQLQHQYGEICAKLDEVNRTLSDFDATKKKLACENADLVRQLEEAENQVSQLSRVKLSLTNQLDDTRKMCDEESRGRATLLGKFRNLEHDIQALRDQLDEESDAKGDVLRMLSKANAEALMWRSKYESEGVARAEELEAARMKLAARLEEAEMQIESLNVRNLHLEKTKMRAAAELDDLHASAERAQALASAAEKKQKNFDKIISEWKLKVDDLAAEVDASQKECRNYSTEHFRLKAANDENIEQLDSIRRENKNLSDEIRDLMDQLGEGGRAYHEVQKNARRLELEKEELQAALEEAEAALEQEENKVLRTQLELSQIRQEIDRRLQEKEEEFDNTRKCHQRAIDSMQASLEVEAKGKAEALRIKKKLESDINELEIALDHANKANSDLHKHLRKVHDEIKDAETRVKEEQRHASEFREQYGIAERRFNALHGELEESRTLLEQSDRGRRHAETELNDAREQINNFTNQNTALTASKRKLEGEMSTLQADLEEMLNEARNSEEKAKKAMLDAARLADELRSEQEHAQAQEKMRKALEITVKDLQTRLDESESAAMKAGKKAVSNMEARIRDLESALDEEVRRHADSQKNLRKCERRIKELAFQTEEDKKNHDRMQDLVDKLQQKIKTYKRQIEEAEEIAALNLAKFRKTQQELEESEGVTIIHY

SEQ ID NO: 3 - protein, 24 aa, Litopenaeus vannamei
ATRGEEELEKLEATAVKAEEEFEK

SEQ ID NO: 4 - protein, 16 aa, Litopenaeus vannamei
VREELEAQNALLLAEK

SEQ ID NO: 5 - protein, 11 aa, Litopenaeus vannamei
NELLAAVESSK

SEQ ID NO: 6 - protein, 9 aa, Litopenaeus vannamei
GGVSEYLDK

SEQ ID NO: 7 - protein, 16 aa, Litopenaeus vannamei
AELEGQLNETLERLRK

SEQ ID NO: 8 - protein, 12 aa, Litopenaeus vannamei
EEDARNQISNGK

SEQ ID NO: 9 - protein, 16 aa, Litopenaeus vannamei
ELEELELSVQQGEQDK

SEQ ID NO: 10 - protein, 20 aa, Litopenaeus vannamei
DQQLTNLNEEISHQEELISK

SEQ ID NO: 11 - protein, 11 aa, Litopenaeus vannamei
TAEDLQGIEDK

SEQ ID NO: 12 - protein, 16 aa, Litopenaeus vannamei
LESGLDELEDTLEREK

SEQ ID NO: 13 - protein, 20 aa, Litopenaeus vannamei
VEGDLRLTQEAVSDLERNLK

SEQ ID NO: 14 - protein, 9 aa, Litopenaeus vannamei
ELEVAAERK

SEQ ID NO: 15 - protein, 8 aa, Litopenaeus vannamei
EIAAMTAK

SEQ ID NO: 16 - protein, 16 aa, Litopenaeus vannamei
IDDEQALVYRDQRQIK

SEQ ID NO: 17 - protein, 22 aa, Litopenaeus vannamei
ELQARLEELEEEVEHERQARSK

SEQ ID NO: 18 - protein, 21 aa, Litopenaeus vannamei
VRRDIEESNLQHEAALATLRK

SEQ ID NO: 19 - protein, 17 aa, Litopenaeus vannamei
HNDAVAEMSEQVDYLNK

SEQ ID NO: 20 - protein, 12 aa, Litopenaeus vannamei
QLQHQYGEICAK

SEQ ID NO: 21 - protein, 15 aa, Litopenaeus vannamei
LDEVNRTLSDFDATK

SEQ ID NO: 22 - protein, 12 aa, Litopenaeus vannamei
LSLTNQLDDTRK

SEQ ID NO: 23 - protein, 15 aa, Litopenaeus vannamei
MCDEESRGRATLLGK

SEQ ID NO: 24 - protein, 22 aa, Litopenaeus vannamei
FRNLEHDIQALRDQLDEESDAK

SEQ ID NO: 25 - protein, 9 aa, Litopenaeus vannamei
GDVLRMLSK

SEQ ID NO: 26 - protein, 18 aa, Litopenaeus vannamei
YESEGVARAEELEAARMK

SEQ ID NO: 27 - protein, 24 aa, Litopenaeus vannamei
LAARLEEAEMQIESLNVRNLHLEK

SEQ ID NO: 28 - protein, 26 aa, Litopenaeus vannamei
MRAAAELDDLHASAERAQALASAAEK

SEQ ID NO: 29 - protein, 11 aa, Litopenaeus vannamei
ANAEALMWRSK

SEQ ID NO: 30 - protein, 13 aa, Litopenaeus vannamei
VDDLAAEVDASQK

SEQ ID NO: 31 - protein, 13 aa, Litopenaeus vannamei
ECRNYSTEHFRLK

SEQ ID NO: 32 - protein, 18 aa, Litopenaeus vannamei
AANDENIEQLDSIRRENK

SEQ ID NO: 33 - protein, 20 aa, Litopenaeus vannamei
EELQAALEEAEAALEQEENK

SEQ ID NO: 34 - protein, 18 aa, Litopenaeus vannamei
CHQRAIDSMQASLEVEAK

SEQ ID NO: 35 - protein, 17 aa, Litopenaeus vannamei
LESDINELEIALDHANK

SEQ ID NO: 36 - protein, 25 aa, Litopenaeus vannamei
LEGEMSTLQADLEEMLNEARNSEEK

SEQ ID NO: 37 - protein, 24 aa, Litopenaeus vannamei
AMLDAARLADELRSEQEHAQAQEK

SEQ ID NO: 38 - protein, 15 aa, Litopenaeus vannamei
DLQTRLDESESAAMK

SEQ ID NO: 39 - protein, 28 aa, Litopenaeus vannamei
AVSNMEARIRDLESALDEEVRRHADSQK

SEQ ID NO: 40 - protein, 10 aa, Litopenaeus vannamei
ELAFQTEEDK

SEQ ID NO: 41 - protein, 11 aa, Litopenaeus vannamei
NHDRMQDLVDK

SEQ ID NO: 42 - protein, 16 aa, Litopenaeus vannamei
RQIEEAEEIAALNLAK

SEQ ID NO: 43 - protein, 16 aa, Litopenaeus vannamei
TQQELEESEGVTIIHY

SEQ ID NO: 44 - DNA, 3219 bp, Penaeus monodon
gccactcgtggtgaagaggagctggagaaactggaagctactgctgttaaggctgaagaagagtttgggaaggtagttaaggttcgcgaagaacttgaagctcagaatgcacttcttatgcaagaaagaaatgaacttttggcagctgtcgactctactaaaggtggcatgtcggaatatttggacaagcaagctaaacttctggcccaaaaggctgagctcgagggacagcttaatgacactttggaacgcctgagaaaggaggaagacgcgcgcaaccagattgctaatggcaagaagaaatgtgaacaagaagttactaacctgaagaaggagcttgaggaactcgagctttctgtccagaagggtgagcaggataaacaaaccaaggatcaacagcttacaaacttaaacgaggagatctctcaccaggaagagctcattaccaaagttaacaaggaaaagaaacaccttcaggaatgcaaccagaagacagccgaagaccttcagggcgttgaagataaatgcaacaatctgaataaagttaagacaaagttagaatccagccttgatgaacttgaagatactttggagcgcgagaagaagcttcgtgctgaggttgagaagtcaaagaggaaggttgaaggtgaccttaggctgactcaggaagctgtttctgatctggaacgcaatctcaaggaacttgaagttgcagctgagcgcaaggaaaaggaaatttctgccatcactgccaagattgaggatgaacaggctcttgtgtacagggaccagaggcaggttaaggaactgcaagctcgtcttgaggagctcgaggaggacgttgagcatgagcgtcaggcccgtggcaaggccgagaaagccaaaaatgttttgtctcgcgagctgtcagaacttggagagcgactggatgaagctggcggcgctaccgcggctcagatcgaaatcaataagaagcgtgaaggtgaactgggcaaggtccgccgcgacattgaggagtccaaccttcagcatgaggctgctcttgccactctccgcaagaagcacaacgacgtcgttgcagagatgtctgagcaagttgactacctcaataagatgaaggccaggactgagaaggacaaagaagccatgaagcgagatgctgatgatgctaaggcttccatggattcacttgctcgtgacaagacaaccgctgagaagaccaccaagcagcttcagcaccagtacggcgagctctgcgccaagttagatgaggtcaatcgcactctgagtgactttgacgccaccaagaagaagcttgcctgcgagaacactgaccttgttcgccagctggaagaggccgaaaaccaggtcagccagctgtcaagggtcaagctttctctcaccaaccagctcgacgacaccaggaagatgtgcgatgaagagagcagaggtcgtgccactctcctgggtaagttccgcaacctggagcacgatattcaagctctccgtgatcagctggatgaggagagcgatgccaagggagatgttctccgaatgctgtctgctgctaacgctgaagctctcatgtggcgctccaagtatgagtctgagggtgttgcccgtgcagaggaactcgaggctgctcgaatgaagctcgccgctcgccttgaggaggccgaaatgcaaatcgagtctcttaatgtgaggaacctgcatctcgagaagactaaaatgcgtgctgctgctgagctggacgacctccatgcttccgctgagcgtgcacaggccctcgctagtgctgctgaaaagaagcagaagaacttcgacaagatcatttccgaatggaaactgaaggttgatgacttggccgctgaggtagatgcctctcagaaggaatgccgcaactactccaccgagcatttccgcctgaaggccgccaatgatgagaacatcgaacagcttgacagcattcgccgagagaacaagaacctgagcgacgagatcagggatctgatggaccagcttggggagggtggccgtgcataccatgaagttcagaagaatgccagacgtcttgagctcgagaaggaagaactccaggctgctcttgaggaggctgaggccgctctcgagcaagaagagaacaaggtcctccgcactcaacttgaactcagccaggtcaggcaagagattgacaggcgtgttcaggagaaggaggaagaattcgacaacacacgcaagtgtcaccagagagctatcgactccatgcaagcttctcttgaggttgaagccaagggtaaggccgaggctcttcgcatgaagaagaagcttgagtccgacatcaacgagctcgagattgccctggaccacgccaataaggcaaactctgaccttcacaaacaccttaggagggtccatgatgaaatcaaggatgcggaaacccgtgttaaggaggagcagcgtgttgcctccgagttccgtgaacagtatggcattgctgaacgccgcttcaacgcccttcacggagagcttgaagaatcccgcactcttctggaacagtctgaccgcggccgtcgccacgctgagactgagctcaatgatgcacgtgaacagatcaacaacttcactaaccagaatactgctctcactgcctcaaagaggaagcttgaaggtgaaatgtcaacactccaggctgacctcgaagagatgctcaacgaggcaaagaactctgaggagaaggcgaagaaggcaatgcttgacgctgcacgtctggccgacgaactccgctctgagcaggaacacgctcagtcccaagagaagatgcgtaaggccttggaaattactgctaaggatctccagacccgtctcgaggaaagtgagagtgctgccatgaaagctggtaagaaggcagtcagtaacatggaagctcgcattcgtgatctcgagtctgcgctggatgatgagactcgccgtcacgccgattcccagaagaacctgaggaagtgcgagaggcgcatcaaggagctcgccttccagactgaagaggacaagaagaaccacgacaggatgcaggacctcgtcgataagctccagcagaagatcaagacctacaagcgccagatcgaggaggctgaggagatcgccgccctcaacctggccaagttccgcaagactcagcaggagctcgaagaatctgagacagtaactgtcgtccactat

SEQ ID NO: 45 - protein, 1073 aa, Penaeus monodon
ATRGEEELEKLEATAVKAEEEFGKVVKVREELEAQNALLMQERNELLAAVDSTKGGMSEYLDKQAKLLAQKAELEGQLNDTLERLRKEEDARNQIANGKKKCEQEVTNLKKELEELELSVQKGEQDKQTKDQQLTNLNEEISHQEELITKVNKEKKHLQECNQKTAEDLQGVEDKCNNLNKVKTKLESSLDELEDTLEREKKLRAEVEKSKRKVEGDLRLTQEAVSDLERNLKELEVAAERKEKEISAITAKIEDEQALVYRDQRQVKELQARLEELEEDVEHERQARGKAEKAKNVLSRELSELGERLDEAGGATAAQIEINKKREGELGKVRRDIEESNLQHEAALATLRKKHNDVVAEMSEQVDYLNKMKARTEKDKEAMKRDADDAKASMDSLARDKTTAEKTTKQLQHQYGELCAKLDEVNRTLSDFDATKKKLACENTDLVRQLEEAENQVSQLSRVKLSLTNQLDDTRKMCDEESRGRATLLGKFRNLEHDIQALRDQLDEESDAKGDVLRMLSAANAEALMWRSKYESEGVARAEELEAARMKLAARLEEAEMQIESLNVRNLHLEKTKMRAAAELDDLHASAERAQALASAAEKKQKNFDKIISEWKLKVDDLAAEVDASQKECRNYSTEHFRLKAANDENIEQLDSIRRENKNLSDEIRDLMDQLGEGGRAYHEVQKNARRLELEKEELQAALEEAEAALEQEENKVLRTQLELSQVRQEIDRRVQEKEEEFDNTRKCHQRAIDSMQASLEVEAKGKAEALRMKKKLESDINELEIALDHANKANSDLHKHLRRVHDEIKDAETRVKEEQRVASEFREQYGIAERRFNALHGELEESRTLLEQSDRGRRHAETELNDAREQINNFTNQNTALTASKRKLEGEMSTLQADLEEMLNEAKNSEEKAKKAMLDAARLADELRSEQEHAQSQEKMRKALEITAKDLQTRLEESESAAMKAGKKAVSNMEARIRDLESALDDETRRHADSQKNLRKCERRIKELAFQTEEDKKNHDRMQDLVDKLQQKIKTYKRQIEEAEEIAALNLAKFRKTQQELEESETVTVVHY

SEQ ID NO: 46 - protein, 27 aa, Penaeus monodon
VREELEAQNALLMQERNELLAAVDSTK

SEQ ID NO: 47 - protein, 9 aa, Penaeus monodon
GGMSEYLDK

SEQ ID NO: 48 - protein, 16 aa, Penaeus monodon
AELEGQLNDTLERLRK

SEQ ID NO: 49 - protein, 12 aa, Penaeus monodon
EEDARNQIANGK

SEQ ID NO: 50 - protein, 9 aa, Penaeus monodon
CEQEVTNLK

SEQ ID NO: 51 - protein, 11 aa, Penaeus monodon
ELEELELSVQK

SEQ ID NO: 52 - protein, 20 aa, Penaeus monodon
DQQLTNLNEEISHQEELITK

SEQ ID NO: 53 - protein, 11 aa, Penaeus monodon
TAEDLQGVEDK

SEQ ID NO: 54 - protein, 16 aa, Penaeus monodon
LESSLDELEDTLEREK

SEQ ID NO: 55 - protein, 20 aa, Penaeus monodon
VEGDLRLTQEAVSDLERNLK

SEQ ID NO: 56 - protein, 9 aa, Penaeus monodon
ELEVAAERK

SEQ ID NO: 57 - protein, 8 aa, Penaeus monodon
EISAITAK

SEQ ID NO: 58 - protein, 16 aa, Penaeus monodon
IEDEQALVYRDQRQVK

SEQ ID NO: 59 - protein, 22 aa, Penaeus monodon
ELQARLEELEEDVEHERQARGK

SEQ ID NO: 60 - protein, 21 aa, Penaeus monodon
VRRDIEESNLQHEAALATLRK

SEQ ID NO: 61 - protein, 17 aa, Penaeus monodon
HNDVVAEMSEQVDYLNK

SEQ ID NO: 62 - protein, 12 aa, Penaeus monodon
QLQHQYGELCAK

SEQ ID NO: 63 - protein, 15 aa, Penaeus monodon
LDEVNRTLSDFDATK

SEQ ID NO: 64 - protein, 12 aa, Penaeus monodon
LSLTNQLDDTRK

SEQ ID NO: 65 - protein, 15 aa, Penaeus monodon
MCDEESRGRATLLGK

SEQ ID NO: 66 - protein, 22 aa, Penaeus monodon
FRNLEHDIQALRDQLDEESDAK

SEQ ID NO: 67 - protein, 9 aa, Penaeus monodon
GDVLRMLSA

SEQ ID NO: 68 - protein, 11 aa, Penaeus monodon
ANAEALMWRSK

SEQ ID NO: 69 - protein, 18 aa, Penaeus monodon
YESEGVARAEELEAARMK

SEQ ID NO: 70 - protein, 24 aa, Penaeus monodon
LAARLEEAEMQIESLNVRNLHLEK

SEQ ID NO: 71 - protein, 26 aa, Penaeus monodon
MRAAAELDDLHASAERAQALASAAEK

SEQ ID NO: 72 - protein, 15 aa, Penaeus monodon
LKVDDLAAEVDASQK

SEQ ID NO: 73 - protein, 13 aa, Penaeus monodon
ECRNYSTEHFRLK

SEQ ID NO: 74 - protein, 18 aa, Penaeus monodon
AANDENIEQLDSIRRENK

SEQ ID NO: 75 - protein, 20 aa, Penaeus monodon
EELQAALEEAEAALEQEENK

SEQ ID NO: 76 - protein, 22 aa, Penaeus monodon
VLRTQLELSQVRQEIDRRVQEK

SEQ ID NO: 77 - protein, 18 aa, Penaeus monodon
CHQRAIDSMQASLEVEAK

SEQ ID NO: 78 - protein, 17 aa, Penaeus monodon
LESDINELEIALDHANK

SEQ ID NO: 79 - protein, 20 aa, Penaeus monodon
LEGEMSTLQADLEEMLNEAK

SEQ ID NO: 80 - protein, 24 aa, Penaeus monodon
AMLDAARLADELRSEQEHAQSQEK

SEQ ID NO: 81 - protein, 15 aa, Penaeus monodon
DLQTRLEESESAAMK

SEQ ID NO: 82 - protein, 10 aa, Penaeus monodon
ELAFQTEEDK

SEQ ID NO: 83 - protein, 11 aa, Penaeus monodon
NHDRMQDLVDK

SEQ ID NO: 84 - protein, 16 aa, Penaeus monodon
RQIEEAEEIAALNLAK

SEQ ID NO: 85 - protein, 16 aa, Penaeus monodon
TQQELEESETVTVVHY

SEQ ID NO: 86 - DNA, 3216 bp, Marsupenaeus japonicus
gcctgtcgcgctgaagaggagttggagaaactggaagctactgctgcaaaggctgaggaacagtatgaaaaggaagtcaaagttcgcgaagaacttgaagcccaaaatgcagctctactggcagaaaagaatgagcttttggcagctgtcgagtcttccaaaggtggtatgtcggaatacttagataagcaagctaaacttctggctcaaaagggtgaacttgaagcgcagctcaacgaaactttggaacgccttagaaaggaggaagacgcacgcaatcagattgccaacggcaagaaaaagtgtgaacaagaagtttcgaacctgaagaaggagcttgaagaactcgaactttctgtccaaaagggtgagcaagataaacaaactaaggatcaacagcttactagcttgaacgaggagatttcccatcaggaagaactcatcaccaaggttaacaaggaaaagaagcaccttcaggaatgcaatcaaaagactgccgaagaccttcagagcattgaagataaatgcaacaatctcaataaagttaagacgaagttagagtccacccttgacgaacttgaagatacactggagcgtgagaagaagcttcgtgctgaagttgaaaagtcgaagaggaaggttgagggtgaccttcggctgactcaggaagctgtttctgatctggaacgtaatctcaaggaacttgaagtggcagctgagcgcaaggaaaaggaaattggtgctataactgccaagattgaggatgaacaggctcttgtatacagagaccagagacaggttaaggaactgcaggctcgtcttgaggagctcgaagaggaagttgaacatgaacgtcaggcccgaggtaaggccgagaaagctaagaatctgctatctcgcgagttgtcagaacttggtgagcgactggatgaggctggtggtgctactgcagcccagattgaaatcaataagaagcgtgaaagtgaactggctaaggtccgccgcgatattgaagagtccaaccttcagcatgaggcagctcttgctactctccgcaagaagcacaacgatgctgtagccgagatgtctgagcaagtagactaccttaataagatgaaggccagggctgaaaaggacaaggaagccatgaagcgtgatgctgatgatgctaaggcttccatggattcacttgctcgtgataagactactgctgagaagaccaccaagcagctgcagcatcagtatggagaaatctgcgccaagttagatgaggtcaaccgtaccctaagtgactttgatgccaccaagaaaaagcttgcctgcgagaacagtgaccttgttcgccagctggaagaagctgaaaaccaggtttcccagctctcgagggtcaagctttctctcaccaaccagcttgacgacaccagaaagatgtgtgatgaagaaagcagggctcgtgccactctcctcggtaagttccgcaacttggagcacgatattcaagctctccgtgatcagctggatgaggagagtgatgctaagggtgatgttctccgaatgctctcaaaggctaacgctgaagctctcatgtggcgctccaagtacgagtctgagggtgttgcccgtgccgaggaacttgaggctgctcgcatgaagctcgccgctcgtctcgaggaagccgaaatgcaaatcgagtctctcaatgttaggaacttgcatctcgaaaaaacaaagatgcgtgcggctgttgagctggacgatctccatgcttctgctgagcgtgcacaggccctggccaatgctgctgaaaagaagcagaagaacttcgacaagatcatttctgaatggaagctgaaggttgatgaccttgctgctgaagtagatgcctcacagaaagagtgccgcaactactccactgaacacttccgcctcaaggctgccaatgatgagaatatcgaacagctcgacagcattcgccgcgagaacaagaacctcagtgacgagatcagagacctgatggatcagattggtgagggtggccgagcattccatgagactcagaagaatgccagacgtcttgagctcgagaaggtagaactccaggctgctcttgaagaagctgaggccgctcttgaacaagaagaaaacaaggtgctccgcacccagcttgaactcagccaggttagacgggagatcgacaggcgtgttcaagagaaggaagaagaattcgacaatactcgcaagtgtcaccaaagagccatcgattccctacaagcttctctagaggttgaaaccaagggtaaggctgaagctcttcgcttgaaaaagaagctcgagtccgatatcaacgagctcgagattgcccttgaccacgctaataaggccaattcagaccttcacaaacatcttaggaaggttcatgatgaaatcaaggacgcggaaactcgtgttaaggaggaacagcgtcttgcatccgagtatcgtgaacagtatggcattgctgaacgccgcttcaacgcccttcatggtgagctggaggaatctcgtactcttcttgaacagtctgaccgtggccgccgtcatgctgagactgagctcaacgatgcacgtgaacagatcaacaacttcaccaaccagaatgctggtctcaccgcctcaaagaggaaactcgagggtgaaatgcatactctccaggctgacctcgaagagatgctcggcgaggcaaagaattctgaggagaaggcaaagaaggcaatgcttgacgctgcccgattggccgatgaacttcgctctgagcaggaacacgctcagacccaggagaaaatgcgtagggcactggaagttactgccaaggatctccagacccgtcttgaggagagcgagagtgctgctatgaaggctggcaagaaggcagttggcaacatggaagctcgcattcgtgaactcgagtctgcactggatgatgagactcgccgtcacgctgattctcagaagaacctgaggaagtgcgagaggcgcatcaaggagctcgcattccagactgaagaagacaagaagaaccacgacaggatgcaggacctcgtcgataagctccagcagaagatcaagacctacaagcgccagatcgaggaggctgaggagatcgccgccctcaacctggccaagttccgcaagactcagcaggagctcgaggaatctgaggtgattgtttctcacttc

SEQ ID NO: 87 - protein, 1072 aa, Marsupenaeus japonicus
ACRAEEELEKLEATAAKAEEQYEKEVKVREELEAQNAALLAEKNELLAAVESSKGGMSEYLDKQAKLLAQKGELEAQLNETLERLRKEEDARNQIANGKKKCEQEVSNLKKELEELELSVQKGEQDKQTKDQQLTSLNEEISHQEELITKVNKEKKHLQECNQKTAEDLQSIEDKCNNLNKVKTKLESTLDELEDTLEREKKLRAEVEKSKRKVEGDLRLTQEAVSDLERNLKELEVAAERKEKEIGAITAKIEDEQALVYRDQRQVKELQARLEELEEEVEHERQARGKAEKAKNLLSRELSELGERLDEAGGATAAQIEINKKRESELAKVRRDIEESNLQHEAALATLRKKHNDAVAEMSEQVDYLNKMKARAEKDKEAMKRDADDAKASMDSLARDKTTAEKTTKQLQHQYGEICAKLDEVNRTLSDFDATKKKLACENSDLVRQLEEAENQVSQLSRVKLSLTNQLDDTRKMCDEESRARATLLGKFRNLEHDIQALRDQLDEESDAKGDVLRMLSKANAEALMWRSKYESEGVARAEELEAARMKLAARLEEAEMQIESLNVRNLHLEKTKMRAAVELDDLHASAERAQALANAAEKKQKNFDKIISEWKLKVDDLAAEVDASQKECRNYSTEHFRLKAANDENIEQLDSIRRENKNLSDEIRDLMDQIGEGGRAFHETQKNARRLELEKVELQAALEEAEAALEQEENKVLRTQLELSQVRREIDRRVQEKEEEFDNTRKCHQRAIDSLQASLEVETKGKAEALRLKKKLESDINELEIALDHANKANSDLHKHLRKVHDEIKDAETRVKEEQRLASEYREQYGIAERRFNALHGELEESRTLLEQSDRGRRHAETELNDAREQINNFTNQNAGLTASKRKLEGEMHTLQADLEEMLGEAKNSEEKAKKAMLDAARLADELRSEQEHAQTQEKMRRALEVTAKDLQTRLEESESAAMKAGKKAVGNMEARIRELESALDDETRRHADSQKNLRKCERRIKELAFQTEEDKKNHDRMQDLVDKLQQKIKTYKRQIEEAEEIAALNLAKFRKTQQELEESEVIVSHF

SEQ ID NO: 88 - protein, 10 aa, Marsupenaeus japonicus
ACRAEEELEK

SEQ ID NO: 89 - protein, 16 aa, Marsupenaeus japonicus
VREELEAQNAALLAEK

SEQ ID NO: 90 - protein, 11 aa, Marsupenaeus japonicus
NELLAAVESSK

SEQ ID NO: 91 - protein, 9 aa, Marsupenaeus japonicus
GGMSEYLDK

SEQ ID NO: 92 - protein, 11 aa, Marsupenaeus japonicus
ELEELELSVQK

SEQ ID NO: 93 - protein, 20 aa, Marsupenaeus japonicus
DQQLTSLNEEISHQEELITK

SEQ ID NO: 94 - protein, 11 aa, Marsupenaeus japonicus
TAEDLQSIEDK

SEQ ID NO: 95 - protein, 16 aa, Marsupenaeus japonicus
IEDEQALVYRDQRQVK

SEQ ID NO: 96 - protein, 22 aa, Marsupenaeus japonicus
ELQARLEELEEEVEHERQARGK

SEQ ID NO: 97 - protein, 21 aa, Marsupenaeus japonicus
VRRDIEESNLQHEAALATLRK

SEQ ID NO: 98 - protein, 17 aa, Marsupenaeus japonicus
HNDAVAEMSEQVDYLNK

SEQ ID NO: 99 - protein, 12 aa, Marsupenaeus japonicus
QLQHQYGEICAK

SEQ ID NO: 100 - protein, 15 aa, Marsupenaeus japonicus
LDEVNRTLSDFDATK

SEQ ID NO: 101 - protein, 12 aa, Marsupenaeus japonicus
LSLTNQLDDTRK

SEQ ID NO: 102 - protein, 22 aa, Marsupenaeus japonicus
FRNLEHDIQALRDQLDEESDAK

SEQ ID NO: 103 - protein, 18 aa, Marsupenaeus japonicus
YESEGVARAEELEAARMK

SEQ ID NO: 104 - protein, 24 aa, Marsupenaeus japonicus
LAARLEEAEMQIESLNVRNLHLEK

SEQ ID NO: 105 - protein, 14 aa, Marsupenaeus japonicus
SAERAQALANAAEK

SEQ ID NO: 106 - protein, 13 aa, Marsupenaeus japonicus
VDDLAAEVDASQK

SEQ ID NO: 107 - protein, 18 aa, Marsupenaeus japonicus
AANDENIEQLDSIRRENK

SEQ ID NO: 108 - protein, 15 aa, Marsupenaeus japonicus
ALEEAEAALEQEENK

SEQ ID NO: 109 - protein, 17 aa, Marsupenaeus japonicus
LESDINELEIALDHANK

SEQ ID NO: 110 - protein, 20 aa, Marsupenaeus japonicus
LEGEMHTLQADLEEMLGEAK

SEQ ID NO: 111 - protein, 24 aa, Marsupenaeus japonicus
AMLDAARLADELRSEQEHAQTQEK

SEQ ID NO: 112 - protein, 15 aa, Marsupenaeus japonicus
DLQTRLEESESAAMK

SEQ ID NO: 113 - protein, 10 aa, Marsupenaeus japonicus
ELAFQTEEDK

SEQ ID NO: 114 - protein, 16 aa, Marsupenaeus japonicus
RQIEEAEEIAALNLAK

SEQ ID NO: 115 - protein, 15 aa, Marsupenaeus japonicus
TQQELEESEVIVSHF

SEQ ID NO: 116 - DNA, 2424 bp, Litopenaeus vannamei
agcacgggtccagaccccgaccccactgaatacctcttcatctctcgggagcagaagatgaaggatcagacgaaaccctacgatcctaagaagtcttattggtgtcctgaccccaatgagggcttcgtcgagtgtgagtttcaggctcctaagggtgataaacttgtcacagtaaagcttcccagcggcgagacgaaggacttcaagaaggagcaggtcggacaggtcaaccctcccaagtacgagaagtgtgaggatgtgtccaacctgaccttcctcaacgatccctccgtcttctacgtcctcaagtcccgttaccaggccaagcttatctacacctactctggtctcttctgtatcgccgtcaacccctacaagcgttaccccatctacaccaaccgtgccgtcaagatctatatcggcaagaggcgtaatgaggtgccccctcatctcttcgccatttgcgacggtgcctaccagaacatgaatcaagaacgccagaaccagtctatgcttattaccggcgaatctggcgccggcaagactgagaacacaaagaaggtgttgtcttacttcgccaacgtcggtgcctctgagaagaaagagggcgagagcaaacagaatcttgaggaccagattatccaaaccaaccccatccttgaagcttacggcaatgccaagaccacccgtaacgacaactcctctcgtttcggtaagttcatccgcgtccacttcgctcccaacggcaagctctctggcgctgatatcgaggtctacctgctggagaaggctcgtgtcatctcccagtcccccgccgagcgaggctaccatatcttctaccagctcatgtgcgaccagattgattatatgaagaaaatttgctgtttgtctgacgacatctacgactaccactacgaggctcagggtaaggttaccgtcccatccatcgacgacaaggaagacatgcaatttactcacgacgctttcgacatcctgaacttctcacacgaggaaagagacgattgctataaggttacagcttctgtcatgcaccatggtaacatgaagttcaagcagaggggtcgcgaagagcaggctgaggccgatggcactgaggccggagaaattgttgctaaactgctcggtgttgacgccgaggagctctacaggaacttctgcaagcccaagatcaaggtcggtgccgagttcgtcaccaagggtatgaatgtcgaccaagtcaactacaacgttggtgccatggccaagggtctcttctctcgtgtgttctcatggctcgtcaggaagtgtaacatgacactcgagactggccagactcgcgccatgttcatcggtgtgctcgatattgccggctttgagatcttcgacttcaacggtttcgagcagatctgtatcaacttctgtaacgagaagctgcagcagttcttcaaccaccacatgttcgtactggaacaagaagaatacgcaaaggaaggcattgtgtggcagttcgtcgacttcggtatggatctgcaggcttgcattgaactcttcgagaagaaaatgggtctcctctccatccttgaggaagagtccatgttccccaaggccactgacaagaccttcgaggagaagctgaacaacaaccatctcggaaagtctcgttgcttcatcaagcccaagcctccaaaggccggtcaacctgagaaccactttgccattgttcactacgctggcactgtgtcctacaacctgactggctggcttgagaagaacaaggatcctctcaacgacaccgtcgtcgaccagctcaagaaggcctccaacgccctcacagtcgagatcttcgctgaccatcctggtcaatccggtgatggaggtggcaaaggaaagggaggcaagcagcagactggtttcaaaaccgtgtcttctgggtacaaggatcagcttgccaacctcatgaagactctcaacgctactcatcctcacttcatccgttgcattgtgcccaacgagttcaagaagcccggcgaagtagacgctggcctcatcatgcatcagctgacctgtaacggtgtacttgagggcatccgtatttgccagaagggcttccccaacaggatgccttatcctgacttcaaacagcgatacaacatccttgccgctaaggagatgcttgaagcgaaggacgacaagaaggcagcaacagcttgcttcgagagggccggcctcgaccctgagttgtaccgtaccggcaatactaaggtattcttccgtgccggtgtcttgggtacccttgaagagattcgtgatgaccgtattatgaagctggtatcctggcttcaagcatggattcgtggctgggccagccgcaaatactattccaagatgcagaagcaacgcactgctctcatcgtcatgcaacgt

SEQ ID NO: 117 - protein, 808 aa, Litopenaeus vannamei
STGPDPDPTEYLFISREQKMKDQTKPYDPKKSYWCPDPNEGFVECEFQAPKGDKLVTVKLPSGETKDFKKEQVGQVNPPKYEKCEDVSNLTFLNDPSVFYVLKSRYQAKLIYTYSGLFCIAVNPYKRYPIYTNRAVKIYIGKRRNEVPPHLFAICDGAYQNMNQERQNQSMLITGESGAGKTENTKKVLSYFANVGASEKKEGESKQNLEDQIIQTNPILEAYGNAKTTRNDNSSRFGKFIRVHFAPNGKLSGADIEVYLLEKARVISQSPAERGYHIFYQLMCDQIDYMKKICCLSDDIYDYHYEAQGKVTVPSIDDKEDMQFTHDAFDILNFSHEERDDCYKVTASVMHHGNMKFKQRGREEQAEADGTEAGEIVAKLLGVDAEELYRNFCKPKIKVGAEFVTKGMNVDQVNYNVGAMAKGLFSRVFSWLVRKCNMTLETGQTRAMFIGVLDIAGFEIFDFNGFEQICINFCNEKLQQFFNHHMFVLEQEEYAKEGIVWQFVDFGMDLQACIELFEKKMGLLSILEEESMFPKATDKTFEEKLNNNHLGKSRCFIKPKPPKAGQPENHFAIVHYAGTVSYNLTGWLEKNKDPLNDTVVDQLKKASNALTVEIFADHPGQSGDGGGKGKGGKQQTGFKTVSSGYKDQLANLMKTLNATHPHFIRCIVPNEFKKPGEVDAGLIMHQLTCNGVLEGIRICQKGFPNRMPYPDFKQRYNILAAKEMLEAKDDKKAATACFERAGLDPELYRTGNTKVFFRAGVLGTLEEIRDDRIMKLVSWLQAWIRGWASRKYYSKMQKQRTALIVMQR

SEQ ID NO: 118 - protein, 19 aa, Litopenaeus vannamei
STGPDPDPTEYLFISREQK

SEQ ID NO: 119 - protein, 12 aa, Litopenaeus vannamei
LVTVKLPSGETK

SEQ ID NO: 120 - protein, 10 aa, Litopenaeus vannamei
EQVGQVNPPK

SEQ ID NO: 121 - protein, 11 aa, Litopenaeus vannamei
MLITGESGAGK

SEQ ID NO: 122 - protein, 13 aa, Litopenaeus vannamei
VLSYFANVGASEK

SEQ ID NO: 123 - protein, 21 aa, Litopenaeus vannamei
QNLEDQIIQTNPILEAYGNAK

SEQ ID NO: 124 - protein, 11 aa, Litopenaeus vannamei
FIRVHFAPNGK

SEQ ID NO: 125 - protein, 13 aa, Litopenaeus vannamei
LSGADIEVYLLEK

SEQ ID NO: 126 - protein, 18 aa, Litopenaeus vannamei
ICCLSDDIYDYHYEAQGK

SEQ ID NO: 127 - protein, 9 aa, Litopenaeus vannamei
VTVPSIDDK

SEQ ID NO: 128 - protein, 16 aa, Litopenaeus vannamei
GMNVDQVNYNVGAMAK

SEQ ID NO: 129 - protein, 18 aa, Litopenaeus vannamei
QQFFNHHMFVLEQEEYAK

SEQ ID NO: 130 - protein, 15 aa, Litopenaeus vannamei
MGLLSILEEESMFPK

SEQ ID NO: 131 - protein, 12 aa, Litopenaeus vannamei
DPLNDTVVDQLK

SEQ ID NO: 132 - protein, 23 aa, Litopenaeus vannamei
ASNALTVEIFADHPGQSGDGGGK

SEQ ID NO: 133 - protein, 9 aa, Litopenaeus vannamei
GGKQQTGFK

SEQ ID NO: 134 - protein, 7 aa, Litopenaeus vannamei
TVSSGYK

SEQ ID NO: 135 - protein, 8 aa, Litopenaeus vannamei
DQLANLMK

SEQ ID NO: 136 - protein, 12 aa, Litopenaeus vannamei
GFPNRMPYPDFK

SEQ ID NO: 137 - protein, 9 aa, Litopenaeus vannamei
QRYNILAAK

SEQ ID NO: 138 - protein, 22 aa, Litopenaeus vannamei
AATACFERAGLDPELYRTGNTK

SEQ ID NO: 139 - protein, 10 aa, Litopenaeus vannamei
QRTALIVMQR

SEQ ID NO: 140 - DNA, 2427 bp, Penaeus monodon
agcacgggtcccgaccccgaccccactgaatacctcttcatctctcgggagcagaggatgaaggatcagacgaaaccctacgatcctaagaagtccttctggtgtcctgaccccaatgagggcttcgtcgagtgtgagcttcagggtgctaagggtgacaaacatgtcacagttaagcttcccagcggcgagacgaaggacttcaagaaggagcaggtcggacaggtcaaccctcccaagtacgagaagtgtgaggatgtgtccaacttgaccttcctgaacgatccctccgtcttctacgtcctcaagtcccgttaccaggccaagcttatctacacctactctggtctcttctgtatcgccgtcaatccctacaagcgttaccccatctacaccaaccgcgccgtcaagatttacattggcaagaggcgtaatgaggtgccccctcatctcttcgccatctgcgacggtgcctaccagaacatgaatcaagaacgtcagaaccagtctatgcttatcaccggtgaatctggtgccggcaagactgagaacacaaagaaggtgttgtcttacttcgccaacgtcggtgccagcgagaagaaagagggcgagagcaaacagaatcttgaggaccagattatccaaaccaaccccatccttgaagcttacggcaatgccaagaccacccgtaacgacaactcttctcgtttcggtaagtttatccgcgtccacttcgctccaaacggcaagctttccggcgctgacattgaggtctacctgctggagaaggctcgtgtcatctcccagtcccccgccgagcgaggctaccatatcttctaccagctcatgtgcgaccagatcgactatgtcaagaagatgtgcttattgtctgacgacatctacgactactactacgaggcgcagggtaaagttaccgtcccatccatcgacgacaaggaggacatgcagttcactcatgatgctttcgacgtcttgaacttctctcatgaggaaagagacgattgctacaaggtcacagcttctgtcatgcaccatggcaacatgaaattcaagcagaggggtcgtgaggagcaggctgaggccgatggcactgaggccggagaaattgttgctaaactgctcggtgttgacgctgaggagctctacaggaatttctgcaagcccaagatcaaggtcggtgccgagttcgtcaccaagggtatgaatgtcgaccaagtaaactacaacatcggtgccatggccaagggtctcttttcacgtgtattctcatggctcgtcaagaagtgtaacatgacacttgagactggccagactcgtgctatgttcatcggcgtactggatattgccggttttgagatcttcgacttcaacggtttcgagcagatctgtatcaacttctgtaacgagaagctgcagcagttcttcaaccatcacatgttcgtgctggaacaagaagaatatgcaaaagagggtattgtctggcagttcgtcgacttcggcatggatctgcaggcctgcattgaactcttcgagaagaaaatgggtctcctctccatccttgaggaagagtccatgttccccaaggctactgacaagaccttcgaggagaagctcaacaacaaccatctcggaaagtctcgctgcttcatcaagcccaagcctccaaaggccggccagcctgagaaccactttgccatcgttcactacgctggcactgtgtcctacaacctgactggctggctcgagaagaacaaggatcctctcaacgacaccgtcgtcgaccagctcaagaaggcctccaacgccctcacagtcgagatctttgctgaccatcccggccaatccggtgacggtggtggcaaaggaaagggaggcaagcagcagaccggcttcaaaactgtgtcttctgggtacaaggatcagcttgccaacctgatgaagactctcaacgctactcatcctcatttcatccgttgcattgtgcctaacgagttcaagaagccgggcgaagtagactctggcctcatcatgcatcagctgacttgtaatggtgtacttgagggccatccgttatttgccagaagggcttccccaacagggatgccttataaagacttcaagttgcgatacaacatcctagccgctaaggagatgcttgaagcgaaggacgacaagaaggcagcaacagcttgcttcgagagggccggcctcaaccctgaattgtatcgtacaggcaataccaaggtattcttccgtgctggtgtcctgggtacccttgaagaggtccgtgatgaccgtattatgaaactggtatcctggcttcaagcatgggttcgaggctgggccagccgcaaatactattccaagatgcaaaagcagcgcactgctctcatcgttatgcaacgc

SEQ ID NO: 141 - protein, 809 aa, Penaeus monodon
STGPDPDPTEYLFISREQRMKDQTKPYDPKKSFWCPDPNEGFVECELQGAKGDKHVTVKLPSGETKDFKKEQVGQVNPPKYEKCEDVSNLTFLNDPSVFYVLKSRYQAKLIYTYSGLFCIAVNPYKRYPIYTNRAVKIYIGKRRNEVPPHLFAICDGAYQNMNQERQNQSMLITGESGAGKTENTKKVLSYFANVGASEKKEGESKQNLEDQIIQTNPILEAYGNAKTTRNDNSSRFGKFIRVHFAPNGKLSGADIEVYLLEKARVISQSPAERGYHIFYQLMCDQIDYVKKMCLLSDDIYDYYYEAQGKVTVPSIDDKEDMQFTHDAFDVLNFSHEERDDCYKVTASVMHHGNMKFKQRGREEQAEADGTEAGEIVAKLLGVDAEELYRNFCKPKIKVGAEFVTKGMNVDQVNYNIGAMAKGLFSRVFSWLVKKCNMTLETGQTRAMFIGVLDIAGFEIFDFNGFEQICINFCNEKLQQFFNHHMFVLEQEEYAKEGIVWQFVDFGMDLQACIELFEKKMGLLSILEEESMFPKATDKTFEEKLNNNHLGKSRCFIKPKPPKAGQPENHFAIVHYAGTVSYNLTGWLEKNKDPLNDTVVDQLKKASNALTVEIFADHPGQSGDGGGKGKGGKQQTGFKTVSSGYKDQLANLMKTLNATHPHFIRCIVPNEFKKPGEVDSGLIMHQLTCNGVLEGHPLFARRASPTGMPYKDFKLRYNILAAKEMLEAKDDKKAATACFERAGLNPELYRTGNTKVFFRAGVLGTLEEVRDDRIMKLVSWLQAWVRGWASRKYYSKMQKQRTALIVMQR

SEQ ID NO: 142 - protein, 13 aa, Penaeus monodon
VLSYFANVGASEK

SEQ ID NO: 143 - protein, 16 aa, Penaeus monodon
GMNVDQVNYNIGAMAK

SEQ ID NO: 144 - protein, 12 aa, Penaeus monodon
DPLNDTVVDQLK

SEQ ID NO: 145 - DNA, 2424 bp, Marsupenaeus japonicus
agcacgggtcccgaccccgaccccaccgaatatctcttcatctctcgggagcagaggatgaaggaccaaacgaaaccttacgatcctaagaagtctttctggtgtcccgatcccaatgaaggtttcgtcgagtgtgagcttcaaggtgcaaagggcgacaagcatgttacagttaagcttcccagtggcgagacgaaggactttaagaaggagcaggttggacaggtcaaccctcccaagtacgagaagtgtgaggatgtgtccaacttgaccttcctcaacgatccctccgtcttctacgttctcaagtcccgttaccaggccaagcttatctacacttattctggtctcttctgtatcgccgtcaacccttacaagcgctatcccatctataccaaccgtgccgtcaagatttatattggcaagaggcgtaatgaggtgccccctcatcttttcgccatctgcgacggcgcttaccagaacatgaatcaagaacgtcaaaaccagtctatgcttatcaccggtgaatccggtgctggaaagactgagaacacaaagaaggtgttgtcctacttcgccaacgttggtgcctcagagaaaaaagagggcgagtccaaacagaatcttgaggaccagattatccaaaccaaccccatccttgaggcttacggtaacgccaagaccactcgtaacgataactcttctcgtttcggtaagttcatccgcgtccactttgctcccaacggcaagctttccggcgctgatatcgaggtctacctgctggagaaggctcgtgtcatctcccagtcccccgccgagcgtggctaccatatcttctaccagctcatgtgtgatcaaattgactacatcaagaaaatatgtctcttgtccgacgacatttacgactaccattacgaagctcagggtaaggtcaccgtcccatccatcgacgacaaggaggacatgcagttcactcacgatgctttcgacgttctcaacttctcccatgaggaaagggacaactgctacaaggttactgcgtcagtcatgcattttggtaacatgaagttcaagcagaggggtcgtgaggagcaggctgaagccgacggtactgaggccggagaaattgttgcaactctgctcggtgttgacgccgaggagctctacaggaacttctgcaagcccaagatcaaggtcggtgctgagttcgtcaccaagggtatgaatgtcgaccaagtgaactacaatatcggtgccatggctaagggtatcttctcacgcgtgttctcatggctcgtcaggaagtgtaacatgacacttgagactggccagactcgtgccatgttcatcggtgtactcgatattgccggcttcgagatttttgatttcaacggtttcgagcagatttgtatcaacttctgtaatgagaagttgcagcaattcttcaaccatcacatgttcgtgctggagcaagaagaatatgcaaaggagggtattgtttggcagttcgtcgacttcggtatggatttgcaggcttgcattgaactcttcgagaagaaaatgggtctcctctccatcctcgaggaagagtctatgttccccaaggctactgacaagactttcgaggagaagctcaacaacaaccatctcggaaagtctcgttgcttcatcaagcccaagcctccgaagcccggccaacccgacaaccactttgccattgttcactacgctggcactgtgtcctacaacctgactggctggcttgagaagaacaaggatcctctcaacgacaccgttgtcgaccagctcaagaagtcctccaacgccctgacggttgagatcttcgctgaccatcccggccagtctggagatggaggaggcaaaggaaagggcggcaagcagcagactggtttcaaaactgtatcctctggatacaaggatcagcttggtaacttgatgaagactctcaatgccacccatcctcacttcatccgttgcattgtgcccaatgaattcaagaagcctggtgaagtagacgctggtctcattatgcatcagctaacttgcaacggtgtacttgagggtatccgtatttgccagaagggcttccccaacaggatgccatatcctgacttcaaacaacgatataacatcctggccgcccaggagatgatcgaagcaaaggacgataagaaggcagctcaagcatgtttccagagagctggactcgaccctgagttataccgcactggcaataccaaggtattcttccgagctggtgttttgggtacccttgaagaaattcgtgatgatcgtattatgaaactagtatcctggcttcaggcatggattcgtggctgggccagccgcaaattctatgctaagatgcagaagcagcgcactgcccttcttgttatgcagcgt

SEQ ID NO: 146 - protein, 808 aa, Marsupenaeus japonicus
STGPDPDPTEYLFISREQRMKDQTKPYDPKKSFWCPDPNEGFVECELQGAKGDKHVTVKLPSGETKDFKKEQVGQVNPPKYEKCEDVSNLTFLNDPSVFYVLKSRYQAKLIYTYSGLFCIAVNPYKRYPIYTNRAVKIYIGKRRNEVPPHLFAICDGAYQNMNQERQNQSMLITGESGAGKTENTKKVLSYFANVGASEKKEGESKQNLEDQIIQTNPILEAYGNAKTTRNDNSSRFGKFIRVHFAPNGKLSGADIEVYLLEKARVISQSPAERGYHIFYQLMCDQIDYIKKICLLSDDIYDYHYEAQGKVTVPSIDDKEDMQFTHDAFDVLNFSHEERDNCYKVTASVMHFGNMKFKQRGREEQAEADGTEAGEIVATLLGVDAEELYRNFCKPKIKVGAEFVTKGMNVDQVNYNIGAMAKGIFSRVFSWLVRKCNMTLETGQTRAMFIGVLDIAGFEIFDFNGFEQICINFCNEKLQQFFNHHMFVLEQEEYAKEGIVWQFVDFGMDLQACIELFEKKMGLLSILEEESMFPKATDKTFEEKLNNNHLGKSRCFIKPKPPKPGQPDNHFAIVHYAGTVSYNLTGWLEKNKDPLNDTVVDQLKKSSNALTVEIFADHPGQSGDGGGKGKGGKQQTGFKTVSSGYKDQLGNLMKTLNATHPHFIRCIVPNEFKKPGEVDAGLIMHQLTCNGVLEGIRICQKGFPNRMPYPDFKQRYNILAAQEMIEAKDDKKAAQACFQRAGLDPELYRTGNTKVFFRAGVLGTLEEIRDDRIMKLVSWLQAWIRGWASRKFYAKMQKQRTALLVMQR

SEQ ID NO: 147 - protein, 11 aa, Marsupenaeus japonicus
HVTVKLPSGET

SEQ ID NO: 148 - protein, 13 aa, Marsupenaeus japonicus
EQVGQVNPPKYEK

SEQ ID NO: 149 - protein, 13 aa, Marsupenaeus japonicus
VLSYFANVGASEK

SEQ ID NO: 150 - protein, 21 aa, Marsupenaeus japonicus
QNLEDQIIQTNPILEAYGNAK

SEQ ID NO: 151 - protein, 11 aa, Marsupenaeus japonicus
FIRVHFAPNGK

SEQ ID NO: 152 - protein, 13 aa, Marsupenaeus japonicus
LSGADIEVYLLEK

SEQ ID NO: 153 - protein, 16 aa, Marsupenaeus japonicus
GMNVDQVNYNIGAMAK

SEQ ID NO: 154 - protein, 19 aa, Marsupenaeus japonicus
LQQFFNHHMFVLEQEEYAK

SEQ ID NO: 155 - protein, 15 aa, Marsupenaeus japonicus
MGLLSILEEESMFPK

SEQ ID NO: 156 - protein, 12 aa, Marsupenaeus japonicus
DPLNDTVVDQLK

SEQ ID NO: 157 - protein, 12 aa, Marsupenaeus japonicus
GFPNRMPYPDFK

SEQ ID NO: 158 - protein, 22 aa, Marsupenaeus japonicus
AAQACFQRAGLDPELYRTGNTK

SEQ ID NO: 159 - protein, 10 aa, Marsupenaeus japonicus
QRTALLVMQR

SEQ ID NO: 160 - DNA, 3222 bp, Litopenaeus vannamei
gtgaagcccctcatcaaccaaccaaggattgaagacgagatcaacaagctcaaggacagggctgagaaggctgttgcagacttggatcgcgagtgtactcgccgcaaggagctggaagaatccaacgtgagccttgccgaagagctgaataccctgaaggaaacgcttgaatccacaaagggcaatgtttccaaattcattgaagaacaggccaagattagtgcagccaaagctgacttggaggctcagctctctgatgcttctgctagacttcagaaagaagaggaaaatcgcactgaaatgttccagttgaagaggaaagcggagcaagatgtcaatgccatgaggaaagacctggaagattttgaacttaatgttcagaagactaaccaggataaggctaccaaggatcaccagatcaggaatatcaatgatgaaatatctcaccaggatgaaatcatcaacaaggttaacaaggaaaagaaacttttgcaggagatgaatcaaaagactgctgaggatcttcaggccgtcgaggaaaaggccagccacctcaacaagataaaggccaagttggaacaaaccctcgacgaactcgagggttccgttggacgcgagaagaagcttcgtgctgaaattgagaggtccaagaggaaggtagagggagatctgaaaatgacccaagaaactgttgctgacatcgagcgccagcataaggacctggagcaaaccatccagcgtaaggataaggaaatcggcaatcttgccaataaactggaggaggaacaagtggtagtttcgaaggtacagaagacaatcaaagaaatgcaagcccgcattgaggaactcgagactgaagctgagcatgagcggcaggctcgtgccaaggccgagaagggcaagggaaatatgagccgtgaactcaatgacctcaatgagcgtctggatgaggcaggcggtgcaacaggtgctcaggttgagctcaacaagaagcgggaggcggagctgggtaagcttcgacgtgacctcgaggaagccaacatccaacacgaatcagctcttgctaaccttcgcaagaagcacaatgatgctgttgccgagatgactgaacagatcgaccatctcaacaagacgaaggccaagactgaaaaggaaaaagagatgatgaaatatcaggccgatgaagctaaatcagccatggatagtctcgctcgtgacaaggcacttgccgagaaagcgaacaagaccattcagcagcaaatcaatgaagttaatgtgaagctggatgaagctaaccgcactctgaacgacttcgatgcccagaagaagaagctctctgttgagaacggagaccttctgcgacagctggaggaggctgataatcagattaatcagctgaacaatttgaagttgtctcttaccactcagctggaagatactaagaaaatggttgatgatgaatctagggagcgcggtgttcttcttggcaagttccgcaacctggagcatgatctggatggtcttcgtgagcagcttgatgaagagtgtgaagccaaggctgatgccaaccgccaactgtccaaggcttatgcagaggctcagatgtggcgctctaagtatgaatcagagggcgttgcccgtgctgaagagattgaggctgcccgcctgaaacttgccgctcgcctcgaggaagctgagctgcagattgaacaactcaatgtcaagaacatgcaactggagaaggccaagggacgcatcatttccgaaatcgacgagatgcagatgcaggtagagcgtgcccaaggtctggctaatgctgctgagaggaggcagaaggacttcgacagagttgttaatgagtggaagatcaaggttgaccaactggccactgaacttgatgcttcccagaaggaatgtcgccagtactccactgagcacttccgcatcaaagccgtgtatgaggaaaacctggaacacctggactctgttcgtcgtgagaacaagggtctcgctgaggagatcaaggacctgatggagcagatcagtgagggtggccgctctcttcatgagattgaaaagaacgccaagcgtttcgagatcgagaaggaggagctccaggctgctcttgaggaagccgaagctgcccttgaacaggaagagaacaaggttcttcgtggtcagctggagctgagccaagtcaggcaagagattgataagcgcattcaggagaaggaggaagagtttgatgctactcgtaagtgccaccaacgtgcaatcgaatccatgcaagcctcacttgaagcagaagctaagagcaaggctgaggctcttcgtatgaagaagaagcttgagtctgacattggtgagctggagattgctctcgatcacgctaacaaggcaaatgccgacattcagaagcaggtgaagaaggctcaggctgagatgaaagacatgcaagctcgtgtggaggaggagcagcgtcttgcttctgagtatcgcgagcagtgcagcgcctccgagcgtaaggccaatgctgtcaatggtgaactggaggaatcccgcactcttctggagcagtctgatcgcggacgccgtcaggctgaatccgaacttgctgatgccaatgagtccctgagccatcttactgctcagcatggatccctctccatggcaaagaggaaacttgagggcgagatccagactctccatgctgaacttgatgacatgctgaacgaggccaagaactctgaggacaaggccaagaaggccatggttgatgctgctcgtctggctgacgaactccgtgctgagcaagaacatgcccaaacccaggagaagatgcgcaagggcctcgatttgtctgtcaaggatctccaggcccgcctggatgaattcgaatcttcagctcacaagaccggcaagaaggccctcgctaagctggaagctcgcatccgtgaactggagaatcagctggacgacgagagtcgccgtcacgccgacgctcagaagaacctgaggaagtgcgagaggcgcatcaaggagctcagcttccagtctgaagaggacaagaagaaccacgagaggatgcaggacctggtggacaagctccagcagaagatcaagacctacaagcgccagatcgaggaggccgaggagatcgccgccctcaacctggccaagtaccgtaaagcacagcaggagcttgagacagtgcagaggagc

SEQ ID NO: 161 - protein, 1074 aa, Litopenaeus vannamei
VKPLINQPRIEDEINKLKDRAEKAVADLDRECTRRKELEESNVSLAEELNTLKETLESTKGNVSKFIEEQAKISAAKADLEAQLSDASARLQKEEENRTEMFQLKRKAEQDVNAMRKDLEDFELNVQKTNQDKATKDHQIRNINDEISHQDEIINKVNKEKKLLQEMNQKTAEDLQAVEEKASHLNKIKAKLEQTLDELEGSVGREKKLRAEIERSKRKVEGDLKMTQETVADIERQHKDLEQTIQRKDKEIGNLANKLEEEQVVVSKVQKTIKEMQARIEELETEAEHERQARAKAEKGKGNMSRELNDLNERLDEAGGATGAQVELNKKREAELGKLRRDLEEANIQHESALANLRKKHNDAVAEMTEQIDHLNKTKAKTEKEKEMMKYQADEAKSAMDSLARDKALAEKANKTIQQQINEVNVKLDEANRTLNDFDAQKKKLSVENGDLLRQLEEADNQINQLNNLKLSLTTQLEDTKKMVDDESRERGVLLGKFRNLEHDLDGLREQLDEECEAKADANRQLSKAYAEAQMWRSKYESEGVARAEEIEAARLKLAARLEEAELQIEQLNVKNMQLEKAKGRIISEIDEMQMQVERAQGLANAAERRQKDFDRVVNEWKIKVDQLATELDASQKECRQYSTEHFRIKAVYEENLEHLDSVRRENKGLAEEIKDLMEQISEGGRSLHEIEKNAKRFEIEKEELQAALEEAEAALEQEENKVLRGQLELSQVRQEIDKRIQEKEEEFDATRKCHQRAIESMQASLEAEAKSKAEALRMKKKLESDIGELEIALDHANKANADIQKQVKKAQAEMKDMQARVEEEQRLASEYREQCSASERKANAVNGELEESRTLLEQSDRGRRQAESELADANESLSHLTAQHGSLSMAKRKLEGEIQTLHAELDDMLNEAKNSEDKAKKAMVDAARLADELRAEQEHAQTQEKMRKGLDLSVKDLQARLDEFESSAHKTGKKALAKLEARIRELENQLDDESRRHADAQKNLRKCERRIKELSFQSEEDKKNHERMQDLVDKLQQKIKTYKRQIEEAEEIAALNLAKYRKAQQELETVQRS

SEQ ID NO: 162 - protein, 11 aa, Litopenaeus vannamei
TAEDLQAVEEK

SEQ ID NO: 163 - protein, 8 aa, Litopenaeus vannamei
EIGNLANK

SEQ ID NO: 164 - protein, 10 aa, Litopenaeus vannamei
LEEEQVVVSK

SEQ ID NO: 165 - protein, 29 aa, Litopenaeus vannamei
GNMSRELNDLNERLDEAGGATGAQVELNK

SEQ ID NO: 166 - protein, 11 aa, Litopenaeus vannamei
LSLTTQLEDTK

SEQ ID NO: 167 - protein, 18 aa, Litopenaeus vannamei
LAARLEEAELQIEQLNVK

SEQ ID NO: 168 - protein, 13 aa, Litopenaeus vannamei
VDQLATELDASQK

SEQ ID NO: 169 - protein, 13 aa, Litopenaeus vannamei
ECRQYSTEHFRIK

SEQ ID NO: 170 - protein, 18 aa, Litopenaeus vannamei
AVYEENLEHLDSVRRENK

SEQ ID NO: 171 - protein, 18 aa, Litopenaeus vannamei
DLMEQISEGGRSLHEIEK

SEQ ID NO: 172 - protein, 20 aa, Litopenaeus vannamei
EELQAALEEAEAALEQEENK

SEQ ID NO: 173 - protein, 17 aa, Litopenaeus vannamei
VLRGQLELSQVRQEIDK

SEQ ID NO: 174 - protein, 15 aa, Litopenaeus vannamei
DLQARLDEFESSAHK

SEQ ID NO: 175 - protein, 11 aa, Litopenaeus vannamei
NHERMQDLVDK

SEQ ID NO: 176 - protein, 16 aa, Litopenaeus vannamei
RQIEEAEEIAALNLAK

SEQ ID NO: 177 - protein, 11 aa, Litopenaeus vannamei
AQQELETVQRS

SEQ ID NO: 178 - DNA, 3222 bp, Penaeus monodon
gtcaagcccctcatcaaccagcctaggattgaagatgagatcaacaaactcaaggacagggctgagaaggctgttgcagacttggatcgcgaaacaactcgccgaaaggagctggaagattccaacctaagccttgccgaagagctgaataccctgaaagaaacgcttgaatccacaaagggcaatgtttccaaatttattgaagaacaggccaagattagcgcagccaaagctgacttggaggcacagctctctgatgcttctgcaagacttcagaaggaagaagaatctcgcactgaaatgttccagttgaagaggaaagcggagcaagatgtcaatgccatgaggaaagacctggaagactttgaacttaatgtccagaagactaaccaggataaggctaccaaggatcatcagatcaggaatatcaatgatgagatcgcccaccaggatgaaatcatcaacaaggttaacaaggaaaagaaactgctgcaggagatgaatcaaaagactgctgaggatcttcaggccgtcgaggagaaggccagccacctcaacaagatcaagtccaagttggagcaaaccctcgacgaactcgagagttccgttggacgcgagaagaagcttcgtgccgaaattgagaggtccaagaggaaggtagagggagatcttaaaatgacccaagaaactgttgctgacatcgagcgccaacacaaggacctagaacaaaccatccagcgcaaggacaaggaaatcggcaatcttgccaataagctggaggaggaacagggagttgtttcgaaggtacagaaaacaatcaaagaaatgcaagcccgcattgaggaactggagactgaagctgagcacgagcgacaggctcgtgccaaggctgagaagggaaagggtaatatgagccgtgaactgaatgacctcaatgaacgtctggatgaagcaggtggtgcaactggtgctcagatggaactcaacaagaagagggaggcggagcttgctaagcttcgtcgtgacctcgaggaagccaacatccaacacgaatcggctcttgctaatcttcgcaagaagcacaatgatgctgttgccgagatgactgaacagatcgatcatctcaataaaatgaaggccaaaactgagaaggaaaaggagatgatgaaatatcaggccgatgaagctaaatcagccatggatagtctcgctcgtgacaaggcacttgccgagaaagcgaacaagactattcagcagcaaatcaacgaagtgaatgtgaagctggatgaagctaaccgcacactgagagactttgatgcccagaagaagaagctctccgttgagaatggagacctgctgcgacagctggaagaagctgataatcagattaatcagctaaacaatctgaaggtgtctcttaccactcaactggaagatactaagaaaatggttgatgatgaatctagggagcgcagcgttcttcttggcaagttccgcaacttggagcatgatctggatggtcttcgtgagcagcttgatgaagagtgtgaagccaaggctgatgccaaccgccagctgtccaaggctcatgctgaggctcagatgtggcgctcaaagtatgaatctgagggcgttgcccgtgctgaagagatcgaagctgcccgcctgaagcttgccgctcgtctcgaggaagccgagctgcagattgaacaactcaatgtcaagaatatgcagctggagaaggccaagggacgcatcatttccgaaatcgacgagatgcagatgcaggtagagcgtgcccagggaatggctattgctgctgagaggaggcagaaagacttcgacagggttgttaatgagtggaagatcaaggttgaccaactggccactgagcttgatgcttctcaaaaggaatgtcgtcagtactccactgagcacttccgcatcaaggccgtgtatgaggaaaacctggaacacctggactctgttcgtcgtgagaacaagggtctcgctgaggagatcaaggacttgatggagcagatcagcgagggtggccgctctcttcatgagattgaaaagaacgccaagcgtttcgagatcgagaaggaggagctccaggctgctcttgaggaggccgaagctgcccttgaacaggaagagaacaaggttcttcgtggtcagttggagctgagccaagtcaggcaggagattgataagcgcattcaggagaaggaagaagagtttgatgccactcgtaaatgtcaccaacgtgcaatcgaatccatgcaagcttcacttgaagcagaagctaagagcaaggctgaggccctccgcatgaagaagaagcttgaatctgacattggtgagctggagattgctctggatcacgctaacaaggccaatgctgacattcagaagcaggtgaagaaggctcaggccgagatgaaggacatgcaggctcgtgtggaggaggagcagcgtcttgcttctgagtatcgcgagcagtgcagtgcctctgagcgtaaggccaatgctgtcaatggtgaactggaggaatcccgcactcttctggaacagtctgatcgcggacgccgtcaggctgaatccgagcttgctgatgccaatgagtccctcagccaccttacggctcagcatggatccctttccatggcgaagaggaagcttgagggcgagattcagactctgcatgctgaacttgatgacatgcttaatgaggccaagaactctgaggacaaggccaagaaggccatggttgatgctgctcgtctggccgatgaactccgagctgagcaagaacatgcccaaacccaggagaagatgcgcaagggactcgatttgtctgttaaggatctccaagctcgcctggatgaattcgagtcttcagctcacaagaccggcaagaaggccctcgctaagttggaagctcgcatccgcgaactggaaaatcagctggacgacgagagtcgccgtcacgccgacgcccagaagaacctgaggaagtgcgagaggcgcatcaaggaactcagcttccagtctgaggaggacaagaagaaccacgagaggatgcaggacctggtcgacaagctccagcagaagatcaagacctacaagcgccagatcgaggaggccgaggagatcgccgcccttgacctggccaagtatcgtaaagcacagcaggagcttgagacagtgcagaggagc

SEQ ID NO: 179 - protein, 1074 aa, Penaeus monodon
VKPLINQPRIEDEINKLKDRAEKAVADLDRETTRRKELEDSNLSLAEELNTLKETLESTKGNVSKFIEEQAKISAAKADLEAQLSDASARLQKEEESRTEMFQLKRKAEQDVNAMRKDLEDFELNVQKTNQDKATKDHQIRNINDEIAHQDEIINKVNKEKKLLQEMNQKTAEDLQAVEEKASHLNKIKSKLEQTLDELESSVGREKKLRAEIERSKRKVEGDLKMTQETVADIERQHKDLEQTIQRKDKEIGNLANKLEEEQGVVSKVQKTIKEMQARIEELETEAEHERQARAKAEKGKGNMSRELNDLNERLDEAGGATGAQMELNKKREAELAKLRRDLEEANIQHESALANLRKKHNDAVAEMTEQIDHLNKMKAKTEKEKEMMKYQADEAKSAMDSLARDKALAEKANKTIQQQINEVNVKLDEANRTLRDFDAQKKKLSVENGDLLRQLEEADNQINQLNNLKVSLTTQLEDTKKMVDDESRERSVLLGKFRNLEHDLDGLREQLDEECEAKADANRQLSKAHAEAQMWRSKYESEGVARAEEIEAARLKLAARLEEAELQIEQLNVKNMQLEKAKGRIISEIDEMQMQVERAQGMAIAAERRQKDFDRVVNEWKIKVDQLATELDASQKECRQYSTEHFRIKAVYEENLEHLDSVRRENKGLAEEIKDLMEQISEGGRSLHEIEKNAKRFEIEKEELQAALEEAEAALEQEENKVLRGQLELSQVRQEIDKRIQEKEEEFDATRKCHQRAIESMQASLEAEAKSKAEALRMKKKLESDIGELEIALDHANKANADIQKQVKKAQAEMKDMQARVEEEQRLASEYREQCSASERKANAVNGELEESRTLLEQSDRGRRQAESELADANESLSHLTAQHGSLSMAKRKLEGEIQTLHAELDDMLNEAKNSEDKAKKAMVDAARLADELRAEQEHAQTQEKMRKGLDLSVKDLQARLDEFESSAHKTGKKALAKLEARIRELENQLDDESRRHADAQKNLRKCERRIKELSFQSEEDKKNHERMQDLVDKLQQKIKTYKRQIEEAEEIAALDLAKYRKAQQELETVQRS

SEQ ID NO: 180 - protein, 14 aa, Penaeus monodon
PLINQPRIEDEINK

SEQ ID NO: 181 - protein, 17 aa, Penaeus monodon
ELEDSNLSLAEELNTLK

SEQ ID NO: 182 - protein, 7 aa, Penaeus monodon
FIEEQAK

SEQ ID NO: 183 - protein, 16 aa, Penaeus monodon
ADLEAQLSDASARLQK

SEQ ID NO: 184 - protein, 12 aa, Penaeus monodon
EEESRTEMFQLK

SEQ ID NO: 185 - protein, 11 aa, Penaeus monodon
DLEDFELNVQK

SEQ ID NO: 186 - protein, 20 aa, Penaeus monodon
DHQIRNINDEIAHQDEIINK

SEQ ID NO: 187 - protein, 8 aa, Penaeus monodon
LLQEMNQK

SEQ ID NO: 188 - protein, 11 aa, Penaeus monodon
TAEDLQAVEEK

SEQ ID NO: 189 - protein, 16 aa, Penaeus monodon
LEQTLDELESSVGREK

SEQ ID NO: 190 - protein, 14 aa, Penaeus monodon
MTQETVADIERQHK

SEQ ID NO: 191 - protein, 9 aa, Penaeus monodon
DLEQTIQRK

SEQ ID NO: 192 - protein, 10 aa, Penaeus monodon
DKEIGNLANK

SEQ ID NO: 193 - protein, 10 aa, Penaeus monodon
LEEEQGVVSK

SEQ ID NO: 194 - protein, 22 aa, Penaeus monodon
EMQARIEELETEAEHERQARAK

SEQ ID NO: 195 - protein, 29 aa, Penaeus monodon
GNMSRELNDLNERLDEAGGATGAQMELNK

SEQ ID NO: 196 - protein, 21 aa, Penaeus monodon
LRRDLEEANIQHESALANLRK

SEQ ID NO: 197 - protein, 17 aa, Penaeus monodon
HNDAVAEMTEQIDHLNK

SEQ ID NO: 198 - protein, 10 aa, Penaeus monodon
SAMDSLARDK

SEQ ID NO: 199 - protein, 12 aa, Penaeus monodon
TIQQQINEVNVK

SEQ ID NO: 200 - protein, 26 aa, Penaeus monodon
LSVENGDLLRQLEEADNQINQLNNLK

SEQ ID NO: 201 - protein, 11 aa, Penaeus monodon
VSLTTQLEDTK

SEQ ID NO: 202 - protein, 15 aa, Penaeus monodon
MVDDESRERSVLLGK

SEQ ID NO: 203 - protein, 22 aa, Penaeus monodon
FRNLEHDLDGLREQLDEECEAK

SEQ ID NO: 204 - protein, 11 aa, Penaeus monodon
AHAEAQMWRSK

SEQ ID NO: 205 - protein, 18 aa, Penaeus monodon
YESEGVARAEEIEAARLK

SEQ ID NO: 206 - protein, 18 aa, Penaeus monodon
LAARLEEAELQIEQLNVK

SEQ ID NO: 207 - protein, 29 aa, Penaeus monodon
GRIISEIDEMQMQVERAQGMAIAAERRQK

SEQ ID NO: 208 - protein, 10 aa, Penaeus monodon
DFDRVVNEWK

SEQ ID NO: 209 - protein, 13 aa, Penaeus monodon
VDQLATELDASQK

SEQ ID NO: 210 - protein, 13 aa, Penaeus monodon
ECRQYSTEHFRIK

SEQ ID NO: 211 - protein, 13 aa, Penaeus monodon
VDQLATELDASQK

SEQ ID NO: 212 - protein, 18 aa, Penaeus monodon
AVYEENLEHLDSVRRENK

SEQ ID NO: 213 - protein, 8 aa, Penaeus monodon
DSVRRENK

SEQ ID NO: 214 - protein, 18 aa, Penaeus monodon
DLMEQISEGGRSLHEIEK

SEQ ID NO: 215 - protein, 20 aa, Penaeus monodon
EELQAALEEAEAALEQEENK

SEQ ID NO: 216 - protein, 17 aa, Penaeus monodon
VLRGQLELSQVRQEIDK

SEQ ID NO: 217 - protein, 9 aa, Penaeus monodon
EEEFDATRK

SEQ ID NO: 218 - protein, 18 aa, Penaeus monodon
CHQRAIESMQASLEAEAK

SEQ ID NO: 219 - protein, 17 aa, Penaeus monodon
LESDIGELEIALDHANK

SEQ ID NO: 220 - protein, 26 aa, Penaeus monodon
DMQARVEEEQRLASEYREQCSASERK

SEQ ID NO: 221 - protein, 50 aa, Penaeus monodon
ANAVNGELEESRTLLEQSDRGRRQAESELADANESLSHLTAQHGSLSMAK

SEQ ID NO: 222 - protein, 20 aa, Penaeus monodon
LEGEIQTLHAELDDMLNEAK

SEQ ID NO: 223 - protein, 24 aa, Penaeus monodon
AMVDAARLADELRAEQEHAQTQEK

SEQ ID NO: 224 - protein, 15 aa, Penaeus monodon
DLQARLDEFESSAHK

SEQ ID NO: 225 - protein, 24 aa, Penaeus monodon
LEARIRELENQLDDESRRHADAQK

SEQ ID NO: 226 - protein, 10 aa, Penaeus monodon
ELSFQSEEDK

SEQ ID NO: 227 - protein, 11 aa, Penaeus monodon
NHERMQDLVDK

SEQ ID NO: 228 - protein, 11 aa, Penaeus monodon
AQQELETVQRS

SEQ ID NO: 229 - DNA, 3225 bp, Marsupenaeus japonicus
gtgaagcccctcatcaaccagccaaggttggaagacgagatcaacaagctcaaggacagggctgagaaggctgttgcagacttagatcgcgagtctactcgccgcaaggagctggaagagtctaacgtaactcttgcagaagagctgaacaacctgaaggttactctcgaatccacaaagggcaatgtctccaaattcattgaagaacaagccaagattagtgcagctaaagctgacttggaagctcagctctctgatgccagcgcaaaactccataaggaagaggaatctcgtactgagatgttccagttgaagaggaaagcagagcaagatgtcaatgctatgaggaaagaccttgaagattttgaactcaatgttcagaaaactaaccaggataaggctaccaaggatcatcagatcaggaacatcaatgacgagatctcccatcaggatgaactcatcaacaaggttaacaaagaaaagaagcacctgcaggagatgaaccagaagactgctgaggatctccagagtgtcgaggagaaggccagccatctcaacaagatcaaggccaagttggagcaaacccttgacgaactcgagagctccgttggacgcgagaagaagcttcgtgctgagattgagaggtccaagaggaaggtagagggtgatcttaaaatgacccaagaaaccgttgctgacatcgagcgccagcacaaggacctggaacaaaccatccagcgcaaggataaggaaatcggcaaccttgccaataagctggaagaggaacagggagttgtctcgaaggttcaaaagggtattaggaaaaatgcaaggcccgcatttgaggagcttgagactgaagctgagcatgagcgacaggctcgcgccaaggctgagaagggcaagggcatgatgagccgagagctcaatgacctcaatgaacgtctggatgaggcaggtggtgcaactggtgctcagattgaactcaacaagaagcgtgaggctgaactgggcaagctccgtcgtgacctcgaggaagctaacatccagcacgaatcagctcttgccaatcttcgcaagaagcacaatgatgctgttgctgagatgacagagcagatcgaccatctcaataagatgaaggccaaaactgaaaaggaaaaggagatgatgaagtaccaggccgatgaagctaaatcagctatggacaatctcgctcgtgacaaggcacttgctgagaaagcaaacaagactattcagcagcaaatcagtgaagtgaatgtcaagctggatgaagctaaccgcacactgaacgacttcgatgtccacaagaagaaacttgccgttgagaacggagaccttctgcgacagctggaggaggctgataatcagattaatcagctgaacaatctgaaggtgtctctaaccactcagctggaggacaccaagaaaatggtcgatgatgaatctagggaacgcagtgttctcctgggcaagttccgcaacttggagcatgatctggatggtcttcgtgagcagctcgacgaagagtgtgaagctaaggctgatgctaatcgccagctgtccaaggcccatggcgaagcacaaatgtggcgctctaagtacgaatctgaaggcgttgctcgtgctgaggagatcgaggctgcccgtctgaagcttgctgctcgtcttgaggaggctgagctgcagatcgagcaactcaatgtcaagaatatgcaactggagaaggccaagggacgcattattaccgaaatcgacgagatgcagatgcaagtagagcgtgcccagggtctggctaatgcagcggataggaggcagaaggacttcgacagggttgttaatgaatggaagattaaggttgaccaacttgccactgagcttgatgcttcccagaaggaatgtcgccaatactcaactgaacacttccgcatcaaagctgtgtatgaggaaaacctggagcacctggactctgttcgtcgcgagaacaagggtcttgctgaggagatcaaggacttgatggaacagatcagcgaaggtggccgatcccttcacgaaattgaaaagaacgccaagcgtttcgagatcgagaaggaagagctccaggctgcccttgaggaggccgaagctgcccttgaacaggaagagaacaaggtccttcgtggccagctggagctgagccaagtcaggcaggagattgataagcgcattcaggagaaggaggaggaatttgatgccactcgtaagtgccaccagcgcgcaattgagtccatgcaagcttctcttgaagcagaggctaagagcaaggctgaagctcttcgcatgaagaagaagctcgagtctgacatcggcgaactcgagattgctcttgatcacgctaacaaggccaatgccgacattcagaagcaggtgaagaaggcccaggccgagatgaaggacatgcaagctcgcatggaggaagaacagcgtcttgcttctgagtatcgtgagcagtgcagcgcttccgagcgtaaggccaacgctgttaacggtgaactggaagaatcccgcactcttctggagcagtctgatcgcggacgccgccaggctgaatccgagcttgctgatgccaacgaatccctcagccaccttacagctcagcatggatccctctccatggcgaagaggaaacttgagggcgagattcagactctccatgctgaacttgatgacatgctgaacgaggccaagaactccgaggacaaggccaagaaggccatggttgatgctgcccgtctggctgacgaacttcgtgctgaacaagagcatgcccaaacccaggagaagatgcgcaagggcctggatttgtctgtcaaggatctccaagctcgcctggatgaattcgagtctacagctcacaagactggcaagaaggcactcgctaagctggaaggtcgcatccgtgatctcgaaagtcacttggacgacgaggctcgccgccacgccgacgcccagaagaacctgaggaagtgcgagaggcgcatcaaggagctcaccttccagtccgacgaggacaagaagaaccacgagaggatgcaggacctggtcgacaagctgcagcagaagatcaagacctacaagcgccagatcgaggaggctgaggagatcgccgccctcaacctggccaagtaccgcaaagctcaacaggaacttgaaacagttcagaggagc

SEQ ID NO: 230 - protein, 1075 aa, Marsupenaeus japonicus
VKPLINQPRLEDEINKLKDRAEKAVADLDRESTRRKELEESNVTLAEELNNLKVTLESTKGNVSKFIEEQAKISAAKADLEAQLSDASAKLHKEEESRTEMFQLKRKAEQDVNAMRKDLEDFELNVQKTNQDKATKDHQIRNINDEISHQDELINKVNKEKKHLQEMNQKTAEDLQSVEEKASHLNKIKAKLEQTLDELESSVGREKKLRAEIERSKRKVEGDLKMTQETVADIERQHKDLEQTIQRKDKEIGNLANKLEEEQGVVSKVQKGIRKNARPAFEELETEAEHERQARAKAEKGKGMMSRELNDLNERLDEAGGATGAQIELNKKREAELGKLRRDLEEANIQHESALANLRKKHNDAVAEMTEQIDHLNKMKAKTEKEKEMMKYQADEAKSAMDNLARDKALAEKANKTIQQQISEVNVKLDEANRTLNDFDVHKKKLAVENGDLLRQLEEADNQINQLNNLKVSLTTQLEDTKKMVDDESRERSVLLGKFRNLEHDLDGLREQLDEECEAKADANRQLSKAHGEAQMWRSKYESEGVARAEEIEAARLKLAARLEEAELQIEQLNVKNMQLEKAKGRIITEIDEMQMQVERAQGLANAADRRQKDFDRVVNEWKIKVDQLATELDASQKECRQYSTEHFRIKAVYEENLEHLDSVRRENKGLAEEIKDLMEQISEGGRSLHEIEKNAKRFEIEKEELQAALEEAEAALEQEENKVLRGQLELSQVRQEIDKRIQEKEEEFDATRKCHQRAIESMQASLEAEAKSKAEALRMKKKLESDIGELEIALDHANKANADIQKQVKKAQAEMKDMQARMEEEQRLASEYREQCSASERKANAVNGELEESRTLLEQSDRGRRQAESELADANESLSHLTAQHGSLSMAKRKLEGEIQTLHAELDDMLNEAKNSEDKAKKAMVDAARLADELRAEQEHAQTQEKMRKGLDLSVKDLQARLDEFESTAHKTGKKALAKLEGRIRDLESHLDDEARRHADAQKNLRKCERRIKELTFQSDEDKKNHERMQDLVDKLQQKIKTYKRQIEEAEEIAALNLAKYRKAQQELETVQRS

SEQ ID NO: 231 - protein, 14 aa, Marsupenaeus japonicus
PLINQPRLEDEINK

SEQ ID NO: 232 - protein, 13 aa, Marsupenaeus japonicus
AVADLDRESTRRK

SEQ ID NO: 233 - protein, 17 aa, Marsupenaeus japonicus
ELEESNVTLAEELNNLK

SEQ ID NO: 234 - protein, 7 aa, Marsupenaeus japonicus
FIEEQAK

SEQ ID NO: 235 - protein, 13 aa, Marsupenaeus japonicus
ADLEAQLSDASAK

SEQ ID NO: 236 - protein, 12 aa, Marsupenaeus japonicus
EEESRTEMFQLK

SEQ ID NO: 237 - protein, 11 aa, Marsupenaeus japonicus
DLEDFELNVQK

SEQ ID NO: 238 - protein, 11 aa, Marsupenaeus japonicus
TAEDLQSVEEK

SEQ ID NO: 239 - protein, 16 aa, Marsupenaeus japonicus
LEQTLDELESSVGREK

SEQ ID NO: 240 - protein, 14 aa, Marsupenaeus japonicus
MTQETVADIERQHK

SEQ ID NO: 241 - protein, 9 aa, Marsupenaeus japonicus
DLEQTIQRK

SEQ ID NO: 242 - protein, 10 aa, Marsupenaeus japonicus
LEEEQGVVSK

SEQ ID NO: 243 - protein, 8 aa, Marsupenaeus japonicus
EIGNLANK

SEQ ID NO: 244 - protein, 29 aa, Marsupenaeus japonicus
GMMSRELNDLNERLDEAGGATGAQIELNK

SEQ ID NO: 245 - protein, 21 aa, Marsupenaeus japonicus
LRRDLEEANIQHESALANLRK

SEQ ID NO: 246 - protein, 17 aa, Marsupenaeus japonicus
HNDAVAEMTEQIDHLNK

SEQ ID NO: 247 - protein, 12 aa, Marsupenaeus japonicus
TIQQQISEVNVK

SEQ ID NO: 248 - protein, 26 aa, Marsupenaeus japonicus
LAVENGDLLRQLEEADNQINQLNNLK

SEQ ID NO: 249 - protein, 11 aa, Marsupenaeus japonicus
VSLTTQLEDTK

SEQ ID NO: 250 - protein, 15 aa, Marsupenaeus japonicus
MVDDESRERSVLLGK

SEQ ID NO: 251 - protein, 22 aa, Marsupenaeus japonicus
FRNLEHDLDGLREQLDEECEAK

SEQ ID NO: 252 - protein, 18 aa, Marsupenaeus japonicus
YESEGVARAEEIEAARLK

SEQ ID NO: 253 - protein, 18 aa, Marsupenaeus japonicus
LAARLEEAELQIEQLNVK

SEQ ID NO: 254 - protein, 18 aa, Marsupenaeus japonicus
AVYEENLEHLDSVRRENK

SEQ ID NO: 255 - protein, 29 aa, Marsupenaeus japonicus
GRIITEIDEMQMQVERAQGLANAADRRQK

SEQ ID NO: 256 - protein, 10 aa, Marsupenaeus japonicus
DFDRVVNEWK

SEQ ID NO: 257 - protein, 13 aa, Marsupenaeus japonicus
VDQLATELDASQK

SEQ ID NO: 258 - protein, 13 aa, Marsupenaeus japonicus
ECRQYSTEHFRIK

SEQ ID NO: 259 - protein, 8 aa, Marsupenaeus japonicus
DSVRRENK

SEQ ID NO: 260 - protein, 18 aa, Marsupenaeus japonicus
DLMEQISEGGRSLHEIEK

SEQ ID NO: 261 - protein, 20 aa, Marsupenaeus japonicus
EELQAALEEAEAALEQEENK

SEQ ID NO: 262 - protein, 17 aa, Marsupenaeus japonicus
VLRGQLELSQVRQEIDK

SEQ ID NO: 263 - protein, 9 aa, Marsupenaeus japonicus
EEEFDATRK

SEQ ID NO: 264 - protein, 18 aa, Marsupenaeus japonicus
CHQRAIESMQASLEAEAK

SEQ ID NO: 265 - protein, 17 aa, Marsupenaeus japonicus
LESDIGELEIALDHANK

SEQ ID NO: 266 - protein, 26 aa, Marsupenaeus japonicus
DMQARMEEEQRLASEYREQCSASERK

SEQ ID NO: 267 - protein, 50 aa, Marsupenaeus japonicus; identical to SEQ ID NO: 221

SEQ ID NO: 268 - protein, 20 aa, Marsupenaeus japonicus
LEGEIQTLHAELDDMLNEAK

SEQ ID NO: 269 - protein, 24 aa, Marsupenaeus japonicus
AMVDAARLADELRAEQEHAQTQEK

SEQ ID NO: 270 - protein, 24 aa, Marsupenaeus japonicus
LEGRIRDLESHLDDEARRHADAQK

SEQ ID NO: 271 - protein, 10 aa, Marsupenaeus japonicus
ELTFQSDEDK

SEQ ID NO: 272 - protein, 11 aa, Marsupenaeus japonicus
NHERMQDLVDK

SEQ ID NO: 273 - protein, 16 aa, Marsupenaeus japonicus
RQIEEAEEIAALNLAK

SEQ ID NO: 274 - protein, 11 aa, Marsupenaeus japonicus
AQQELETVQRS

SEQ ID NO: 275 - DNA, 2241 bp, Litopenaeus vannamei
gagggcttcgctgaaggcttgatccaggaagccaagggtgacaaactagtcagcgtccagctgaagagcggcgaggtcaaggactttaagaaggatcttgtggttcaggtcaaccctcccaagtacgaaaagtgcgaagatgtgtccaacttgaccttcctcaacgatgcttctgtcctgtacaacttgaagagccgttaccaggccaagctgatctacacctactccggcctcttctgtattgtcattaacccctacaagcgttaccccatctacaccaaccgcaccgtcaagatctaccagggcaagaggcgcaatgaggtgcctcctcatctcttcgccatctccgacggcgcctacatggacatgttgcaatctcagcagaaccagtcgatgcttatcactggcgaatctggcgccggtaagaccgagaacacgaagaaggtgctgtcctacttcgccaacgtcggcgccaccaccaagaagaaggaagatgagaaaaaacagaacctggaggaccagatcgtgcagaccaaccctcccctggaggcttacggcaacgccaagactactcgtaatgacaattcttctcgtttcggcaaattcatccgcatccacttcgcccccaacggcaagctctccggggctgacatcgaggtgtacctgctggagaaggctcgcgtggtgtcccaggcccctgccgagcgtggctaccatatcttctaccagatgatgtcagatcaagtagattacttaaaaaaactgtgtcatctttccgacgatatttacgactaccgctacgagtgccagggcaaggtcactgtgccttccattgacgacaaggaagacatggaattcacacataatgctttcaccattttgaacttcactaacgaagaacgtgacagctgctacaaagtcactgccgctgtcatgcaccatggtaacatgaagttcaagcagaggggtcgcgaggagcaggctgagcccgacggcacagatgccggtgatattgttgctactattatgggagttgaaagtgaggaattgtacaggaatttctgtaagcccaagatcaaggtcggtgccgagttcgtcacccagggtaggaatgtcgaccaggtgtactattccattagcgccatggctaagggcttgttcgaccgtctcttcaagtggatcgtgaagaagtgtaaccagaccctggagaccggcatgaagcgtgccatgttcattggtgtgctcgatattgccggcttcgagatcttcgacttcaacggcttcgagcagatctgtattaacttctgtaacgagaagttgcagcagttcttcaaccaccacatgttcgtgcttgagcaagaggagtacaaggccgagggcattgactgggtctttgtcgacttcggtatggatctgcaggcttgcattgagctcttcgaaaagaaactcggcctcctcgccattctagaagaagagtccatgttccccaaagccaccgacaagtcgtttgaggagaagctgaaggccaaccatctgggcaagtctccctgcttcatcaagcctaagcctccaaaggctggacaggctgaaggtcacttcgccatcgtccactacgccggcactgtgacttacaacctgagtggctggctggagaagaacaaggatcccctcaacgacaccgtcgtggaccagctcaagaagtccaaaatggatctcgttgtggagctcttcgccgatcatcccggccagtctgctcccgctgaggccaagggaggcaaaaagaagaagactggaggtttcaagactgtatcttctggctacagggagcagttgaacagcctcatgacgaccctgcactccactcatccccacttcgtccgttgcattgtgcccaacgagaccaagtcaccaggtgtcgtggaggctggccttatcatgcatcagctgacctgcaatggtgtacttgagggcattcgtatttgccagaagggcttccccaacaggatgcaataccctgacttcaaacaccgttacaagattttggccgctgacgtcatggccacagaaaaggatgacaagaaggcagcagaaatgacattccagaaatctggacttgataaggagttgtataggtgcggtaagacaaaggtattcttccgtgctggcgtcctgggtaccatggaagagcttcgtgatgaacgtttggccaagatcatcacttggatgcagtcatggatccgt

SEQ ID NO: 276 - protein, 747 aa, Litopenaeus vannamei
EGFAEGLIQEAKGDKLVSVQLKSGEVKDFKKDLVVQVNPPKYEKCEDVSNLTFLNDASVLYNLKSRYQAKLIYTYSGLFCIVINPYKRYPIYTNRTVKIYQGKRRNEVPPHLFAISDGAYMDMLQSQQNQSMLITGESGAGKTENTKKVLSYFANVGATTKKKEDEKKQNLEDQIVQTNPPLEAYGNAKTTRNDNSSRFGKFIRIHFAPNGKLSGADIEVYLLEKARVVSQAPAERGYHIFYQMMSDQVDYLKKLCHLSDDIYDYRYECQGKVTVPSIDDKEDMEFTHNAFTILNFTNEERDSCYKVTAAVMHHGNMKFKQRGREEQAEPDGTDAGDIVATIMGVESEELYRNFCKPKIKVGAEFVTQGRNVDQVYYSISAMAKGLFDRLFKWIVKKCNQTLETGMKRAMFIGVLDIAGFEIFDFNGFEQICINFCNEKLQQFFNHHMFVLEQEEYKAEGIDWVFVDFGMDLQACIELFEKKLGLLAILEEESMFPKATDKSFEEKLKANHLGKSPCFIKPKPPKAGQAEGHFAIVHYAGTVTYNLSGWLEKNKDPLNDTVVDQLKKSKMDLVVELFADHPGQSAPAEAKGGKKKKTGGFKTVSSGYREQLNSLMTTLHSTHPHFVRCIVPNETKSPGVVEAGLIMHQLTCNGVLEGIRICQKGFPNRMQYPDFKHRYKILAADVMATEKDDKKAAEMTFQKSGLDKELYRCGKTKVFFRAGVLGTMEELRDERLAKIITWMQSWIR

SEQ ID NO: 277 - protein, 12 aa, Litopenaeus vannamei
EGFAEGLIQEAK

SEQ ID NO: 278 - protein, 10 aa, Litopenaeus vannamei
DLVVQVNPPK

SEQ ID NO: 279 - protein, 13 aa, Litopenaeus vannamei
VLSYFANVGATTK

SEQ ID NO: 280 - protein, 21 aa, Litopenaeus vannamei
QNLEDQIVQTNPPLEAYGNAK

SEQ ID NO: 281 - protein, 11 aa, Litopenaeus vannamei
FIRIHFAPNGK

SEQ ID NO: 282 - protein, 28 aa, Litopenaeus vannamei
ARVVSQAPAERGYHIFYQMMSDQVDYLK

SEQ ID NO: 283 - protein, 13 aa, Litopenaeus vannamei
LSGADIEVYLLEK

SEQ ID NO: 284 - protein, 18 aa, Litopenaeus vannamei
LCHLSDDIYDYRYECQGK

SEQ ID NO: 285 - protein, 14 aa, Litopenaeus vannamei
VTVPSIGLFDRLFK

SEQ ID NO: 286 - protein, 10 aa, Litopenaeus vannamei
CNQTLETGMK

SEQ ID NO: 287 - protein, 18 aa, Litopenaeus vannamei
LQQFFNHHMFVLEQEEYK

SEQ ID NO: 288 - protein, 25 aa, Litopenaeus vannamei
EDMEFTHNAFTILNFTNEERDSCYK

SEQ ID NO: 289 - protein, 15 aa, Litopenaeus vannamei
LGLLAILEEESMFPK

SEQ ID NO: 290 - protein, 12 aa, Litopenaeus vannamei
DPLNDTVVDQLK

SEQ ID NO: 291 - protein, 28 aa, Litopenaeus vannamei
SPGVVEAGLIMHQLTCNGVLEGIRICQK

SEQ ID NO: 292 - protein, 12 aa, Litopenaeus vannamei
GFPNRMQYPDFK

SEQ ID NO: 293 - protein, 11 aa, Litopenaeus vannamei
ILAADVMATEK

SEQ ID NO: 294 - protein, 8 aa, Litopenaeus vannamei
AAEMTFQK

SEQ ID NO: 295 - protein, 21 aa, Litopenaeus vannamei
VFFRAGVLGTMEELRDERLAK

SEQ ID NO: 296 - protein, 10 aa, Litopenaeus vannamei
IITWMQSWIR

SEQ ID NO: 297 - protein, 11 aa, Litopenaeus vannamei
MLITGESGAGK

SEQ ID NO: 298 - protein, 11 aa, Litopenaeus vannamei
TVSSGYREQLN

SEQ ID NO: 299 - DNA, 2241 bp, Penaeus monodon
gagggcttcgctgagggcttgatccagggcgccaagggtgacaaactagtcagcgtccagctgaagagcggtgaggtcaaggacttcaagaaggatcttgtggttcaggtcaaccctcccaagtacgaaaagtgcgaagatgtgtccaacttgaccttcctcaatgatgcttctgtcctgtacaacttgaagagccgttaccaggccaagctcatctacacctactctggcctcttctgtattgtcatcaacccctacaagcgttaccccatctacaccaaccgcaccgtcaagatctaccagggcaagaggcgtaatgaggtgcctccccatctcttcgccatttccgacggcgcctacatggatatgttgcaatctcagcagaaccagtcgatgcttatcaccggcgaatctggtgccggcaagactgagaacacgaagaaggtgctgtcctacttcgccaacgtcggtgccacctccaagaagaaggaagacgagaataagcagaacctggaggaccagatcgtgcagaccaaccctcccctggaggcctacggtaatgccaagactacccgtaatgacaactcctctcgtttcggtaagttcatccgcatccacttcgcccccaacggcaagctctccggtgctgacatcgaggtgtacctgctggagaaggctcgcgtcgtgtcccaggcccctgccgagcgtggctaccatatcttctaccaaatgatgtccgatcaagtagattatctaaagaaactgtgtcatctttcggacgacatctacgactaccgctacgagtgccagggcaaggtcactgtgccttccatcgacgacaaggaagacatggaattcacacataatgctttcaccatcttgaatttcactaacgaagaacgtgacagctgctacaagatcactgccgctgtcatgcaccatggcaacatgaagttcaagcagaggggtcgcgaggagcaggctgagcccgacggcacagatgccggtgatgttattgctgaccttatgggtgttgagactgaggaactgtacaagaatttctgtaagcccaagatcaaggtcggtgccgagttcgtcacccagggtaggaatgtcgaccaggtctactattccgttagtgccatggctaaaggcttgttcgaccgtctctttaagtggattgtgaagaagtgtaaccagaccctcgagaccggcatgaagcgtgccatgttcattggtgtgctcgatattgccggcttcgagatcttcgacttcaacggcttcgagcagatctgcatcaacttctgtaacgagaagttgcagcagttcttcaaccaccacatgttcgtgcttgagcaagaggagtacaaggccgaaggaattgactgggtctttgtcgacttcggtatggatctgcaggcttgcattgagctcttcgaaaagaaacttggccttctcgccatcctagaagaagagtctatgttccccaaagccaccgacaagtcgtttgaggagaagctgaaggccaaccatctgggcaagtctccctgcttcattaagcctaagcctcccaaggctggacagtctgagggtcacttcgccatcgttcactacgccggcactgtgacttacaacctgtctggttggctggagaagaacaaggaccccctcaacgacaccgtcgtcgaccagctcaagaaatccaagttgcctcttgttgtggagctctttgccgatcatcccggccagtctgctccggctgaggccaagggaggcaagaagaagaagactggaggtttcaagactgtatcttctggctatagggagcagttgaacagcctcatgacgaccctgcactccactcaccctcacttcgtccgttgcattgtgcccaacgagaccaagtccccaggtgtcgtggaggctggtctcatcatgcatcagctgacttgcaatggtgtacttgagggtattcgtatttgccagaagggcttccccaacaggatgcaataccctgacttcaaacaccgttacaaaattttggctgctgacgtcatggccacagaaaaggatgacaaaaaggcagcagaaatgacattccagaaagctgggcttgataaggagctgtataggtgcggtaagacaaaggtattcttccgtgctggtgtcctgggtaccatggaagagcttcgtgatgaccgtttggccaagatcatcacttggatgcagtcttggatccgc

SEQ ID NO: 300 - protein, 747 aa, Penaeus monodon
EGFAEGLIQGAKGDKLVSVQLKSGEVKDFKKDLVVQVNPPKYEKCEDVSNLTFLNDASVLYNLKSRYQAKLIYTYSGLFCIVINPYKRYPIYTNRTVKIYQGKRRNEVPPHLFAISDGAYMDMLQSQQNQSMLITGESGAGKTENTKKVLSYFANVGATSKKKEDENKQNLEDQIVQTNPPLEAYGNAKTTRNDNSSRFGKFIRIHFAPNGKLSGADIEVYLLEKARVVSQAPAERGYHIFYQMMSDQVDYLKKLCHLSDDIYDYRYECQGKVTVPSIDDKEDMEFTHNAFTILNFTNEERDSCYKITAAVMHHGNMKFKQRGREEQAEPDGTDAGDVIADLMGVETEELYKNFCKPKIKVGAEFVTQGRNVDQVYYSVSAMAKGLFDRLFKWIVKKCNQTLETGMKRAMFIGVLDIAGFEIFDFNGFEQICINFCNEKLQQFFNHHMFVLEQEEYKAEGIDWVFVDFGMDLQACIELFEKKLGLLAILEEESMFPKATDKSFEEKLKANHLGKSPCFIKPKPPKAGQSEGHFAIVHYAGTVTYNLSGWLEKNKDPLNDTVVDQLKKSKLPLVVELFADHPGQSAPAEAKGGKKKKTGGFKTVSSGYREQLNSLMTTLHSTHPHFVRCIVPNETKSPGVVEAGLIMHQLTCNGVLEGIRICQKGFPNRMQYPDFKHRYKILAADVMATEKDDKKAAEMTFQKAGLDKELYRCGKTKVFFRAGVLGTMEELRDDRLAKIITWMQSWIR

SEQ ID NO: 301 - protein, 13 aa, Penaeus monodon
VLSYFANVGATSK

SEQ ID NO: 302 - protein, 21 aa, Penaeus monodon
QNLEDQIVQTNPPLEAYGNAK

SEQ ID NO: 303 - protein, 12 aa, Penaeus monodon
DPLNDTVVDQLK

SEQ ID NO: 304 - protein, 11 aa, Penaeus monodon
ILAADVMATEK

SEQ ID NO: 305 - DNA, 2241 bp, Marsupenaeus japonicus
gagggcttcgccgagggcttgattcagggcgccaagggtgacaaattcgtcagcgtccagctgaagagtggtgaggtcaaggacttcaagaaggatactgtagttcaggtcaaccctcccaagtatgaaaagtgcgaggatgtgtccaacttgaccttccttaatgacgcctccgtcctgtacaacttgaagacccgttaccaggccaagcttatctacacctactctggtctcttctgtattgtgatcaacccctataagcgttaccccatctacaccaaccgcaccgtgaagatctaccagggcaagaggcgtaatgaggtgcctccccatctcttcgccatctccgacggcgcctacatggacatgttgcagtctgggctgaaccagtctatgcttatcaccggcgagtccggcgcaggcaagaccgagaacacaaagaaggtgctgtcctacttcgccaacgtcggcgctaccagcaagaagaaggaagacgagaaaaagcagaacttggaggaccagatcgtgcagaccaatcctccactggaagcttacggcaatgccaagaccacccgtaatgacaattcctctcgcttcggtaagttcatccgcatccacttcgcccccaacggcaagctgtccggtgctgatatcgaggtgtacctgctggagaaggctcgcgtcgtgtcccaagcccctgccgagcgtggctaccacatcttctatcagatgatgtccgatcaagttcctacccttaagaaaacatgtctcctctcggatgacatttacgattatcgctacgagtgccagggtaaggtcactgtgccctccattgacgacaaggaagacatggaattcacgcacaatgctttcaccatcttgaacttcaccgacgaagagcgtgacagctgctacaagatcactgccgctgtcatgcaccatggtaacatgaagttcaagcagaggggtcgtgaggagcaggctgagcccgacggcacagaggccggcgaaatttgcgctgagctaatgggtgttgatagtgaggagttgtacaagaacttgtgcaagcccaagattaaggtcggcgccgagtttgtcacccagggtaggaatgtcgaccaggtgtactactccgttagcgccatggctaaaggtttgttcgaccgtctgttcaagtggattgtgaagaagtgtaaccagaccctcgagacaggcatgaagcgtgccatgttcatcggtgtgcttgatattgccggcttcgagatcttcgacttcaacggcttcgaacaaatctgtatcaacttctgtaatgagaagttgcagcagttcttcaaccaccacatgttcgtgcttgagcaagaggaatacaaggcagaaggcattgactgggtctttgtcgacttcggtatggatctgcaggcttgcattgagctcttcgagaagaaacttgggctcctcgccatcctcgaggaagagtccatgttccccaaggccactgacaaatccttcgaggagaagctgaaggccaaccatctgggcaaatctccctgcttcatcaagcccaagcctccaaagtctggtcaggctgagggtcacttcgccatcgttcactacgccggcactgtgacttacaacctcagtggctggctggagaagaacaaggatcccctcaacgacactgtcgtcgaccagcttaagaagtctaaattgcctcttattgtggagctcttcgctgaccatcccggacagtctgctcctgctgaggccaagggaggcaaaaagaagaagaccggtggcttcaagactgtatcttctggctacagggagcagctcaacagcctcatgacaaccctgcactccactcaccctcactttgtccgttgtattgtgcccaacgagacaaagtcaccaggtgtcgtggacgctggccttatcatgcatcagctgacctgtaatggtgtacttgagggtatccgtatttgtcagaagggcttccccaacaggatgcaataccctgatttcaaacaccgttacaagattttggctgctgacatcatgacatcagaaaaagatgacaggaaggcagcagaaaagactttcgaaagatctggccttgataaggagctgtataggtgcggtaagacaaaggtattcttccgtgctggtgtcctgggtacaatggaagagcttcgtgacgaacgtttgagcaagatcatcacatggatgcagtcatggatccgt

SEQ ID NO: 306 - protein, 747 aa, Marsupenaeus japonicus
EGFAEGLIQGAKGDKFVSVQLKSGEVKDFKKDTVVQVNPPKYEKCEDVSNLTFLNDASVLYNLKTRYQAKLIYTYSGLFCIVINPYKRYPIYTNRTVKIYQGKRRNEVPPHLFAISDGAYMDMLQSGLNQSMLITGESGAGKTENTKKVLSYFANVGATSKKKEDEKKQNLEDQIVQTNPPLEAYGNAKTTRNDNSSRFGKFIRIHFAPNGKLSGADIEVYLLEKARVVSQAPAERGYHIFYQMMSDQVPTLKKTCLLSDDIYDYRYECQGKVTVPSIDDKEDMEFTHNAFTILNFTDEERDSCYKITAAVMHHGNMKFKQRGREEQAEPDGTEAGEICAELMGVDSEELYKNLCKPKIKVGAEFVTQGRNVDQVYYSVSAMAKGLFDRLFKWIVKKCNQTLETGMKRAMFIGVLDIAGFEIFDFNGFEQICINFCNEKLQQFFNHHMFVLEQEEYKAEGIDWVFVDFGMDLQACIELFEKKLGLLAILEEESMFPKATDKSFEEKLKANHLGKSPCFIKPKPPKSGQAEGHFAIVHYAGTVTYNLSGWLEKNKDPLNDTVVDQLKKSKLPLIVELFADHPGQSAPAEAKGGKKKKTGGFKTVSSGYREQLNSLMTTLHSTHPHFVRCIVPNETKSPGVVDAGLIMHQLTCNGVLEGIRICQKGFPNRMQYPDFKHRYKILAADIMTSEKDDRKAAEKTFERSGLDKELYRCGKTKVFFRAGVLGTMEELRDERLSKIITWMQSWIR

SEQ ID NO: 307 - protein, 13 aa, Marsupenaeus japonicus
DTVVQVNPPKYEK

SEQ ID NO: 308 - protein, 7 aa, Marsupenaeus japonicus
FVSVQLK

SEQ ID NO: 309 - protein, 12 aa, Marsupenaeus japonicus
EGFAEGLIQGAK

SEQ ID NO: 310 - protein, 21 aa, Marsupenaeus japonicus
QNLEDQIVQTNPPLEAYGNAK

SEQ ID NO: 311 - protein, 11 aa, Marsupenaeus japonicus
FIRIHFAPNGK

SEQ ID NO: 312 - protein, 13 aa, Marsupenaeus japonicus
LSGADIEVYLLEK

SEQ ID NO: 313 - protein, 28 aa, Marsupenaeus japonicus
ARVVSQAPAERGYHIFYQMMSDQVPTLK

SEQ ID NO: 314 - protein, 32 aa, Marsupenaeus japonicus
QRGREEQAEPDGTEAGEICAELMGVDSEELYK

SEQ ID NO: 315 - protein, 15 aa, Marsupenaeus japonicus
LGLLAILEEESMFPK

SEQ ID NO: 316 - protein, 12 aa, Marsupenaeus japonicus
DPLNDTVVDQLK

SEQ ID NO: 317 - protein, 28 aa, Marsupenaeus japonicus
SPGVVDAGLIMHQLTCNGVLEGIRICQK

SEQ ID NO: 318 - protein, 12 aa, Marsupenaeus japonicus
GFPNRMQYPDFK

SEQ ID NO: 319 - protein, 11 aa, Marsupenaeus japonicus
ILAADIMTSEK

SEQ ID NO: 320 - protein, 9 aa, Marsupenaeus japonicus
TFERSGLDK

SEQ ID NO: 321 - protein, 9 aa, Litopenaeus vannamei
AAPQTDLEK

SEQ ID NO: 322 - protein, 17 aa, Litopenaeus vannamei
QISVRGIAQVENVGNVK

SEQ ID NO: 323 - protein, 22 aa, Litopenaeus vannamei
IRNGEQVEEPDDWLRYGNPWEK

SEQ ID NO: 324 - protein, 22 aa, Litopenaeus vannamei
ARPEYMIPVNFYGRVEDTPQGK

SEQ ID NO: 325 - protein, 20 aa, Litopenaeus vannamei
WVDTQIVFAMPYDNPIPGYK

SEQ ID NO: 326 - protein, 13 aa, Litopenaeus vannamei
NNVVNTMRLWSAK

SEQ ID NO: 327 - protein, 8 aa, Litopenaeus vannamei
SPNNFNLK

SEQ ID NO: 328 - protein, 9 aa, Litopenaeus vannamei
DFAEMSPEK

SEQ ID NO: 329 - protein, 14 aa, Litopenaeus vannamei
IGEEWVVHLDQLTK

SEQ ID NO: 330 - protein, 12 aa, Litopenaeus vannamei
DAGFIRAVQTAK

SEQ ID NO: 331 - protein, 9 aa, Litopenaeus vannamei
QLEQDYGVK

SEQ ID NO: 332 - protein, 12 aa, Litopenaeus vannamei
VNPSSMFDIQVK

SEQ ID NO: 333 - protein, 17 aa, Litopenaeus vannamei
ANPGAPFVPRTVMIGGK

SEQ ID NO: 334 - protein, 10 aa, Litopenaeus vannamei
AIMNIASSGK

SEQ ID NO: 335 - protein, 23 aa, Litopenaeus vannamei
FSSDRTIAQYGREIWGVEPSWEK

SEQ ID NO: 336 - protein, 18 aa, Litopenaeus vannamei
LPAPHEPRDTDITREEAK

SEQ ID NO: 337 - protein, 9 aa, Penaeus monodon
AAPQTDLEK

SEQ ID NO: 338 - protein, 17 aa, Penaeus monodon
QISVRGIAQVENVGNVK

SEQ ID NO: 339 - protein, 12 aa, Penaeus monodon
TFNRHLHYTLVK

SEQ ID NO: 340 - protein, 22 aa, Penaeus monodon
IRNGEQVEEPDDWLRYGNPWEK

SEQ ID NO: 341 - protein, 22 aa, Penaeus monodon
ARPEYMIPVNFYGRVEDTPQGK

SEQ ID NO: 342 - protein, 20 aa, Penaeus monodon
WVDTQIVFAMPYDNPIPGYK

SEQ ID NO: 343 - protein, 13 aa, Penaeus monodon
NNVVNTMRLWSAK

SEQ ID NO: 344 - protein, 8 aa, Penaeus monodon
SPNNFNLK

SEQ ID NO: 345 - protein, 27 aa, Penaeus monodon
RINMAHLCIVGSHAVNGVAAIHSEIIK

SEQ ID NO: 346 - protein, 9 aa, Penaeus monodon
DFAEMSPEK

SEQ ID NO: 347 - protein, 24 aa, Penaeus monodon
TNGITPRRWLLLCNPALADVIAEK

SEQ ID NO: 348 - protein, 14 aa, Penaeus monodon
IGEEWVVHLDQLTK

SEQ ID NO: 349 - protein, 12 aa, Penaeus monodon
DAGFIRAVQTAK

SEQ ID NO: 350 - protein, 9 aa, Penaeus monodon
QENKLRLAK

SEQ ID NO: 351 - protein, 9 aa, Penaeus monodon
QLEQDYGVK

SEQ ID NO: 352 - protein, 12 aa, Penaeus monodon
VNPSSMFDIQVK

SEQ ID NO: 353 - protein, 17 aa, Penaeus monodon
RQLLNCLHIITMYNRIK

SEQ ID NO: 354 - protein, 17 aa, Penaeus monodon
ANPGAPFVPRTVMIGGK

SEQ ID NO: 355 - protein, 22 aa, Penaeus monodon
QIIRLICAVARVVNNDPIVGDK

SEQ ID NO: 356 - protein, 39 aa, Penaeus monodon
VVYLENYRVTLAEQIIPAADLSEQISTAGTEASGTGNMK

SEQ ID NO: 357 - protein, 25 aa, Penaeus monodon
FMLNGALTIGTLDGANIEMMEEMGK

SEQ ID NO: 358 - protein, 10 aa, Penaeus monodon
AIMNIASSGK

SEQ ID NO: 359 - protein, 23 aa, Penaeus monodon
FSSDRTIAQYGREIWGVEPSWEK

SEQ ID NO: 360 - protein, 18 aa, Penaeus monodon
LPAPHEPRDTDITREEAK

SEQ ID NO: 361 - DNA, 2556 bp, Marsupenaeus japonicus
atggccgccccgcagaccgacttggagaaaaggaagcagatctctgttagagggattgctcaagttgagaatgttggaaacgtaaagaaaaccttcaaccgacatctccattatacgttggtaaaggacaggaacgtggcaactccgcgagattactatttcgctcttgctcacacaatcagagatcatctaacctcaagatggatcagaactcaacaacattactacgagaaggatcccaagcgcgtgtactacctctccctagagtactacatgggccgctcattgaccaacaccatgatcaacttgggcattcagtcggcctgtgatgaagccctctatcaacttggtctagatattgaggaacttgaatctctggaggaggatgcaggcttgggcaatggaggtctcgggcggctggcagcgtgcttcttggattctatggctaccttgggtatggcagcctatggttatggcatccgttatgagtatggtatctttgctcagaagatccgaaacggagagcaggtggaagagcctgatgattggctgcgctatggcaacccatgggagaaggctcgtccagagtacatgatcccagttaacttctatggacgtgtggaggacacaccccagggcaagaaatgggttgatactcagattgtgtttgctatgccttacgacaaccctattcctgggtacaagaacaatgttgtgaatactatgaggctgtggtctgcaaagtcccccaataacttcaatttgaagttcttcaatgatggtgactatatccaggctgtccttgaccgtaactttgctgagaacatctcacgtgtcttgtaccccaatgacaatttctttgagggtaaagagcttcgcttgaagcaagaatatttcatggttgctgccactcttcaagatatcattaggcgcttcaaagcctcaaagttcggctcaaaagaccatgtccgcacgacttttgacacattcccagaaaaggtagcactccagctgaatgacactcatccttccctggccattcctgaactgatgcgcctcttggttgacattgaagggctcccatgggctaaggcatgggatgtttgtgtgaagacctgtgcatacaccaaccacacagtgttgcctgaagctctggagcgctggcccacaagcatgctggaacacattctcccaaggcatctccagattatctatgagatcaaccatttccatctgcaagaagtctcaaagaggtggcctggagacatggaacgcatgaggcgtatgtccctggtggaagaacatggtgaaaagagaatcaacatggctcatctctgcattgtgggttctcatgctgtgaatggtgttgctgccattcactctgagatcatcaagcgagatatcttcaaggactttgctgaaatgagtcctgaaaagttccagaacaagaccaatggtatcactcctcgtcgttggcttctgctttgcaatccagctcttgctgatgtaattgcagagaagattggagaagaatgggttgtgcatcttgatcagctaaccaaactaaaaccccttgctaaggatgctggtttcatccgtgctgtgcaaacagcaaagcaagaaaacaaactgcgtcttgctaaacagctggagcaggattatggtgtgaaggtgaatccctcctccatgtttgacattcaggttaagcgtattcatgagtataagcgtcagttgctaaactgtctgcacattatcactatgtacaatcgcatcaaggccaacccaggagctccatttgtacctcgcacagttatgattggtggtaaagctgcacctggctaccacacagctaagcagataatccgtctcatctgtgctgtagctcgtgtagtgaacaatgatcctattgttggggataaactgaaggttgtgtacttggagaactaccgagttactttggctgaacagatcatcccagctgctgatctctctgaacagatctccacagctggaactgaagcctctggtactggcaacatgaagttcatgcttaatggtgcactgacaattggcactcttgatggtgcaaatattgagatgatggaagagatgggcaaggaaaacatcttcatctttggcatgaatgttgaggaagtagaggagctcaagcgacgtggttacaatgctcatgactattacaatcgcatcccagagttgcgtcagtgtattgaccagatcagcagtggattcttctcccctagcaaccctgaccaattcaaagacttggtcaacatcctcatgcatcatgatcgcttctacctgtttgctgactttgagtcttacattaaatgccaagactctgttaacaagctgtaccaaaagccaaatgattggacccacaaggcaatcatgaacattgcctcatctggcaagttctctagtgacagaaccattgctcagtatggccgtgaaatctggggagttgagccctcatgggagaagttgcctgctccccatgagccacgagatacagatattaccagagaagaagctaag

SEQ ID NO: 362 - protein, 852 aa, Marsupenaeus japonicus
MAAPQTDLEKRKQISVRGIAQVENVGNVKKTFNRHLHYTLVKDRNVATPRDYYFALAHTIRDHLTSRWIRTQQHYYEKDPKRVYYLSLEYYMGRSLTNTMINLGIQSACDEALYQLGLDIEELESLEEDAGLGNGGLGRLAACFLDSMATLGMAAYGYGIRYEYGIFAQKIRNGEQVEEPDDWLRYGNPWEKARPEYMIPVNFYGRVEDTPQGKKWVDTQIVFAMPYDNPIPGYKNNVVNTMRLWSAKSPNNFNLKFFNDGDYIQAVLDRNFAENISRVLYPNDNFFEGKELRLKQEYFMVAATLQDIIRRFKASKFGSKDHVRTTFDTFPEKVALQLNDTHPSLAIPELMRLLVDIEGLPWAKAWDVCVKTCAYTNHTVLPEALERWPTSMLEHILPRHLQIIYEINHFHLQEVSKRWPGDMERMRRMSLVEEHGEKRINMAHLCIVGSHAVNGVAAIHSEIIKRDIFKDFAEMSPEKFQNKTNGITPRRWLLLCNPALADVIAEKIGEEWVVHLDQLTKLKPLAKDAGFIRAVQTAKQENKLRLAKQLEQDYGVKVNPSSMFDIQVKRIHEYKRQLLNCLHIITMYNRIKANPGAPFVPRTVMIGGKAAPGYHTAKQIIRLICAVARVVNNDPIVGDKLKVVYLENYRVTLAEQIIPAADLSEQISTAGTEASGTGNMKFMLNGALTIGTLDGANIEMMEEMGKENIFIFGMNVEEVEELKRRGYNAHDYYNRIPELRQCIDQISSGFFSPSNPDQFKDLVNILMHHDRFYLFADFESYIKCQDSVNKLYQKPNDWTHKAIMNIASSGKFSSDRTIAQYGREIWGVEPSWEKLPAPHEPRDTDITREEAK

SEQ ID NO: 363 - protein, 17 aa, Marsupenaeus japonicus
QISVRGIAQVENVGNVK

SEQ ID NO: 364 - protein, 22 aa, Marsupenaeus japonicus
IRNGEQVEEPDDWLRYGNPWEK

SEQ ID NO: 365 - protein, 22 aa, Marsupenaeus japonicus
ARPEYMIPVNFYGRVEDTPQGK

SEQ ID NO: 366 - protein, 20 aa, Marsupenaeus japonicus
WVDTQIVFAMPYDNPIPGYK

SEQ ID NO: 367 - protein, 13 aa, Marsupenaeus japonicus
NNVVNTMRLWSAK

SEQ ID NO: 368 - protein, 8 aa, Marsupenaeus japonicus
SPNNFNLK

SEQ ID NO: 369 - protein, 13 aa, Marsupenaeus japonicus
DHVRTTFDTFPEK

SEQ ID NO: 370 - protein, 9 aa, Marsupenaeus japonicus
DFAEMSPEK

SEQ ID NO: 371 - protein, 12 aa, Marsupenaeus japonicus
DAGFIRAVQTAK

SEQ ID NO: 372 - protein, 9 aa, Marsupenaeus japonicus
QLEQDYGVK

SEQ ID NO: 373 - protein, 12 aa, Marsupenaeus japonicus
VNPSSMFDIQVK

SEQ ID NO: 374 - protein, 17 aa, Marsupenaeus japonicus
ANPGAPFVPRTVMIGGK

SEQ ID NO: 375 - protein, 17 aa, Marsupenaeus japonicus
ENIFIFGMNVEEVEELK

SEQ ID NO: 376 - protein, 11 aa, Marsupenaeus japonicus
LYQKPNDWTHK

SEQ ID NO: 377 - protein, 10 aa, Marsupenaeus japonicus
AIMNIASSGK

SEQ ID NO: 378 - protein, 23 aa, Marsupenaeus japonicus
FSSDRTIAQYGREIWGVEPSWEK

SEQ ID NO: 379 - protein, 18 aa, Marsupenaeus japonicus
LPAPHEPRDTDITREEAK

SEQ ID NO: 380 - DNA, 2031 bp, Litopenaeus vannamei
atgaaggtcctgctgctcctcgccctcgttgcggctgctgccgcctggccgaactttggcttccagtcggacgcaggaggtgagtctgatgcccagaagcagcatgacgtcaacttcctgcttcataagatctacgggaatattcgtgactctgacctaaaagccaaagctgattcctttgaccccgcggccgatttatcccattacagcgatggaggtgaagctgtacagaaacttgttagagaccttaaggatgacaggcttctccaacagaggcactggttctctctcttcaacccgaggcagcgtcatgaagcactcatgcttttcgatgttctcattcactgcaaggactggaatacatttgtcagcaacgctgcctacttccgtcagcatatgaatgaaggagagtttgtctatgctctgtatgttgcagtcatccactcacctctgactgagcacgttgtacttcctccactctatgaggtcacgcctcacctcttcactaacagcgaagtcattgaatcagcttatcgtgccaagcagacacaaaaacctggtaaatttaagtctagtttcactggaaccaagaagaatcctgaacagagagtagcctatttcggagaggacattggaatgaacactcaccatgttacctggcacatggaattcccattctggtgggacgacaaatatagccatcatctggatcgcaaaggagagaacttcttctgggtacatcatcaacttaccgttcgctttgatgccgaacgtctctccaattacttagatcccgtcgaggaacttagctgggataaacccatcgtacaaggttttgctcctcacaccacttacaagtatggcggtcagttcccctctcgtccagataatgtagacttcgaggatgtggacggtgttgctcgcattcgagacttgcttattatcgagagccgaattcgcgatgctattgcccacggttatattgtcgataaggctggcaatcacattgacatcatgaatgagcgtggaatcgacgtccttggagatgttattgaatcatctttgtatagccctaacgtccagtactatggagctttgcacaatactgctcacattgtacttggtcgacagagtgatcctcatggaaagtacgctttaccccctggtgtactagaacactttgaaactgccacccgtgatcctagcttctttaggctgcataaatacatggataacatcttcaaggaacacaaggacagtctccctccctacacagtggaagaactaacatttgccggtgtaagtgtagacagcgtagcaattgaaggcgaactagagacctacttcgaggacttcgaatacaatcttattaacgccgtcgatgacactgaacagattgcagatgtagacatttctacttatgttcctcgtctcaaccacaaggactttaaaatcaaagttgatattagcaataacaagggcgaggaagttctagctaccgtgcgcattttcgcctggcctcacctcgacaacaatggtatcaagttcacctttgacgaaggccgttggaatgccattgaactggataagttctgggtcaagttgcctggtggaacacaccatatcgagcgtaaatgctcggaatctgctgttactgtgcctgatgtgcctagttttgcaacactctttgagaagaccaaagaagccttaggtggagcagactccggacttaaagatttcgagagtgccactggtattccaaatcgattcctcatccccaagggtaatgaacagggtctggagttcgaccttgttgttgccgtgactgatggcgcagccgacgcagcagtggatggcctccacgaaaacaccgaattcaatcattatggttcccatggcaagtaccctgacaatcgcccacatggctaccctctggatcgcagggttcccgatgaacgtgtattcgaagatcttcccaacttcggccacatccaagttaaggtcttcaatcatggcgagcatatccatcat

SEQ ID NO: 381 - protein, 677 aa, Litopenaeus vannamei
MKVLLLLALVAAAAAWPNFGFQSDAGGESDAQKQHDVNFLLHKIYGNIRDSDLKAKADSFDPAADLSHYSDGGEAVQKLVRDLKDDRLLQQRHWFSLFNPRQRHEALMLFDVLIHCKDWNTFVSNAAYFRQHMNEGEFVYALYVAVIHSPLTEHVVLPPLYEVTPHLFTNSEVIESAYRAKQTQKPGKFKSSFTGTKKNPEQRVAYFGEDIGMNTHHVTWHMEFPFWWDDKYSHHLDRKGENFFWVHHQLTVRFDAERLSNYLDPVEELSWDKPIVQGFAPHTTYKYGGQFPSRPDNVDFEDVDGVARIRDLLIIESRIRDAIAHGYIVDKAGNHIDIMNERGIDVLGDVIESSLYSPNVQYYGALHNTAHIVLGRQSDPHGKYALPPGVLEHFETATRDPSFFRLHKYMDNIFKEHKDSLPPYTVEELTFAGVSVDSVAIEGELETYFEDFEYNLINAVDDTEQIADVDISTYVPRLNHKDFKIKVDISNNKGEEVLATVRIFAWPHLDNNGIKFTFDEGRWNAIELDKFWVKLPGGTHHIERKCSESAVTVPDVPSFATLFEKTKEALGGADSGLKDFESATGIPNRFLIPKGNEQGLEFDLVVAVTDGAADAAVDGLHENTEFNHYGSHGKYPDNRPHGYPLDRRVPDERVFEDLPNFGHIQVKVFNHGEHIHH

SEQ ID NO: 382 - protein, 10 aa, Litopenaeus vannamei
QHDVNFLLHK

SEQ ID NO: 383 - protein, 11 aa, Litopenaeus vannamei
IYGNIRDSDLK

SEQ ID NO: 384 - protein, 22 aa, Litopenaeus vannamei
ADSFDPAADLSHYSDGGEAVQK

SEQ ID NO: 385 - protein, 9 aa, Litopenaeus vannamei
FKSSFTGTK

SEQ ID NO: 386 - protein, 13 aa, Litopenaeus vannamei
PIVQGFAPHTTYK

SEQ ID NO: 387 - protein, 52 aa, Litopenaeus vannamei
AGNHIDIMNERGIDVLGDVIESSLYSPNVQYYGALHNTAHIVLGRQSDPHGK

SEQ ID NO: 388 - protein, 25 aa, Litopenaeus vannamei
YALPPGVLEHFETATRDPSFFRLHK

SEQ ID NO: 389 - protein, 23 aa, Litopenaeus vannamei
AVDDTEQIADVDISTYVPRLNHK

SEQ ID NO: 390 - protein, 22 aa, Litopenaeus vannamei
GEEVLATVRIFAWPHLDNNGIK

SEQ ID NO: 391 - protein, 15 aa, Litopenaeus vannamei
FTFDEGRWNAIELDK

SEQ ID NO: 392 - protein, 11 aa, Litopenaeus vannamei
LPGGTHHIERK

SEQ ID NO: 393 - protein, 20 aa, Litopenaeus vannamei
CSESAVTVPDVPSFATLFEK

SEQ ID NO: 394 - protein, 11 aa, Litopenaeus vannamei
EALGGADSGLK

SEQ ID NO: 395 - protein, 16 aa, Litopenaeus vannamei
DFESATGIPNRFLIPK

SEQ ID NO: 396 - protein, 19 aa, Litopenaeus vannamei
VPDERVFEDLPNFGHIQVK

SEQ ID NO: 397 - protein, 10 aa, Litopenaeus vannamei
VFNHGEHIHH

SEQ ID NO: 398 - DNA, 2034 bp, Penaeus monodon
atgaaggtcttgttgttgttcgctctcgttgcggctgctgccgcctggccgaactttggcttccagtcggacgcggggggtgcggctgatgctcagaagcaacatgacgtaaacttcctgcttcataagatctacggggatatccgtgactctaatctaaaaggcaaagctgattcctttgacccggaagccaatttatcccattacagtgacggaggtaaagcagtacagaaacttatgagagacctgaaggataacaggcttcttcaacaaaggcattggttctctctcttcaatcctaggcaacgcgaagaagcacttatgctttttgatgttctcattcactgcaaggattgggatacatttgtcagcaatgctgcctacttccgccaaattatgaatgagggagaatttgtttatgccttgtatgttgcggtcatccactcacctctgtctgaacacgttgtacttcctccactctatgaagtcacgccacatctcttcaccaacagcgaagtcattgaagcagcttatcgtgccaagcaaacacaaaaacctggtaaatttaagtctagcttcactggaactaagaagaatcctgaacaaagagtagcctatttcggagaggacattggaatgaacactcatcacgtcacctggcatatggaattcccattctggtgggacgacaaatacagccatcatctggatcgcaaaggagagaatttcttctgggtacatcatcaacttaccgttcgttttgatgctgaacgtctctccaattatttggatcccgtcgacgaacttcactgggagaagccaatcgtacaaggttttgctccccacaccacttacaagtatggaggtcagttcccctctcgtccagataatgtagacttcgaggatgtggatggtgttgctcgtattcgagacttgcttattgtagagagccgaatccgcgatgctattgcacatggttatatcgtcgacagggctggtaatcatattgatatcatgaatgagcgtggaattgacgttcttggagatgttattgaatcatctttgtacagccctaatgtgcagtactatggagccttgcacaatactgctcacattgtacttggtcgacagagtgatccacatggaaaatatgatttaccccctggtgtgctggaacactttgaaactgccacccgtgatcctagcttctttaggctgcataaatacatggataacatcttcaaggaacacaaggacagtctccctccatacaccgtggaagaactaacatttgccggtgtaagtgtagacaatgtagcaattgaaggagaactagagaccttcttcgaggatttcgaatacaatctcattaacgctgttgatgacactgaacaaattccagatgtagaaatttctacttacgtgcctcgtctgaaccataaggactttaaaattaagattgatgttagcaataacaagggccaggaagttctagctaccgttcgcattttcgcctggcctcacctagacaataatggtattgaattcaccttcgacgaaggccgttggaatgctattgaactggataagttctgggtcaagttgcctgctggaacacaccatttcgaacgtaaatcctcggaatctgctgtcactgtgcctgatgtgcctagtttcgcaactctcttcgagaagaccaaagaagccttagctggtgcagactccggacttacagatttcgagagtgcaactggtattcctaatcgattccttctccctaagggtaatgaacagggtctggaattcgatcttgttgtagcggtgactgatggcgcagccgatgcagcagtggatggcctccacgaaaataccgaattcaatcactacggttcccatggaaagtaccctgacaatcgcccacatggctaccctctggatcgcaaggttcccgatgaacgtgtattcgaagatctgcccaacttcggtcacatccaagttaaggtcttcaatcatggcgaatatatccaacatgat

SEQ ID NO: 399 - protein, 678 aa, Penaeus monodon
MKVLLLFALVAAAAAWPNFGFQSDAGGAADAQKQHDVNFLLHKIYGDIRDSNLKGKADSFDPEANLSHYSDGGKAVQKLMRDLKDNRLLQQRHWFSLFNPRQREEALMLFDVLIHCKDWDTFVSNAAYFRQIMNEGEFVYALYVAVIHSPLSEHVVLPPLYEVTPHLFTNSEVIEAAYRAKQTQKPGKFKSSFTGTKKNPEQRVAYFGEDIGMNTHHVTWHMEFPFWWDDKYSHHLDRKGENFFWVHHQLTVRFDAERLSNYLDPVDELHWEKPIVQGFAPHTTYKYGGQFPSRPDNVDFEDVDGVARIRDLLIVESRIRDAIAHGYIVDRAGNHIDIMNERGIDVLGDVIESSLYSPNVQYYGALHNTAHIVLGRQSDPHGKYDLPPGVLEHFETATRDPSFFRLHKYMDNIFKEHKDSLPPYTVEELTFAGVSVDNVAIEGELETFFEDFEYNLINAVDDTEQIPDVEISTYVPRLNHKDFKIKIDVSNNKGQEVLATVRIFAWPHLDNNGIEFTFDEGRWNAIELDKFWVKLPAGTHHFERKSSESAVTVPDVPSFATLFEKTKEALAGADSGLTDFESATGIPNRFLLPKGNEQGLEFDLVVAVTDGAADAAVDGLHENTEFNHYGSHGKYPDNRPHGYPLDRKVPDERVFEDLPNFGHIQVKVFNHGEYIQHD

SEQ ID NO: 400 - protein, 10 aa, Penaeus monodon
QHDVNFLLHK

SEQ ID NO: 401 - protein, 11 aa, Penaeus monodon
IYGDIRDSNLK

SEQ ID NO: 402 - protein, 18 aa, Penaeus monodon
ADSFDPEANLSHYSDGGK

SEQ ID NO: 403 - protein, 7 aa, Penaeus monodon
SSFTGTK

SEQ ID NO: 404 - protein, 13 aa, Penaeus monodon
PIVQGFAPHTTYK

SEQ ID NO: 405 - protein, 7 aa, Penaeus monodon
YMDNIFK

SEQ ID NO: 406 - protein, 7 aa, Penaeus monodon
IDVSNNK

SEQ ID NO: 407 - protein, 11 aa, Penaeus monodon
LPAGTHHFERK

SEQ ID NO: 408 - protein, 20 aa, Penaeus monodon
SSESAVTVPDVPSFATLFEK

SEQ ID NO: 409 - protein, 27 aa, Penaeus monodon
EALAGADSGLTDFESATGIPNRFLLPK

SEQ ID NO: 410 - protein, 14 aa, Penaeus monodon
YPDNRPHGYPLDRK

SEQ ID NO: 411 - protein, 19 aa, Penaeus monodon
VPDERVFEDLPNFGHIQVK

SEQ ID NO: 412 - protein, 11 aa, Penaeus monodon
VFNHGEYIQHD

SEQ ID NO: 413 - DNA, 2034 bp, Marsupenaeus japonicus
atgaaggtcttggtgctgttcgctctcgttgcggctgctgccgcctggccgagctttggcttccagtcggacgccggaggagtgtctgacgcccagaagcaacatgacatcaacttcctgctgcacaagatctacggggatatccgtgatgatgccctgaaggccaaggctgattcctttgacccggaggctgatctatcccattacagtgacgacggtgaagcagtgcatacactcatcagagacctcaaggatgacaggcttctccaacagaagcactggttctctctcttcaactccaggcagcgtcatgaagcacttatgctattcgatgtcctcattcattgcaaggactgggatacattcgtcagcaatgctgcctacttccgccaacgtatgaatgagggagagtttgtcaatgccttgtatgttgcggtcatccactcatccttggctgagtatgttgtacttccacctctgtatgaggttacccctcacctctttaccaacagtgaggttatcgaggcagcttatcgtgctaagcagacacaaaagccaggtaaattcaagtcgtcctttactggaactaagaagaaccctgaacaaagagttgcctactttggagaggacattggaatgaacactcaccacgtgacttggcatatggaattcccattctggtggcaggacaaatacagccatcatctggatcgcaaaggagagaacttcttctgggttcatcatcaacttaccgtccgttttgatgccgaacgtctttccaattacttggatcctgtagatgagcttcactgggaaaagcccatcgtacaaggctttgctccccacaccacttacaagtatggaggtcagttcccctctcgtccagataatgcacgattcgaggatgtggacggcgttgcccgaattcgagacttgctcattgttgagagccgaatccgtgatgctattgcccacggttacattgtcgacagggaaggcaaacacattgatatcatgaatgagcgtggtattgacgtccttggagacattatcgaatcgtctttgtacagtcctaatgtccagtactacggggccttgcataatactgctcacattgtgcttggtcgacagagtgatccccatggcaaatacgatttgcccccaggtgtgctagaacacttcgaaactgccacccgtgaccccagtttcttcaggctacataaatatatggataacatcttcaaggaacacaaggacactctccctccttatactgcagaagaactgacatttgctggtgttagtgttgacagtattgcaatcgagggtgcactagaaacgtacttcgaggactttgaatacaatcttattaatgctgttgacgacactgaacaaattccagatgtagaaatctctacatatgtacctcgtctgaatcacaaggactttgctttcaaaattggtgttagcaataacaagggtgaagaaactctggccaccgttcgcattttcgcctggcctcacctcgacaacaatgggattgagttcagcttcgacgagggccgttggcatgctattgaactggataaattctgggttaagttgggcactggagttaccgaaatcactcgcaaatgttcggaatccgcggtgactgttcctgatgtccccagtttcgcaactctctttgagaagaccaaagcagccttgggtggcgccgactccggacttacagatttcgagagtgccactggcattccaaatcgattccttctccccaagggtaacgaaaagggtcttgagttcgaccttgttgtggccgtgaccgatggtgcagctgacgcagcagtggacggacttcacgaaaataccgaattcaaccactatggtgcttatggcaagtaccctgacaaccgcccacatggataccctctggatcgcagcgttccagatgaacgagtattcgaggatcttcctaactttggccacatccaagtaaaggtcttcaatcacggggaacatatccaccatgat

SEQ ID NO: 414 - protein, 678 aa, Marsupenaeus japonicus
MKVLVLFALVAAAAAWPSFGFQSDAGGVSDAQKQHDINFLLHKIYGDIRDDALKAKADSFDPEADLSHYSDDGEAVHTLIRDLKDDRLLQQKHWFSLFNSRQRHEALMLFDVLIHCKDWDTFVSNAAYFRQRMNEGEFVNALYVAVIHSSLAEYVVLPPLYEVTPHLFTNSEVIEAAYRAKQTQKPGKFKSSFTGTKKNPEQRVAYFGEDIGMNTHHVTWHMEFPFWWQDKYSHHLDRKGENFFWVHHQLTVRFDAERLSNYLDPVDELHWEKPIVQGFAPHTTYKYGGQFPSRPDNARFEDVDGVARIRDLLIVESRIRDAIAHGYIVDREGKHIDIMNERGIDVLGDIIESSLYSPNVQYYGALHNTAHIVLGRQSDPHGKYDLPPGVLEHFETATRDPSFFRLHKYMDNIFKEHKDTLPPYTAEELTFAGVSVDSIAIEGALETYFEDFEYNLINAVDDTEQIPDVEISTYVPRLNHKDFAFKIGVSNNKGEETLATVRIFAWPHLDNNGIEFSFDEGRWHAIELDKFWVKLGTGVTEITRKCSESAVTVPDVPSFATLFEKTKAALGGADSGLTDFESATGIPNRFLLPKGNEKGLEFDLVVAVTDGAADAAVDGLHENTEFNHYGAYGKYPDNRPHGYPLDRSVPDERVFEDLPNFGHIQVKVFNHGEHIHHD

SEQ ID NO: 415 - protein, 10 aa, Marsupenaeus japonicus
QHDINFLLHK

SEQ ID NO: 416 - protein, 11 aa, Marsupenaeus japonicus
IYGDIRDDALK

SEQ ID NO: 417 - protein, 7 aa, Marsupenaeus japonicus
YMDNIFK

SEQ ID NO: 418 - protein, 20 aa, Marsupenaeus japonicus
CSESAVTVPDVPSFATLFEK

SEQ ID NO: 419 - protein, 27 aa, Marsupenaeus japonicus
AALGGADSGLTDFESATGIPNRFLLPK

SEQ ID NO: 420 - DNA, 1773 bp, Litopenaeus vannamei
atgtcgaaggtagcacccatgcaacttggggccgcagatacccacacccaggtggaccatatggcggccctggatattgactccaaaccattctcgaagcgactctccggcatcatctgcaccattggacctgtctctcggtctgtagagatgctggagaaaatgatggaggctggcatgaacatcgcacgtatgaacttctcccacggcacccatgaataccacagcgagaccatgatgaatgtccgtaaggcagcccagaagtattccgacaagattgggcattcttatcctgttgccattgctcttgacacaaagggacctgaaattcgtactggccttttggaaggtggaccatcagctgaaattgaattgaaagaaggtgctacaatcaagttgaccacagatgccagttactatgaaaagtgctcagaagacgtgctttacttggactatgtcaacattaccaaagttgtgaagcctggcaaccgcatctttgttgatgatggccttatctctcttattgctaaggacgtgggcagtgattccattgactgtgaggttgaaaatggaggtatgcttgggagcaagaagggagtgaatctcccaggtgttccagtagaccttcctgcagtctctgagaaggaccgtggtgatctcctccttggtgtcaaaatgggagtagacattgtgtttgcatccttcatccgtgatgctgctggagtccgtgagatcagagatgttcttggcgaaaagggcaagaatatcaaaatcatcagcaagattgagaatcaccagggatgcaagaacattgatgacatcattgaagagggagatggtatcatgattgctcgtggtgatttgggtattgagattcctgctgagaaggtcttcgtggcccagaaacagatgattgccaagtgcaacaaagttggaaagccagtcatttgtgctacccagatgttggaatccatggtgaagaagccccgtcccacacgtgctgaagtgtctgatgtgggtaatgctatccttgatggtgctgactgtgtcatgctgtctggtgaaactgctaagggaggctaccctcttgtttgtgtacgaaccatggccaacattgcacgtgaagctgaagctgcaatttggcacaagcaactcttcactgagctgtctcagcaggtccatctgcctactgactcaacacacaccacagctattgctgctgttgaagcttcattcaaagcaatggccacagctattattgttattaccaccactggtcgctctgctcatctggtttcaaagtacaggcctcgctgcccaattgtggctgtaacacgatacccacaggtggccagacagtgccatctctaccgtggcattattcccatccactacactgtgcctcagaatgctgaacgtattgaagactggatgaatgacgtcaatgctcgtgtagactatgctgttcagtatggcaaggagtgtggtttcattaagcccggcgaccctgttgttgtggtgactggctggcagaagggagctggctttaccaataccatgcgcgtcctcgttgtaccttcaactggcccaacagcctccattgtgaaactaggagcacactcatctgttaagtcaggccctgttaagtcaggccctcaagccagtggagagcaccagagaactggaaaggctcagccagatattccatggccgagtttccttgcgcacatgggtccttaccacctatgtgctgcagcagttgctaacaagatt

SEQ ID NO: 421 - protein, 591 aa, Litopenaeus vannamei
MSKVAPMQLGAADTHTQVDHMAALDIDSKPFSKRLSGIICTIGPVSRSVEMLEKMMEAGMNIARMNFSHGTHEYHSETMMNVRKAAQKYSDKIGHSYPVAIALDTKGPEIRTGLLEGGPSAEIELKEGATIKLTTDASYYEKCSEDVLYLDYVNITKVVKPGNRIFVDDGLISLIAKDVGSDSIDCEVENGGMLGSKKGVNLPGVPVDLPAVSEKDRGDLLLGVKMGVDIVFASFIRDAAGVREIRDVLGEKGKNIKIISKIENHQGCKNIDDIIEEGDGIMIARGDLGIEIPAEKVFVAQKQMIAKCNKVGKPVICATQMLESMVKKPRPTRAEVSDVGNAILDGADCVMLSGETAKGGYPLVCVRTMANIAREAEAAIWHKQLFTELSQQVHLPTDSTHTTAIAAVEASFKAMATAIIVITTTGRSAHLVSKYRPRCPIVAVTRYPQVARQCHLYRGIIPIHYTVPQNAERIEDWMNDVNARVDYAVQYGKECGFIKPGDPVVVVTGWQKGAGFTNTMRVLVVPSTGPTASIVKLGAHSSVKSGPVKSGPQASGEHQRTGKAQPDIPWPSFLAHMGPYHLCAAAVANKI

SEQ ID NO: 422 - protein, 26 aa, Litopenaeus vannamei
VAPMQLGAADTHTQVDHMAALDIDSK

SEQ ID NO: 423 - protein, 21 aa, Litopenaeus vannamei
RLSGIICTIGPVSRSVEMLEK

SEQ ID NO: 424 - protein, 14 aa, Litopenaeus vannamei
IGHSYPVAIALDTK

SEQ ID NO: 425 - protein, 20 aa, Litopenaeus vannamei
GPEIRTGLLEGGPSAEIELK

SEQ ID NO: 426 - protein, 10 aa, Litopenaeus vannamei
LTTDASYYEK

SEQ ID NO: 427 - protein, 15 aa, Litopenaeus vannamei
CSEDVLYLDYVNITK

SEQ ID NO: 428 - protein, 17 aa, Litopenaeus vannamei
PGNRIFVDDGLISLIAK

SEQ ID NO: 429 - protein, 20 aa, Litopenaeus vannamei
DVGSDSIDCEVENGGMLGSK

SEQ ID NO: 430 - protein, 17 aa, Litopenaeus vannamei
GVNLPGVPVDLPAVSEK

SEQ ID NO: 431 - protein, 10 aa, Litopenaeus vannamei
DRGDLLLGVK

SEQ ID NO: 432 - protein, 14 aa, Litopenaeus vannamei
PVICATQMLESMVK

SEQ ID NO: 433 - protein, 30 aa, Litopenaeus vannamei
PRPTRAEVSDVGNAILDGADCVMLSGETAK

SEQ ID NO: 434 - protein, 13 aa, Litopenaeus vannamei
PGDPVVVVTGWQK

SEQ ID NO: 435 - protein, 21 aa, Litopenaeus vannamei
AMATAIIVITTTGRSAHLVSK

SEQ ID NO: 436 - protein, 26 aa, Penaeus monodon
VAPMQLGAADTHTQVDHMAALDIDSK

SEQ ID NO: 437 - protein, 21 aa, Penaeus monodon
RLSGIICTIGPVSRSVEMLEK

SEQ ID NO: 438 - protein, 15 aa, Penaeus monodon
CSEDVLYLDYVNITK

SEQ ID NO: 439 - protein, 20 aa, Penaeus monodon
DVGSDSIDCEVENGGMLGSK

SEQ ID NO: 440 - protein, 17 aa, Penaeus monodon
GVNLPGVPVDLPAVSEK

SEQ ID NO: 441 - protein, 17 aa, Penaeus monodon
VGKPVICATQMLESMVK

SEQ ID NO: 442 - protein, 23 aa, Litopenaeus vannamei
VFARTIFDSRGNPTVEVDLYTHK

SEQ ID NO: 443 - protein, 26 aa, Litopenaeus vannamei
GLFRAAVPSGASTGVHEALEMRDGDK

SEQ ID NO: 444 - protein, 15 aa, Litopenaeus vannamei
AVNNVNSIIAPEIIK

SEQ ID NO: 445 - protein, 17 aa, Litopenaeus vannamei
SRLGANAILGVSLAICK

SEQ ID NO: 446 - protein, 24 aa, Litopenaeus vannamei
GRFGLDATAVGDEGGFAPNILNNK

SEQ ID NO: 447 - protein, 12 aa, Litopenaeus vannamei
DALTLIQESIEK

SEQ ID NO: 448 - protein, 14 aa, Litopenaeus vannamei
IEIGMDVAASEFYK

SEQ ID NO: 449 - protein, 10 aa, Litopenaeus vannamei
GENIYDLDFK

SEQ ID NO: 450 - protein, 20 aa, Litopenaeus vannamei
MTSATNIQIVGDDLTVTNPK

SEQ ID NO: 451 - protein, 8 aa, Litopenaeus vannamei
ACNCLLLK

SEQ ID NO: 452 - protein, 18 aa, Litopenaeus vannamei
VNQIGSVTESIDAHLLAK

SEQ ID NO: 453 - protein, 12 aa, Litopenaeus vannamei
TGAPCRSERLAK

SEQ ID NO: 454 - DNA, 1302 bp, Penaeus monodon
atgtctatcaccaaggtttttgcccgtaccatttttgactcccgtggtaaccccactgtggaggttgacctctacacccacaagggcctattccgtgctgctgttccctctggagcatccacaggtgtccatgaggcactggagatgcgtgatggagacaagtcaaagtaccatggcaagtctgtcttcaaggccgtcaacaacgtgaacagcatcattgctcctgaaattattaagagtggactgaaagtcactcagcagaaagagtgtgatgatttcatgtgcaagttggacggcactgaaaacaagagccgccttggtgccaatgccatcttgggtgtctccctggccatttgcaaggctggtgctgctgagcttggcattcccctctacagacacattgctaaccttgccaactactccgatgtgatcctgcctgtgccagccttcaacgtcatcaatggtggttctcacgctggcaacaagctggccatgcaggagttcatgatcctgcccactggtgccaccagcttcactgaggccatgcgcatgggctctgaggtgtaccatcacctcaaggctgtgatcaagggccgctttggtctggatgccactgctgttggtgatgagggtggctttgctcccaacatcctgaataacaaggatgctctcaccctgattcaggaatccattgagaaggctggctacactggcaagattgagattggcatggatgtggctgcttcagagttctacaagggtgagaacatttacgacctggatttcaagactgccaacaacgatggctctcagaagatcactggggaccaacttagggacatgtatatggaattctgcaaagagttccccattgtttctattgaagatcccttcgaccaggacgactgggagaactggaccaagatgacctctgccaccaacatccagattgttggtgatgacttgactgtgaccaaccccaagcgcattgctacagctgttgaaaagaaggcttgcaactgcctcctcctgaaggtcaaccagattggcagtgtgacagagtctattgatgctcaccttctggccaagaagaatggctggggcactatggtttcccataggtctggtgagactgaggactgcttcattgctgatcttgttgttggtctctgcactggccagatcaagactggtgctccctgccgctctgagcgcttggccaagtacaaccagatccttcgcattgaggaggagcttggaggcaatgctaagtttgccggcaagaagttcaggaaaccctgc

SEQ ID NO: 455 - protein, 434 aa, Penaeus monodon
MSITKVFARTIFDSRGNPTVEVDLYTHKGLFRAAVPSGASTGVHEALEMRDGDKSKYHGKSVFKAVNNVNSIIAPEIIKSGLKVTQQKECDDFMCKLDGTENKSRLGANAILGVSLAICKAGAAELGIPLYRHIANLANYSDVILPVPAFNVINGGSHAGNKLAMQEFMILPTGATSFTEAMRMGSEVYHHLKAVIKGRFGLDATAVGDEGGFAPNILNNKDALTLIQESIEKAGYTGKIEIGMDVAASEFYKGENIYDLDFKTANNDGSQKITGDQLRDMYMEFCKEFPIVSIEDPFDQDDWENWTKMTSATNIQIVGDDLTVTNPKRIATAVEKKACNCLLLKVNQIGSVTESIDAHLLAKKNGWGTMVSHRSGETEDCFIADLVVGLCTGQIKTGAPCRSERLAKYNQILRIEEELGGNAKFAGKKFRKPC

SEQ ID NO: 456 - protein, 23 aa, Penaeus monodon
VFARTIFDSRGNPTVEVDLYTHK

SEQ ID NO: 457 - protein, 26 aa, Penaeus monodon
GLFRAAVPSGASTGVHEALEMRDGDK

SEQ ID NO: 458 - protein, 10 aa, Penaeus monodon
SKYHGKSVFK

SEQ ID NO: 459 - protein, 15 aa, Penaeus monodon
AVNNVNSIIAPEIIK

SEQ ID NO: 460 - protein, 9 aa, Penaeus monodon
SGLKVTQQK

SEQ ID NO: 461 - protein, 8 aa, Penaeus monodon
ECDDFMCK

SEQ ID NO: 462 - protein, 7 aa, Penaeus monodon
LDGTENK

SEQ ID NO: 463 - protein, 17 aa, Penaeus monodon
SRLGANAILGVSLAICK

SEQ ID NO: 464 - protein, 42 aa, Penaeus monodon
AGAAELGIPLYRHIANLANYSDVILPVPAFNVINGGSHAGNK

SEQ ID NO: 465 - protein, 35 aa, Penaeus monodon
LAMQEFMILPTGATSFTEAMRMGSEVYHHLKAVIK

SEQ ID NO: 466 - protein, 24 aa, Penaeus monodon
GRFGLDATAVGDEGGFAPNILNNK

SEQ ID NO: 467 - protein, 12 aa, Penaeus monodon
DALTLIQESIEK

SEQ ID NO: 468 - protein, 14 aa, Penaeus monodon
IEIGMDVAASEFYK

SEQ ID NO: 469 - protein, 10 aa, Penaeus monodon
GENIYDLDFK

SEQ ID NO: 470 - protein, 9 aa, Penaeus monodon
TANNDGSQK

SEQ ID NO: 471 - protein, 15 aa, Penaeus monodon
ITGDQLRDMYMEFCK

SEQ ID NO: 472 - protein, 21 aa, Penaeus monodon
EFPIVSIEDPFDQDDWENWTK

SEQ ID NO: 473 - protein, 20 aa, Penaeus monodon
MTSATNIQIVGDDLTVTNPK

SEQ ID NO: 474 - protein, 8 aa, Penaeus monodon
RIATAVEK

SEQ ID NO: 475 - protein, 8 aa, Penaeus monodon
ACNCLLLK

SEQ ID NO: 476 - protein, 18 aa, Penaeus monodon
VNQIGSVTESIDAHLLAK

SEQ ID NO: 477 - protein, 16 aa, Penaeus monodon
YNQILRIEEELGGNAK

SEQ ID NO: 478 - protein, 12 aa, Penaeus monodon
TGAPCRSERLAK

SEQ ID NO: 479 - protein, 10 aa, Penaeus monodon
FAGKKFRKPC

SEQ ID NO: 480 - DNA, 1302 bp, Marsupenaeus japonicus
atgtcgatcaccaaggttttcgctcgtaccatctttgactcccgtggtaaccccactgtggaggtcgacctctacacccacaagggcctcttccgcgctgccgttccctccggagcatccacaggtgtccatgaggccctggagatgcgcgatggagacaagtcaaagtaccatggcaagtctgtcttcaatgccgtcaagaacgtgaacaccatcatcgctcctgaaattattaagagtggactgaaggtcactcagcagaaggagtgtgacgacttcatgcgtaagttggacggcactgagaacaagagccgccttggtgctaatgccatcttgggcgtctccctggccatttgcaaggctggtgctgctgagcttggcattcccctctacagacacattgctaaccttgccaactactctgatgtgatcctgcctgtgccagccttcaatgtcatcaatggtggctctcatgctggcaacaagctggccatgcaggagttcatgatcctgcccactggcgccaccagcttcacagaggccatgcgcatgggctctgaggtctaccatcacctgaaggctgtcatcaagggccgctttggtctggatgccactgccgttggtgatgagggtggctttgctcccaacatccttaacaacaaggatgctctcacactgattcaagaatccattgagaaggatggctacactggcaagattgagatcggcatggacgtggctgcttccgagttctacaagggcgagaacatccacgacttggatttcaagacagccaacaacgatggctctcagaagatcactggggaccaacttagggacttgtacatggaattctgcaacgagttccccattgtctctattgaagatcccttcgaccaggacgactgggagaactggaccaagatgacctctgccaccagcatccagattgttggtgatgacttgactgtgaccaaccccaagcgcattcagacagctgttgaaaagaaggcttgcaactgcctcctcctgaaggtcaaccagattggcagcgtgacggagtctattgatgctcaccttctggccaagaagaatggctggggcactatggtttcccataggtctggtgagactgaggactgcttcattgctgatctcgttgttggtctgtgcaccggccagatcaagactggtgctccctgccgctctgagcgcttggccaagtacaaccagatccttcgcattgaggaggagctcggagccaatgccaagttcgctggcaagaagttcaggcaaccctgc

SEQ ID NO: 481 - protein, 434 aa, Marsupenaeus japonicus
MSITKVFARTIFDSRGNPTVEVDLYTHKGLFRAAVPSGASTGVHEALEMRDGDKSKYHGKSVFNAVKNVNTIIAPEIIKSGLKVTQQKECDDFMRKLDGTENKSRLGANAILGVSLAICKAGAAELGIPLYRHIANLANYSDVILPVPAFNVINGGSHAGNKLAMQEFMILPTGATSFTEAMRMGSEVYHHLKAVIKGRFGLDATAVGDEGGFAPNILNNKDALTLIQESIEKDGYTGKIEIGMDVAASEFYKGENIHDLDFKTANNDGSQKITGDQLRDLYMEFCNEFPIVSIEDPFDQDDWENWTKMTSATSIQIVGDDLTVTNPKRIQTAVEKKACNCLLLKVNQIGSVTESIDAHLLAKKNGWGTMVSHRSGETEDCFIADLVVGLCTGQIKTGAPCRSERLAKYNQILRIEEELGANAKFAGKKFRQPC

SEQ ID NO: 482 - protein, 24 aa, Marsupenaeus japonicus
GRFGLDATAVGDEGGFAPNILNNK

SEQ ID NO: 483 - protein, 20 aa, Marsupenaeus japonicus
MTSATSIQIVGDDLTVTNPK

SEQ ID NO: 484 - protein, 18 aa, Marsupenaeus japonicus
VNQIGSVTESIDAHLLAK

SEQ ID NO: 485 - DNA, 1650 bp, Litopenaeus vannamei
atggctctcgtctccgcacgtcttgcctcttctttggctcgtcaccttcccagggcgactccccaggtcgcaaaggtcctcccagctgcggccattgtgtcccgcaagttcaccaccagcaatgtggtgtcctcggccgaagtgtccaccatccttgaggagcgcatcctgggtgctgcccccaagtccaacctggaagagacaggacgtgtgctgagcattggtgacggtattgcccgtgtctatggcttgaagaacatccaggctgaggagatggtggagttctcctctggacttaagggtatggccctcaacttggagcccgataacgttggtgttgtcgtgttcggtaatgacaagcttatccgtgagggtgatatcgtgaagcgtactggagccattgtggacgtgcctgttggtgaggccatcctgggccgtgttgtggatgctctgggtaaccccattgacggcaagggtcctatcactggtggcctgagggctcgtgtgggtgtgaaggcccctggtatcatccctcgtatctctgtgagggagcccatgcagactggcatcaaggccgtagactctcttgtgcctattggtcgtggccagcgagagttgatcattggtgatcgtcagactggcaagactgccattgccatcgacaccatcatcaaccagaagcgattcaacgatgctgctgaggaaaagaagaaactgtactgtatctacgttgctattggccagaagaggtccactgtggcccagattgtgaagaggctcactgatgctgatgccatgaagtacaccattgtggtgtctgccactgcctctgatgctgctcctctgcagtatttggccccctactctggctgtgccatgggagaattcttccgtgacaatggcaagcacgccctgatcatctatgacgatctgtccaagcaggctgtggcctaccgtcagatgtccctgctgctgcgtcgtcctcccggtcgtgaggcctaccctggtgatgtgttctaccttcactcccgtctccttgagcgtgctgccaagatgaacgacaccaatggaggtggctctctcactgccctgcccgtcatcgagacccaggctggtgatgtgtctgcctacattcctactaacgtgatttccatcactgacggacagatcttcttggagactgagctcttctacaagggtattcgtcctgccatcaacgtcggtctgtctgtatcccgtgtaggatccgctgcccagactaaggccatgaagcaggttgcaggttccatgaagctggaattggcccagtaccgtgaggccgctgcttttgcccagttcggttctgacttggatgcttccacccaacagctgcttaaccgtggtgttcgtcttactgagctcttgaagcagggacagtatgtgcccatggccattgaggaacaggttgccgtcatctactgcggtgtgtgtggccacttggacaagatggacccctccaagatcaccaagttcgagcaggagttcatggccatgctgaagaccagccaccagggactccttgacaacattgccaaggagggacacatcaccccagagagcgatgccaagctgaagcagatcgtcacagacttcctggccaccttccaggcc

SEQ ID NO: 486 - protein, 550 aa, Litopenaeus vannamei
MALVSARLASSLARHLPRATPQVAKVLPAAAIVSRKFTTSNVVSSAEVSTILEERILGAAPKSNLEETGRVLSIGDGIARVYGLKNIQAEEMVEFSSGLKGMALNLEPDNVGVVVFGNDKLIREGDIVKRTGAIVDVPVGEAILGRVVDALGNPIDGKGPITGGLRARVGVKAPGIIPRISVREPMQTGIKAVDSLVPIGRGQRELIIGDRQTGKTAIAIDTIINQKRFNDAAEEKKKLYCIYVAIGQKRSTVAQIVKRLTDADAMKYTIVVSATASDAAPLQYLAPYSGCAMGEFFRDNGKHALIIYDDLSKQAVAYRQMSLLLRRPPGREAYPGDVFYLHSRLLERAAKMNDTNGGGSLTALPVIETQAGDVSAYIPTNVISITDGQIFLETELFYKGIRPAINVGLSVSRVGSAAQTKAMKQVAGSMKLELAQYREAAAFAQFGSDLDASTQQLLNRGVRLTELLKQGQYVPMAIEEQVAVIYCGVCGHLDKMDPSKITKFEQEFMAMLKTSHQGLLDNIAKEGHITPESDAKLKQIVTDFLATFQA

SEQ ID NO: 487 - protein, 15 aa, Litopenaeus vannamei
NIQAEEMVEFSSGLK

SEQ ID NO: 488 - protein, 24 aa, Litopenaeus vannamei
AVDSLVPIGRGQRELIIGDRQTGK

SEQ ID NO: 489 - protein, 12 aa, Litopenaeus vannamei
TAIAIDTIINQK

SEQ ID NO: 490 - protein, 11 aa, Litopenaeus vannamei
HALIIYDDLSK

SEQ ID NO: 491 - protein, 18 aa, Penaeus monodon
SAEVSTILEERILGAAPK

SEQ ID NO: 492 - protein, 23 aa, Penaeus monodon
SNLEETGRVLSIGDGIARVYGLK

SEQ ID NO: 493 - protein, 15 aa, Penaeus monodon
NIQAEEMVEFSSGLK

SEQ ID NO: 494 - protein, 20 aa, Penaeus monodon
GMALNLEPDNVGVVVFGNDK

SEQ ID NO: 495 - protein, 24 aa, Penaeus monodon
AVDSLVPIGRGQRELIIGDRQTGK

SEQ ID NO: 496 - protein, 12 aa, Penaeus monodon
TAIAIDTIINQK

SEQ ID NO: 497 - protein, 11 aa, Penaeus monodon
HALIIYDDLSK

SEQ ID NO: 498 - protein, 18 aa, Marsupenaeus japonicus
SAEVSTILEERILGAAPK

SEQ ID NO: 499 - protein, 23 aa, Marsupenaeus japonicus
SNLEETGRVLSIGDGIARVYGLK

SEQ ID NO: 500 - protein, 15 aa, Marsupenaeus japonicus
NIQAEEMVEFSSGLK

SEQ ID NO: 501 - protein, 20 aa, Marsupenaeus japonicus
GMALNLEPDNVGVVVFGNDK

SEQ ID NO: 502 - protein, 9 aa, Marsupenaeus japonicus
LIREGDIVK

SEQ ID NO: 503 - protein, 29 aa, Marsupenaeus japonicus
RTGAIVDVPVGEAILGRVVDALGNPIDGK

SEQ ID NO: 504 - protein, 14 aa, Marsupenaeus japonicus
GPITGGLRARVGVK

SEQ ID NO: 505 - protein, 19 aa, Marsupenaeus japonicus
APGIIPRISVREPMQTGIK

SEQ ID NO: 506 - protein, 24 aa, Marsupenaeus japonicus
AVDSLVPIGRGQRELIIGDRQTGK

SEQ ID NO: 507 - protein, 12 aa, Marsupenaeus japonicus
TAIAIDTIINQK

SEQ ID NO: 508 - protein, 9 aa, Marsupenaeus japonicus
RFNDAAEEK

SEQ ID NO: 509 - protein, 11 aa, Marsupenaeus japonicus
LYCIYVAIGQK

SEQ ID NO: 510 - protein, 9 aa, Marsupenaeus japonicus
RSTVAQIVK

SEQ ID NO: 511 - protein, 9 aa, Marsupenaeus japonicus
RLTDADAMK

SEQ ID NO: 512 - protein, 11 aa, Marsupenaeus japonicus
HALIIYDDLSK

SEQ ID NO: 513 - protein, 22 aa, Marsupenaeus japonicus
GIRPAINVGLSVSRVGSAAQTK

SEQ ID NO: 514 - protein, 13 aa, Marsupenaeus japonicus
ITKFEQEFMAMLK

SEQ ID NO: 515 - protein, 10 aa, Marsupenaeus japonicus
FEQEFMAMLK

SEQ ID NO: 516 - protein, 12 aa, Marsupenaeus japonicus
TSHQGLLDNIAK

SEQ ID NO: 517 - protein, 11 aa, Marsupenaeus japonicus
EGHITPESDAK

SEQ ID NO: 518 - protein, 12 aa, Marsupenaeus japonicus
QIVTDFLATFQA

SEQ ID NO: 519 - DNA, 630 bp, Litopenaeus vannamei
atggcggacgaggaagcaaagaagaagcaggaggagatcgaccgcaagaaggcggaggtccgcaagcgcctcgaggagcagagcgccaagaagcagaagaagggtttcatgacccctgagcgtaagaagaagctcaggttgttgctccgtaagaaggccgctgaggaactgaagaaggaacaggagaggaaggccgctgagaggcgcaggatcattgatgagcgttgtggcaaggccaagaacctcgatggtgcaaacgaagacgcccttcgcgcaatttgtaaagaataccacgatcacatcgccagcattgagagcggcaagtatgatcttgagatggaaatcatgaggaaggactatgagatcaacgagctgaacattcaggtcaacgatctgcgtggcaagttcatcaaacctaccctgaagaaggtgtccaagtacgagaacaaattcgccaagctgcagaagaaggccgctgagttcaacttcaggaatcagctgaagactgtcaagaagaaggagttcgagctcgaggatgacaagggtgcgacaaagcctgactgggcggcgggcggaccaggagccgctaagaaggcggagggtgatgctcctgcagaggaagccgctgcg

SEQ ID NO: 520 - protein, 210 aa, Litopenaeus vannamei
MADEEAKKKQEEIDRKKAEVRKRLEEQSAKKQKKGFMTPERKKKLRLLLRKKAAEELKKEQERKAAERRRIIDERCGKAKNLDGANEDALRAICKEYHDHIASIESGKYDLEMEIMRKDYEINELNIQVNDLRGKFIKPTLKKVSKYENKFAKLQKKAAEFNFRNQLKTVKKKEFELEDDKGATKPDWAAGGPGAAKKAEGDAPAEEAAA

SEQ ID NO: 521 - protein, 15 aa, Litopenaeus vannamei
NLDGANEDALRAICK

SEQ ID NO: 522 - protein, 13 aa, Litopenaeus vannamei
EYHDHIASIESGK

SEQ ID NO: 523 - protein, 10 aa, Litopenaeus vannamei
YDLEMEIMRK

SEQ ID NO: 524 - protein, 17 aa, Litopenaeus vannamei
DYEINELNIQVNDLRGK

SEQ ID NO: 525 - protein, 11 aa, Litopenaeus vannamei
AAEFNFRNQLK

SEQ ID NO: 526 - protein, 8 aa, Litopenaeus vannamei
EFELEDDK

SEQ ID NO: 527 - protein, 12 aa, Litopenaeus vannamei
PDWAAGGPGAAK

SEQ ID NO: 528 - protein, 15 aa, Penaeus monodon
NLDGANEDALRAICK

SEQ ID NO: 529 - protein, 17 aa, Penaeus monodon
DYEINELNIQVNDLRGK

SEQ ID NO: 530 - protein, 11 aa, Penaeus monodon
AAEFNFRNQLK

SEQ ID NO: 531 - protein, 8 aa, Penaeus monodon
EFELEDDK

SEQ ID NO: 532 - protein, 12 aa, Penaeus monodon
PDWAAGGPGAAK

SEQ ID NO: 533 - protein, 15 aa, Marsupenaeus japonicus
NLDGANEDALRAICK

SEQ ID NO: 534 - protein, 13 aa, Marsupenaeus japonicus
EYHDHIASIESGK

SEQ ID NO: 535 - protein, 10 aa, Marsupenaeus japonicus
YDLEMEIMRK

SEQ ID NO: 536 - protein, 17 aa, Marsupenaeus japonicus
DYEINELNIQVNDLRGK

SEQ ID NO: 537 - protein, 11 aa, Marsupenaeus japonicus
AAEFNFRNQLK

SEQ ID NO: 538 - protein, 8 aa, Marsupenaeus japonicus
EFELEDDK

SEQ ID NO: 539 - protein, 12 aa, Marsupenaeus japonicus
PDWAAGGPGAAK

SEQ ID NO: 540 - DNA, 492 bp, Litopenaeus vannamei
atgggcaatcccaaagtctttttcgacattgccgctgacaaccagcccgttggcaggatcgtcatggagctccgcgccgacgtggtccccaagacggccgagaacttccggtcgctgtgcacgggcgagaagggcttcggctacaagggctcgtgcttccaccgcgtgatccccaacttcatgtgccagggcggcgacttcaccgccggcaacggcacgggcggcaagtccatctacggcaacaaattcgaggacgagaacttcgctctgaagcacaccggccccggcatcctgtccatggccaacgccggccccaacaccaacgggtcgcagttcttcatctgcaccgtcaaaacctcctggctggacaacaagcacgtggtcttcggcaccgtggtggagggcatggacgtcgtgcgccaggtcgagggcttcggcacgcccaacggctcgtgcaagcggaaagtggtgatcgccaactgcggccagctg

SEQ ID NO: 541 - protein, 164 aa, Litopenaeus vannamei
MGNPKVFFDIAADNQPVGRIVMELRADVVPKTAENFRSLCTGEKGFGYKGSCFHRVIPNFMCQGGDFTAGNGTGGKSIYGNKFEDENFALKHTGPGILSMANAGPNTNGSQFFICTVKTSWLDNKHVVFGTVVEGMDVVRQVEGFGTPNGSCKRKVVIANCGQL

SEQ ID NO: 542 - protein, 13 aa, Litopenaeus vannamei
TAENFRSLCTGEK

SEQ ID NO: 543 - protein, 27 aa, Litopenaeus vannamei
GSCFHRVIPNFMCQGGDFTAGNGTGGK

SEQ ID NO: 544 - protein, 9 aa, Litopenaeus vannamei
FEDENFALK

SEQ ID NO: 545 - protein, 27 aa, Litopenaeus vannamei
HTGPGILSMANAGPNTNGSQFFICTVK

SEQ ID NO: 546 - protein, 28 aa, Litopenaeus vannamei
HVVFGTVVEGMDVVRQVEGFGTPNGSCK

SEQ ID NO: 547 - protein, 9 aa, Litopenaeus vannamei
VVIANCGQL

SEQ ID NO: 548 - DNA, 492 bp, Penaeus monodon
atgggcaaccccaaagtctttttcgacattaccgctgacaaccagcccgttggcaggatcatcatggagctccgcgccgacgtggtccccaagaccgccgagaacttccggtcgctgtgcacgggcgagaagggcttcggctacaagggctcctgcttccaccgcgtgatccccaacttcatgtgtcagggaggcgacttcaccgccggcaacggcacgggcggcaagtccatctacggcaacaaattcgaggacgagaacttcgcactgaagcacaccggccccggcaccctgtccatggccaacgccggccccaacaccaacgggtcgcaattcttcatctgcaccgtcaaaaccccctggctggacaacaagcacgtggtcttcggctccgtggtggagggcatggacatcgtgcgccaggtcgagggcttcggcacgcccaacggctcttgcaagcggaaagtgatgatcgccaactgcggccagctg

SEQ ID NO: 549 - protein, 164 aa, Penaeus monodon
MGNPKVFFDITADNQPVGRIIMELRADVVPKTAENFRSLCTGEKGFGYKGSCFHRVIPNFMCQGGDFTAGNGTGGKSIYGNKFEDENFALKHTGPGTLSMANAGPNTNGSQFFICTVKTPWLDNKHVVFGSVVEGMDIVRQVEGFGTPNGSCKRKVMIANCGQL

SEQ ID NO: 550 - protein, 13 aa, Penaeus monodon
TAENFRSLCTGEK

SEQ ID NO: 551 - protein, 27 aa, Penaeus monodon
GSCFHRVIPNFMCQGGDFTAGNGTGGK

SEQ ID NO: 552 - protein, 27 aa, Penaeus monodon
HTGPGTLSMANAGPNTNGSQFFICTVK

SEQ ID NO: 553 - protein, 28 aa, Penaeus monodon
HVVFGSVVEGMDIVRQVEGFGTPNGSCK

SEQ ID NO: 554 - protein, 13 aa, Marsupenaeus japonicus
TAENFRSLCTGEK

SEQ ID NO: 555 - protein, 15 aa, Marsupenaeus japonicus
SIYGNKFEDENFALK

SEQ ID NO: 556 - protein, 27 aa, Marsupenaeus japonicus
HTGPGILSMANAGPNTNGSQFFICTVK

SEQ ID NO: 557 - protein, 9 aa, Marsupenaeus japonicus
FEDENFALK

SEQ ID NO: 558 - protein, 15 aa, Artificial Sequence
  epitope
ADIEVYLLEKARVIS

SEQ ID NO: 559 - protein, 9 aa, Artificial Sequence
  epitope
LLEKARVIS

SEQ ID NO: 560 - protein, 9 aa, Artificial Sequence
  epitope
  misc_feature (2)..(2): Xaa can be any amino acid
  misc_feature (6)..(9): Xaa can be any amino acid
LXEKAXXXX

SEQ ID NO: 561 - protein, 8 aa, Artificial Sequence
  epitope
KARVISPE

SEQ ID NO: 562 - protein, 6 aa, Artificial Sequence
  epitope
  misc_feature (4)..(4): Xaa can be any amino acid
KARXIS

SEQ ID NO: 563 - protein, 10 aa, Artificial Sequence
  epitope
EVYLLEKARV

SEQ ID NO: 564 - protein, 10 aa, Artificial Sequence
  epitope
  misc_feature (1)..(2): Xaa can be any amino acid
  misc_feature (4)..(5): Xaa can be any amino acid
  misc_feature (7)..(8): Xaa can be any amino acid
XXYXXEXXRV

SEQ ID NO: 565 - protein, 6 aa, Artificial Sequence
  epitope
  misc_feature (4)..(5): Xaa can be any amino acid
KARXXS

SEQ ID NO: 566 - protein, 15 aa, Artificial Sequence
  epitope
ARVISQSPAERGYHI

SEQ ID NO: 567 - protein, 10 aa, Artificial Sequence
  epitope
VISQSPAERG

SEQ ID NO: 568 - protein, 10 aa, Artificial Sequence
  epitope
  misc_feature (1)..(3): Xaa can be any amino acid
  misc_feature (5)..(6): Xaa can be any amino acid
  misc_feature (10)..(10): Xaa can be any amino acid
XXXQXXAERX

SEQ ID NO: 569 - protein, 9 aa, Artificial Sequence
  epitope
SPAERGYHI

SEQ ID NO: 570 - protein, 9 aa, Artificial Sequence
  epitope
  misc_feature (1)..(2): Xaa can be any amino acid
  misc_feature (6)..(6): Xaa can be any amino acid
XXAERXYHI

SEQ ID NO: 571 - protein, 8 aa, Artificial Sequence
  epitope
ARVISQSP

SEQ ID NO: 572 - protein, 8 aa, Artificial Sequence
  epitope
  misc_feature (1)..(1): Xaa can be any amino acid
  misc_feature (3)..(3): Xaa can be any amino acid
  misc_feature (5)..(5): Xaa can be any amino acid
  misc_feature (7)..(7): Xaa can be any amino acid
XRXIXQXP

SEQ ID NO: 573 - protein, 6 aa, Artificial Sequence
  epitope
PAERGY

SEQ ID NO: 574 - protein, 5 aa, Artificial Sequence
  epitope
  misc_feature (2)..(2): Xaa can be any amino acid
PXERG

SEQ ID NO: 575 - protein, 4 aa, Artificial Sequence
  epitope
AERG

SEQ ID NO: 576 - protein, 10 aa, Artificial Sequence
  epitope
ARVISQSPAE

SEQ ID NO: 577 - protein, 10 aa, Artificial Sequence
  epitope
  misc_feature (3)..(6): Xaa can be any amino acid
  misc_feature (8)..(8): Xaa can be any amino acid
ARXXXXSXAE

SEQ ID NO: 578 - protein, 8 aa, Artificial Sequence
  epitope
SQSPAERG

SEQ ID NO: 579 - protein, 8 aa, Artificial Sequence
  epitope
  misc_feature (1)..(2): Xaa can be any amino acid
  misc_feature (4)..(4): Xaa can be any amino acid
  misc_feature (8)..(8): Xaa can be any amino acid
XXSXAERX

SEQ ID NO: 580 - protein, 6 aa, Artificial Sequence
  epitope
SPAERG

SEQ ID NO: 581 - protein, 6 aa, Artificial Sequence
  epitope
  misc_feature (5)..(6): Xaa can be any amino acid
SPAEXX

SEQ ID NO: 582 - protein, 15 aa, Artificial Sequence
  epitope
GYKDQLANLMKTLNA

SEQ ID NO: 583 - protein, 10 aa, Artificial Sequence
  epitope
LANLMKTLNA

SEQ ID NO: 584 - protein, 10 aa, Artificial Sequence
  epitope
  misc_feature (4)..(8): Xaa can be any amino acid
LANXXXXXNA

SEQ ID NO: 585 - protein, 4 aa, Artificial Sequence
  epitope
KDQL

SEQ ID NO: 586 - protein, 15 aa, Artificial Sequence
  epitope
HGELEESRTLLEQSD

SEQ ID NO: 587 - protein, 4 aa, Artificial Sequence
  epitope
ELEE

SEQ ID NO: 588 - protein, 10 aa, Artificial Sequence
  epitope
HGELEESRTL

SEQ ID NO: 589 - protein, 10 aa, Artificial Sequence
  epitope
  misc_feature (2)..(2): Xaa can be any amino acid
  misc_feature (4)..(6): Xaa can be any amino acid
  misc_feature (8)..(9): Xaa can be any amino acid
HXEXXXSXXL

SEQ ID NO: 590 - protein, 10 aa, Artificial Sequence
  epitope
  misc_feature (2)..(2): Xaa can be any amino acid
  misc_feature (4)..(7): Xaa can be any amino acid
  misc_feature (10)..(10): Xaa can be any amino acid
HXEXXXXRTX

SEQ ID NO: 591 - protein, 10 aa, Artificial Sequence
  epitope
ELEESRTLLE

SEQ ID NO: 592 - protein, 10 aa, Artificial Sequence
  epitope
  misc_feature (4)..(5): Xaa can be any amino acid
  misc_feature (8)..(10): Xaa can be any amino acid
ELEXXRTXXX

SEQ ID NO: 593 - protein, 6 aa, Artificial Sequence
  epitope
TLLEPE

SEQ ID NO: 594 - protein, 15 aa, Artificial Sequence
  epitope
GTMEELRDERLAKII

SEQ ID NO: 595 - protein, 4 aa, Artificial Sequence
  epitope
MEEL

SEQ ID NO: 596 - protein, 5 aa, Artificial Sequence
  epitope
RLAKI

SEQ ID NO: 597 - protein, 7 aa, Artificial Sequence
  epitope
RDERLAK

SEQ ID NO: 598 - protein, 7 aa, Artificial Sequence
  epitope
  misc_feature (3)..(3): Xaa can be any amino acid
  misc_feature (5)..(6): Xaa can be any amino acid
RDXRXXK

SEQ ID NO: 599 - protein, 15 aa, Artificial Sequence
  epitope
KDHQIRNINDEISHQ

SEQ ID NO: 600 - protein, 8 aa, Artificial Sequence
  epitope
KDHQIRNI

SEQ ID NO: 601 - protein, 8 aa, Artificial Sequence
  epitope
  misc_feature (4)..(4): Xaa can be any amino acid
  misc_feature (6)..(8): Xaa can be any amino acid
KDHXIXXX

SEQ ID NO: 602 - protein, 4 aa, Artificial Sequence
  epitope
HQIR

SEQ ID NO: 603 - protein, 8 aa, Artificial Sequence
  epitope
  misc_feature (2)..(5): Xaa can be any amino acid
KXXXXRNI

SEQ ID NO: 604 - protein, 10 aa, Artificial Sequence
  epitope
IRNINDEISH

SEQ ID NO: 605 - protein, 10 aa, Artificial Sequence
  epitope
  misc_feature (1)..(2): Xaa can be any amino acid
  misc_feature (6)..(9): Xaa can be any amino acid
XXNINXXXXH

SEQ ID NO: 606 - protein, 10 aa, Artificial Sequence
  epitope
DHQIRNINDE

SEQ ID NO: 607 - protein, 10 aa, Artificial Sequence
  epitope
  misc_feature (2)..(5): Xaa can be any amino acid
  misc_feature (9)..(9): Xaa can be any amino acid
DXXXXNINXE

SEQ ID NO: 608 - protein, 10 aa, Artificial Sequence
  epitope
QIRNINDEIS

SEQ ID NO: 609 - protein, 10 aa, Artificial Sequence
  epitope
  misc_feature (1)..(3): Xaa can be any amino acid
  misc_feature (7)..(7): Xaa can be any amino acid
  misc_feature (10)..(10): Xaa can be any amino acid
XXXNINXEIX

SEQ ID NO: 610 - protein, 8 aa, Artificial Sequence
  epitope
  misc_feature (2)..(5): Xaa can be any amino acid
KXXXXRNI

SEQ ID NO: 611 - protein, 6 aa, Artificial Sequence
  epitope
  misc_feature (4)..(4): Xaa can be any amino acid
KDHXIR

SEQ ID NO: 612 - protein, 9 aa, Artificial Sequence
  epitope
DHQIRNIND

SEQ ID NO: 613 - protein, 9 aa, Artificial Sequence
  epitope
  misc_feature (1)..(3): Xaa can be any amino acid
  misc_feature (8)..(9): Xaa can be any amino acid
XXXIRNIXX

SEQ ID NO: 614 - protein, 15 aa, Artificial Sequence
  epitope
AKSAMDSLARDKALA

SEQ ID NO: 615 - protein, 10 aa, Artificial Sequence
  epitope
AKSAMDSLAR

SEQ ID NO: 616 - protein, 10 aa, Artificial Sequence
  epitope
  misc_feature (1)..(1): Xaa can be any amino acid
  misc_feature (3)..(6): Xaa can be any amino acid
  misc_feature (8)..(8): Xaa can be any amino acid
XKXXXXSXAR

SEQ ID NO: 617 - protein, 10 aa, Artificial Sequence
  epitope
DSLARDKALA

SEQ ID NO: 618 - protein, 10 aa, Artificial Sequence
  epitope
  misc_feature (1)..(3): Xaa can be any amino acid
  misc_feature (8)..(10): Xaa can be any amino acid
XXXARDKXXX

SEQ ID NO: 619 - protein, 10 aa, Artificial Sequence
  epitope
KSAMDSLARD

SEQ ID NO: 620 - protein, 10 aa, Artificial Sequence
  epitope
  misc_feature (1)..(3): Xaa can be any amino acid
  misc_feature (8)..(9): Xaa can be any amino acid
XXXMDSLXXD

SEQ ID NO: 621 - protein, 9 aa, Artificial Sequence
  epitope
AKSAMDSLA

SEQ ID NO: 622 - protein, 9 aa, Artificial Sequence
  epitope
  misc_feature (3)..(3): Xaa can be any amino acid
  misc_feature (8)..(9): Xaa can be any amino acid
AKXAMDSXX

SEQ ID NO: 623 - protein, 4 aa, Artificial Sequence
  epitope
RDKA

SEQ ID NO: 624 - protein, 15 aa, Artificial Sequence
  epitope
LEEADNQINQLNNLK

SEQ ID NO: 625 - protein, 4 aa, Artificial Sequence
  epitope
NQLN

SEQ ID NO: 626 - protein, 7 aa, Artificial Sequence
  epitope
DNQINQL

SEQ ID NO: 627 - protein, 7 aa, Artificial Sequence
  epitope
  misc_feature (2)..(2): Xaa can be any amino acid
  misc_feature (4)..(4): Xaa can be any amino acid
  misc_feature (7)..(7): Xaa can be any amino acid
DXQXNQX

SEQ ID NO: 628 - protein, 10 aa, Artificial Sequence
  epitope
LEEADNQINQ

SEQ ID NO: 629 - protein, 10 aa, Artificial Sequence
  epitope
  misc_feature (3)..(4): Xaa can be any amino acid
  misc_feature (6)..(8): Xaa can be any amino acid
  misc_feature (10)..(10): Xaa can be any amino acid
LEXXDXXXNX

SEQ ID NO: 630 - protein, 9 aa, Artificial Sequence
  epitope
NQINQLNNL

SEQ ID NO: 631 - protein, 9 aa, Artificial Sequence
  epitope
  misc_feature (1)..(3): Xaa can be any amino acid
  misc_feature (5)..(5): Xaa can be any amino acid
  misc_feature (7)..(7): Xaa can be any amino acid
  misc_feature (9)..(9): Xaa can be any amino acid
XXXNXLXNX

SEQ ID NO: 632 - protein, 6 aa, Artificial Sequence
  epitope
NQLNNL

SEQ ID NO: 633 - protein, 6 aa, Artificial Sequence
  epitope
  misc_feature (6)..(6): Xaa can be any amino acid
NQLNNX

SEQ ID NO: 634 - protein, 15 aa, Artificial Sequence
  epitope
DQLATELDASQKECR

SEQ ID NO: 635 - protein, 5 aa, Artificial Sequence
  epitope
QLATE

SEQ ID NO: 636 - protein, 4 aa, Artificial Sequence
  epitope
SQKE

SEQ ID NO: 637 - protein, 10 aa, Artificial Sequence
  epitope
QLATELDASQ

SEQ ID NO: 638 - protein, 10 aa, Artificial Sequence
  epitope
  misc_feature (3)..(5): Xaa can be any amino acid
  misc_feature (7)..(7): Xaa can be any amino acid
  misc_feature (9)..(10): Xaa can be any amino acid
QLXXXLXAXX

SEQ ID NO: 639 - protein, 5 aa, Artificial Sequence
  epitope
ATELD

SEQ ID NO: 640 - protein, 15 aa, Artificial Sequence
  epitope
HFRIKAVYEENLEHL

SEQ ID NO: 641 - protein, 7 aa, Artificial Sequence
  epitope
IKAVYEE

SEQ ID NO: 642 - protein, 7 aa, Artificial Sequence
  epitope
  misc_feature (1)..(1): Xaa can be any amino acid
  misc_feature (3)..(3): Xaa can be any amino acid
  misc_feature (5)..(5): Xaa can be any amino acid
XKXVXEE

SEQ ID NO: 643 - protein, 10 aa, Artificial Sequence
  epitope
AVYEENLEHL

SEQ ID NO: 644 - protein, 10 aa, Artificial Sequence
  epitope
  misc_feature (1)..(1): Xaa can be any amino acid
  misc_feature (3)..(4): Xaa can be any amino acid
  misc_feature (6)..(6): Xaa can be any amino acid
  misc_feature (9)..(10): Xaa can be any amino acid
XVXXEXLEXX

SEQ ID NO: 645 - protein, 5 aa, Artificial Sequence
  epitope
EENLE

SEQ ID NO: 646 - protein, 5 aa, Artificial Sequence
  epitope
KAVYE

SEQ ID NO: 647 - protein, 5 aa, Artificial Sequence
  epitope
YEENL

SEQ ID NO: 648 - protein, 5 aa, Artificial Sequence
  epitope
  misc_feature (1)..(1): Xaa can be any amino acid
XEENL

SEQ ID NO: 649 - protein, 5 aa, Artificial Sequence
  epitope
KAVYE

SEQ ID NO: 650 - protein, 5 aa, Artificial Sequence
  epitope
  misc_feature (2)..(2): Xaa can be any amino acid
KXVYE

SEQ ID NO: 651 - protein, 6 aa, Artificial Sequence
  epitope
IKAVYE

SEQ ID NO: 652 - protein, 6 aa, Artificial Sequence
  epitope
  misc_feature (5)..(5): Xaa can be any amino acid
IKAVXE

SEQ ID NO: 653 - protein, 4 aa, Artificial Sequence
  epitope
AVYE

SEQ ID NO: 654 - protein, 15 aa, Artificial Sequence
  epitope
RSLHEIEKNAKRFEI

SEQ ID NO: 655 - protein, 4 aa, Artificial Sequence
  epitope
KNAK

SEQ ID NO: 656 - protein, 8 aa, Artificial Sequence
  epitope
HEIEKNAK

SEQ ID NO: 657 - protein, 8 aa, Artificial Sequence
  epitope
  misc_feature (1)..(4): Xaa can be any amino acid
XXXXKNAK

SEQ ID NO: 658 - protein, 7 aa, Artificial Sequence
  epitope
NAKRFEI

SEQ ID NO: 659 - protein, 7 aa, Artificial Sequence
  epitope
  misc_feature (1)..(1): Xaa can be any amino acid
  misc_feature (5)..(5): Xaa can be any amino acid
  misc_feature (7)..(7): Xaa can be any amino acid
XAKRXEX

SEQ ID NO: 660 - protein, 7 aa, Artificial Sequence
  epitope
IEKNAKR

SEQ ID NO: 661 - protein, 7 aa, Artificial Sequence
  epitope
  misc_feature (1)..(1): Xaa can be any amino acid
  misc_feature (3)..(3): Xaa can be any amino acid
  misc_feature (7)..(7): Xaa can be any amino acid
XEXNAKX

SEQ ID NO: 662 - protein, 4 aa, Artificial Sequence
  epitope
NAKR

SEQ ID NO: 663 - protein, 4 aa, Artificial Sequence
  epitope
KNAK

SEQ ID NO: 664 - protein, 7 aa, Artificial Sequence
  epitope
SLHEIEK

SEQ ID NO: 665 - protein, 7 aa, Artificial Sequence
  epitope
  misc_feature (1)..(1): Xaa can be any amino acid
  misc_feature (3)..(3): Xaa can be any amino acid
  misc_feature (5)..(5): Xaa can be any amino acid
XLXEXEK

SEQ ID NO: 666 - protein, 6 aa, Artificial Sequence
  epitope
EIEKNA

SEQ ID NO: 667 - protein, 6 aa, Artificial Sequence
  epitope
  misc_feature (2)..(2): Xaa can be any amino acid
  misc_feature (6)..(6): Xaa can be any amino acid
EXEKNX

SEQ ID NO: 668 - protein, 5 aa, Artificial Sequence
  epitope
SLHEI

SEQ ID NO: 669 - protein, 10 aa, Artificial Sequence
  epitope
IEKNAKRFEI

SEQ ID NO: 670 - protein, 10 aa, Artificial Sequence
  epitope
  misc_feature (1)..(1): Xaa can be any amino acid
  misc_feature (4)..(5): Xaa can be any amino acid
  misc_feature (7)..(8): Xaa can be any amino acid
  misc_feature (10)..(10): Xaa can be any amino acid
XEKXXKXXEX

SEQ ID NO: 671 - protein, 15 aa, Artificial Sequence
  epitope
LPEALERWPTSMLEH

SEQ ID NO: 672 - protein, 15 aa, Artificial Sequence
  epitope
EWVVHLDQLTKLKPL

SEQ ID NO: 673 - protein, 8 aa, Artificial Sequence
  epitope
DQLTKLKP

SEQ ID NO: 674 - protein, 8 aa, Artificial Sequence
  epitope
  misc_feature (1)..(3): Xaa can be any amino acid
  misc_feature (8)..(8): Xaa can be any amino acid
XXXTKLKX

SEQ ID NO: 675 - protein, 8 aa, Artificial Sequence
  epitope
  misc_feature (2)..(4): Xaa can be any amino acid
DXXXKLKP

SEQ ID NO: 676 - protein, 5 aa, Artificial Sequence
  epitope
WVVHL

SEQ ID NO: 677 - protein, 5 aa, Artificial Sequence
  epitope
  misc_feature (5)..(5): Xaa can be any amino acid
WVVHX

SEQ ID NO: 678 - protein, 15 aa, Artificial Sequence
  epitope
ERGIDVLGDVIESSL

SEQ ID NO: 679 - protein, 4 aa, Artificial Sequence
  epitope
IDVL

SEQ ID NO: 680 - protein, 5 aa, Artificial Sequence
  epitope
VIESS

SEQ ID NO: 681 - protein, 15 aa, Artificial Sequence
  epitope
LIPKGNEQGLEFDLV

SEQ ID NO: 682 - protein, 4 aa, Artificial Sequence
  epitope
KGNE

SEQ ID NO: 683 - protein, 5 aa, Artificial Sequence
  epitope
KGNEQ

SEQ ID NO: 684 - protein, 6 aa, Artificial Sequence
  epitope
NEQGLE

SEQ ID NO: 685 - protein, 6 aa, Artificial Sequence
  epitope
  misc_feature (2)..(2): Xaa can be any amino acid
  misc_feature (5)..(5): Xaa can be any amino acid
NXQGXE

SEQ ID NO: 686 - protein, 15 aa, Artificial Sequence
  epitope
NVRKAAQKYSDKIGH

SEQ ID NO: 687 - protein, 7 aa, Artificial Sequence
  epitope
YSDKIGH

SEQ ID NO: 688 - protein, 7 aa, Artificial Sequence
  epitope
  misc_feature (1)..(1): Xaa can be any amino acid
  misc_feature (2)..(2): Xaa can be any amino acid
  misc_feature (4)..(4): Xaa can be any amino acid
XXDXIGH

SEQ ID NO: 689 - protein, 10 aa, Artificial Sequence
  epitope
VRKAAQKYSD

SEQ ID NO: 690 - protein, 10 aa, Artificial Sequence
  epitope
  misc_feature (3)..(6): Xaa can be any amino acid
  misc_feature (9)..(9): Xaa can be any amino acid
VRXXXXKYXD

SEQ ID NO: 691 - protein, 15 aa, Artificial Sequence
  epitope
PGNRIFVDDGLISLI

SEQ ID NO: 692 - protein, 7 aa, Artificial Sequence
  epitope
VDDGLIS

SEQ ID NO: 693 - protein, 7 aa, Artificial Sequence
  epitope
  misc_feature (1)..(1): Xaa can be any amino acid
  misc_feature (4)..(4): Xaa can be any amino acid
  misc_feature (6)..(6): Xaa can be any amino acid
XDDXLXS

SEQ ID NO: 694 - protein, 4 aa, Artificial Sequence
  epitope
IFVD

SEQ ID NO: 695 - protein, 7 aa, Artificial Sequence
  epitope
VDDGLIS

SEQ ID NO: 696 - protein, 7 aa, Artificial Sequence
  epitope
  misc_feature (1)..(1): Xaa can be any amino acid
  misc_feature (4)..(4): Xaa can be any amino acid
  misc_feature (6)..(6): Xaa can be any amino acid
XDDXLXS

SEQ ID NO: 697 - protein, 15 aa, Artificial Sequence
  epitope
NKLAMQEFMILPTGA

SEQ ID NO: 698 - protein, 5 aa, Artificial Sequence
  epitope
KLAMQ

SEQ ID NO: 699 - protein, 4 aa, Artificial Sequence
  epitope
LAMQ

SEQ ID NO: 700 - protein, 6 aa, Artificial Sequence
  epitope
NKLAMQ

SEQ ID NO: 701 - protein, 6 aa, Artificial Sequence
  epitope
  misc_feature (1)..(1): Xaa can be any amino acid
  misc_feature (3)..(3): Xaa can be any amino acid
  misc_feature (5)..(5): Xaa can be any amino acid
XKXAXQ

SEQ ID NO: 702 - protein, 8 aa, Artificial Sequence
  epitope
EFMILPTG

SEQ ID NO: 703 - protein, 10 aa, Artificial Sequence
  epitope
MQEFMILPTG

SEQ ID NO: 704 - protein, 15 aa, Artificial Sequence
  epitope
VLSIGDGIARVYGLK

SEQ ID NO: 705 - protein, 15 aa, Artificial Sequence
  epitope
PESDAKLKQIVTDFL

SEQ ID NO: 706 - protein, 5 aa, Artificial Sequence
  epitope
AKLKQ

SEQ ID NO: 707 - protein, 4 aa, Artificial Sequence
  epitope
IVTD

SEQ ID NO: 708 - protein, 15 aa, Artificial Sequence
  epitope
MADEEAKKKQEEIDR

SEQ ID NO: 709 - protein, 10 aa, Artificial Sequence
  epitope
AKKKQEEIDR

SEQ ID NO: 710 - protein, 10 aa, Artificial Sequence
  epitope
  misc_feature (2)..(5): Xaa can be any amino acid
  misc_feature (8)..(8): Xaa can be any amino acid
  misc_feature (10)..(10): Xaa can be any amino acid
AXXXXEEXDX

SEQ ID NO: 711 - protein, 7 aa, Artificial Sequence
  epitope
DEEAKKK

SEQ ID NO: 712 - protein, 7 aa, Artificial Sequence
  epitope
  misc_feature (2)..(3): Xaa can be any amino acid
  misc_feature (5)..(5): Xaa can be any amino acid
DXXAXKK

SEQ ID NO: 713 - protein, 6 aa, Artificial Sequence
  epitope
MADEEA

SEQ ID NO: 714 - protein, 6 aa, Artificial Sequence
  epitope
  misc_feature (1)..(2): Xaa can be any amino acid
XXDEEA

SEQ ID NO: 715 - protein, 10 aa, Artificial Sequence
  epitope
DEEAKKKQEE

SEQ ID NO: 716 - protein, 10 aa, Artificial Sequence
  epitope
  misc_feature (5)..(8): Xaa can be any amino acid
  misc_feature (10)..(10): Xaa can be any amino acid
DEEAXXXXEX

SEQ ID NO: 717 - protein, 15 aa, Artificial Sequence
  epitope
VMELRADVVPKTAEN

SEQ ID NO: 718 - protein, 4 aa, Artificial Sequence
  epitope
VPKT

SEQ ID NO: 719 - protein, 6 aa, Artificial Sequence
  epitope
VMELRA

SEQ ID NO: 720 - protein, 6 aa, Artificial Sequence
  epitope
  misc_feature (2)..(2): Xaa can be any amino acid
  misc_feature (6)..(6): Xaa can be any amino acid
VXELRX

SEQ ID NO: 721 - protein, 10 aa, Artificial Sequence
  epitope
ELRADVVPKT

SEQ ID NO: 722 - protein, 10 aa, Artificial Sequence
  epitope
  misc_feature (2)..(3): Xaa can be any amino acid
  misc_feature (6)..(8): Xaa can be any amino acid
  misc_feature (10)..(10): Xaa can be any amino acid
EXXADXXXKX

SEQ ID NO: 723 - protein, 5 aa, Artificial Sequence
  epitope
ELRAD

SEQ ID NO: 724 - protein, 6 aa, Artificial Sequence
  epitope
VPKTAE

SEQ ID NO: 725 - protein, 15 aa, Artificial Sequence
  epitope
SCFHRVIPNFMCQGG

SEQ ID NO: 726 - protein, 4 aa, Artificial Sequence
  epitope
IPNF

SEQ ID NO: 727 - protein, 4 aa, Artificial Sequence
  epitope
HRVI

SEQ ID NO: 728 - protein, 6 aa, Artificial Sequence
  epitope
FMCQGG

SEQ ID NO: 729 - protein, 15 aa, Artificial Sequence
  epitope
LFDPIIEDYHVGFKQ

SEQ ID NO: 730 - protein, 9 aa, Artificial Sequence
  epitope
DPIIEDYHV

SEQ ID NO: 731 - protein, 9 aa, Artificial Sequence
  epitope
  misc_feature (2)..(5): Xaa can be any amino acid
  misc_feature (7)..(7): Xaa can be any amino acid
DXXXXDXHV

SEQ ID NO: 732 - protein, 6 aa, Artificial Sequence
  epitope
HVGFKQ

SEQ ID NO: 733 - protein, 6 aa, Artificial Sequence
  epitope
  misc_feature (2)..(3): Xaa can be any amino acid
HXXFKQ

SEQ ID NO: 734 - protein, 9 aa, Artificial Sequence
  epitope
DPIIEDYHV

SEQ ID NO: 735 - protein, 9 aa, Artificial Sequence
  epitope
  misc_feature (4)..(5): Xaa can be any amino acid
  misc_feature (7)..(7): Xaa can be any amino acid
  misc_feature (9)..(9): Xaa can be any amino acid
DPIXXDXHX

SEQ ID NO: 736 - protein, 5 aa, Artificial Sequence
  epitope
EDYHV

SEQ ID NO: 737 - protein, 5 aa, Artificial Sequence
  epitope
  misc_feature (3)..(3): Xaa can be any amino acid
  misc_feature (5)..(5): Xaa can be any amino acid
EDXHX

SEQ ID NO: 738 - protein, 10 aa, Artificial Sequence
  epitope
FDPIIEDYHV

SEQ ID NO: 739 - protein, 10 aa, Artificial Sequence
  epitope
  misc_feature (5)..(5): Xaa can be any amino acid
  misc_feature (7)..(8): Xaa can be any amino acid
  misc_feature (10)..(10): Xaa can be any amino acid
FDPIXEXXHX

SEQ ID NO: 740 - protein, 9 aa, Artificial Sequence
  epitope
  misc_feature (3)..(7): Xaa can be any amino acid
  misc_feature (9)..(9): Xaa can be any amino acid
DPXXXXXHX

SEQ ID NO: 741 - protein, 15 aa, Artificial Sequence
  epitope
VNVDPEGKFVISTRV

SEQ ID NO: 742 - protein, 8 aa, Artificial Sequence
  epitope
EGKFVIST

SEQ ID NO: 743 - protein, 8 aa, Artificial Sequence
  epitope
  misc_feature (4)..(6): Xaa can be any amino acid
  misc_feature (8)..(8): Xaa can be any amino acid
EGKXXXSX

SEQ ID NO: 744 - protein, 10 aa, Artificial Sequence
  epitope
VDPEGKFVIS

SEQ ID NO: 745 - protein, 10 aa, Artificial Sequence
  epitope
  misc_feature (1)..(1): Xaa can be any amino acid
  misc_feature (3)..(4): Xaa can be any amino acid
  misc_feature (7)..(9): Xaa can be any amino acid
XDXXGKXXXS

SEQ ID NO: 746 - protein, 6 aa, Artificial Sequence
  epitope
VNVDPE

SEQ ID NO: 747 - protein, 6 aa, Artificial Sequence
  epitope
  misc_feature (3)..(3): Xaa can be any amino acid
VNXDPE

SEQ ID NO: 748 - protein, 9 aa, Artificial Sequence
  epitope
DPEGKFVIS

SEQ ID NO: 749 - protein, 9 aa, Artificial Sequence
  epitope
  misc_feature (5)..(5): Xaa can be any amino acid
  misc_feature (7)..(8): Xaa can be any amino acid
DPEGXFXXS

SEQ ID NO: 750 - protein, 15 aa, Artificial Sequence
  epitope
PDPDPTEYLFISREQ

SEQ ID NO: 751 - protein, 4 aa, Artificial Sequence
  epitope
PTEY

SEQ ID NO: 752 - protein, 15 aa, Artificial Sequence
  epitope
KLVTVKLPSGETKDF

SEQ ID NO: 753 - protein, 5 aa, Artificial Sequence
  epitope
GETKD

SEQ ID NO: 754 - protein, 5 aa, Artificial Sequence
  epitope
  misc_feature (1)..(1): Xaa can be any amino acid
XETKD

SEQ ID NO: 755 - protein, 6 aa, Artificial Sequence
  epitope
KLVTVK

SEQ ID NO: 756 - protein, 6 aa, Artificial Sequence
  epitope
  misc_feature (3)..(4): Xaa can be any amino acid
KLXXVK

SEQ ID NO: 757 - protein, 9 aa, Artificial Sequence
  epitope
KLPSGETKD

SEQ ID NO: 758 - protein, 9 aa, Artificial Sequence
  epitope
  misc_feature (2)..(6): Xaa can be any amino acid
KXXXXXTKD

SEQ ID NO: 759 - protein, 10 aa, Artificial Sequence
  epitope
VTVKLPSGET

SEQ ID NO: 760 - protein, 10 aa, Artificial Sequence
  epitope
  misc_feature (1)..(3): Xaa can be any amino acid
  misc_feature (5)..(6): Xaa can be any amino acid
  misc_feature (8)..(8): Xaa can be any amino acid
XXXKXXSXET

SEQ ID NO: 761 - protein, 10 aa, Artificial Sequence
  epitope
VKLPSGETKD

SEQ ID NO: 762 - protein, 10 aa, Artificial Sequence
  epitope
  misc_feature (1)..(1): Xaa can be any amino acid
  misc_feature (3)..(4): Xaa can be any amino acid
  misc_feature (6)..(6): Xaa can be any amino acid
XKXXSXETKD

SEQ ID NO: 763 - protein, 4 aa, Artificial Sequence
  epitope
GETK

SEQ ID NO: 764 - protein, 5 aa, Artificial Sequence
  epitope
GETKD

SEQ ID NO: 765 - protein, 15 aa, Artificial Sequence
  epitope
RGYHIFYQLMCDQID

SEQ ID NO: 766 - protein, 5 aa, Artificial Sequence
  epitope
YHIFY

SEQ ID NO: 767 - protein, 4 aa, Artificial Sequence
  epitope
MCDQ

SEQ ID NO: 768 - protein, 6 aa, Artificial Sequence
  epitope
RGYHIF

SEQ ID NO: 769 - protein, 6 aa, Artificial Sequence
  epitope
  misc_feature (3)..(3): Xaa can be any amino acid
  misc_feature (5)..(6): Xaa can be any amino acid
RGXHXX

SEQ ID NO: 770 - protein, 15 aa, Artificial Sequence
  epitope
QRYNILAAKEMLEAK

SEQ ID NO: 771 - protein, 5 aa, Artificial Sequence
  epitope
EMLEA

SEQ ID NO: 772 - protein, 10 aa, Artificial Sequence
  epitope
QRYNILAAKE

SEQ ID NO: 773 - protein, 10 aa, Artificial Sequence
  epitope
  misc_feature (1)..(2): Xaa can be any amino acid
  misc_feature (6)..(9): Xaa can be any amino acid
XXYNIXXXXE

SEQ ID NO: 774 - protein, 10 aa, Artificial Sequence
  epitope
YNILAAKEML

SEQ ID NO: 775 - protein, 10 aa, Artificial Sequence
  epitope
  misc_feature (4)..(7): Xaa can be any amino acid
  misc_feature (9)..(10): Xaa can be any amino acid
YNIXXXXEXX

SEQ ID NO: 776 - protein, 8 aa, Artificial Sequence
  epitope
YNILAAKE

SEQ ID NO: 777 - protein, 8 aa, Artificial Sequence
  epitope
  misc_feature (3)..(4): Xaa can be any amino acid
  misc_feature (6)..(6): Xaa can be any amino acid
  misc_feature (8)..(8): Xaa can be any amino acid
YNXXAXKX

SEQ ID NO: 778 - protein, 15 aa, Artificial Sequence
  epitope
MLEAKDDKKAATACF

SEQ ID NO: 779 - protein, 6 aa, Artificial Sequence
  epitope
EAKDDK

SEQ ID NO: 780 - protein, 6 aa, Artificial Sequence
  epitope
  misc_feature (6)..(6): Xaa can be any amino acid
EAKDDX

SEQ ID NO: 781 - protein, 9 aa, Artificial Sequence
  epitope
LEAKDDKKA

SEQ ID NO: 782 - protein, 9 aa, Artificial Sequence
  epitope
  misc_feature (1)..(3): Xaa can be any amino acid
  misc_feature (6)..(6): Xaa can be any amino acid
  misc_feature (9)..(9): Xaa can be any amino acid
XXXKDXKKX

SEQ ID NO: 783 - protein, 10 aa, Artificial Sequence
  epitope
MLEAKDDKKA

SEQ ID NO: 784 - protein, 10 aa, Artificial Sequence
  epitope
  misc_feature (3)..(4): Xaa can be any amino acid
  misc_feature (6)..(8): Xaa can be any amino acid
MLXXKXXXKA

SEQ ID NO: 785 - protein, 10 aa, Artificial Sequence
  epitope
KDDKKAATAC

SEQ ID NO: 786 - protein, 10 aa, Artificial Sequence
  epitope
  misc_feature (2)..(5): Xaa can be any amino acid
  misc_feature (10)..(10): Xaa can be any amino acid
KXXXXAATAX

SEQ ID NO: 787 - protein, 5 aa, Artificial Sequence
  epitope
AKDDK

SEQ ID NO: 788 - protein, 15 aa, Artificial Sequence
  epitope
ESRGRATLLGKFRNL

SEQ ID NO: 789 - protein, 9 aa, Artificial Sequence
  epitope
TLLGKFRNL

SEQ ID NO: 790 - protein, 9 aa, Artificial Sequence
  epitope
  misc_feature (1)..(3): Xaa can be any amino acid
  misc_feature (5)..(5): Xaa can be any amino acid
  misc_feature (7)..(7): Xaa can be any amino acid
XXXGXFXNL

SEQ ID NO: 791 - protein, 8 aa, Artificial Sequence
  epitope
GRATLLGK

SEQ ID NO: 792 - protein, 8 aa, Artificial Sequence
  epitope
  misc_feature (1)..(1): Xaa can be any amino acid
  misc_feature (4)..(4): Xaa can be any amino acid
  misc_feature (7)..(8): Xaa can be any amino acid
XRAXLLXX

SEQ ID NO: 793 - protein, 15 aa, Artificial Sequence
  epitope
INELEIALDHANKAN

SEQ ID NO: 794 - protein, 4 aa, Artificial Sequence
  epitope
HANK

SEQ ID NO: 795 - protein, 8 aa, Artificial Sequence
  epitope
IALDHANK

SEQ ID NO: 796 - protein, 8 aa, Artificial Sequence
  epitope
  misc_feature (1)..(1): Xaa can be any amino acid
  misc_feature (5)..(5): Xaa can be any amino acid
  misc_feature (7)..(7): Xaa can be any amino acid
XALDXAXK

SEQ ID NO: 797 - protein, 9 aa, Artificial Sequence
  epitope
EIALDHANK

SEQ ID NO: 798 - protein, 9 aa, Artificial Sequence
  epitope
  misc_feature (4)..(6): Xaa can be any amino acid
EIAXXXANK

SEQ ID NO: 799 - protein, 9 aa, Artificial Sequence
  epitope
NELEIALDH

SEQ ID NO: 800 - protein, 9 aa, Artificial Sequence
  epitope
  misc_feature (2)..(5): Xaa can be any amino acid
  misc_feature (8)..(8): Xaa can be any amino acid
NXXXXALXH

SEQ ID NO: 801 - protein, 10 aa, Artificial Sequence
  epitope
LEIALDHANK

SEQ ID NO: 802 - protein, 10 aa, Artificial Sequence
  epitope
  misc_feature (1)..(3): Xaa can be any amino acid
  misc_feature (6)..(6): Xaa can be any amino acid
  misc_feature (10)..(10): Xaa can be any amino acid
XXXALXHANX

SEQ ID NO: 803 - protein, 10 aa, Artificial Sequence
  epitope
IALDHANKAN

SEQ ID NO: 804 - protein, 10 aa, Artificial Sequence
  epitope
  misc_feature (1)..(1): Xaa can be any amino acid
  misc_feature (4)..(4): Xaa can be any amino acid
  misc_feature (8)..(9): Xaa can be any amino acid
XALXHANXXN

SEQ ID NO: 805 - protein, 9 aa, Artificial Sequence
  epitope
ALDHANKAN

SEQ ID NO: 806 - protein, 9 aa, Artificial Sequence
  epitope
  misc_feature (2)..(4): Xaa can be any amino acid
  misc_feature (7)..(7): Xaa can be any amino acid
  misc_feature (9)..(9): Xaa can be any amino acid
AXXXANXAX

SEQ ID NO: 807 - protein, 9 aa, Artificial Sequence
  epitope
  misc_feature (1)..(1): Xaa can be any amino acid
  misc_feature (3)..(5): Xaa can be any amino acid
  misc_feature (8)..(8): Xaa can be any amino acid
XIXXXHAXK

SEQ ID NO: 808 - protein, 8 aa, Artificial Sequence
  epitope
LDHANKAN

SEQ ID NO: 809 - protein, 8 aa, Artificial Sequence
  epitope
  misc_feature (2)..(2): Xaa can be any amino acid
  misc_feature (4)..(4): Xaa can be any amino acid
  misc_feature (7)..(8): Xaa can be any amino acid
LXHXNKXX

SEQ ID NO: 810 - protein, 15 aa, Artificial Sequence
  epitope
TKPYDPKKSCWVPDD

SEQ ID NO: 811 - protein, 10 aa, Artificial Sequence
  epitope
KPYDPKKSCW

SEQ ID NO: 812 - protein, 10 aa, Artificial Sequence
  epitope
  misc_feature (1)..(1): Xaa can be any amino acid
  misc_feature (3)..(3): Xaa can be any amino acid
  misc_feature (5)..(6): Xaa can be any amino acid
  misc_feature (8)..(9): Xaa can be any amino acid
XPXDXXKXXW

SEQ ID NO: 813 - protein, 8 aa, Artificial Sequence
  epitope
KKSCWVPD

SEQ ID NO: 814 - protein, 8 aa, Artificial Sequence
  epitope
  misc_feature (1)..(2): Xaa can be any amino acid
  misc_feature (6)..(6): Xaa can be any amino acid
  misc_feature (8)..(8): Xaa can be any amino acid
XXSCWXPX

SEQ ID NO: 815 - protein, 10 aa, Artificial Sequence
  epitope
TKPYDPKKSC

SEQ ID NO: 816 - protein, 10 aa, Artificial Sequence
  epitope
  misc_feature (4)..(8): Xaa can be any amino acid
  misc_feature (10)..(10): Xaa can be any amino acid
TKPXXXXXSX

SEQ ID NO: 817 - protein, 15 aa, Artificial Sequence
  epitope
VQVNPPKYEKCEDVS

SEQ ID NO: 818 - protein, 8 aa, Artificial Sequence
  epitope
KYEKCEDV

SEQ ID NO: 819 - protein, 8 aa, Artificial Sequence
  epitope
  misc_feature (1)..(3): Xaa can be any amino acid
XXXKCEDV

SEQ ID NO: 820 - protein, 10 aa, Artificial Sequence
  epitope
VNPPKYEKCE

SEQ ID NO: 821 - protein, 10 aa, Artificial Sequence
  epitope
  misc_feature (2)..(3): Xaa can be any amino acid
  misc_feature (5)..(5): Xaa can be any amino acid
  misc_feature (7)..(7): Xaa can be any amino acid
  misc_feature (9)..(10): Xaa can be any amino acid
VXXPXYXKXX

SEQ ID NO: 822 - protein, 10 aa, Artificial Sequence
  epitope
VQVNPPKYEK

SEQ ID NO: 823 - protein, 10 aa, Artificial Sequence
  epitope
  misc_feature (2)..(2): Xaa can be any amino acid
  misc_feature (4)..(5): Xaa can be any amino acid
  misc_feature (8)..(9): Xaa can be any amino acid
VXVXXPKXXK

SEQ ID NO: 824 - protein, 10 aa, Artificial Sequence
  epitope
PPKYEKCEDV

SEQ ID NO: 825 - protein, 10 aa, Artificial Sequence
  epitope
  misc_feature (1)..(1): Xaa can be any amino acid
  misc_feature (5)..(5): Xaa can be any amino acid
  misc_feature (7)..(10): Xaa can be any amino acid
XPKYXKXXXX

SEQ ID NO: 826 - protein, 15 aa, Artificial Sequence
  epitope
ERGYHIFYQMMSDQV

SEQ ID NO: 827 - protein, 6 aa, Artificial Sequence
  epitope
QMMSDQ

SEQ ID NO: 828 - protein, 6 aa, Artificial Sequence
  epitope
  misc_feature (3)..(4): Xaa can be any amino acid
QMXXDQ

SEQ ID NO: 829 - protein, 10 aa, Artificial Sequence
  epitope
ERGYHIFYQM

SEQ ID NO: 830 - protein, 10 aa, Artificial Sequence
  epitope
  misc_feature (2)..(3): Xaa can be any amino acid
  misc_feature (5)..(5): Xaa can be any amino acid
  misc_feature (8)..(10): Xaa can be any amino acid
EXXYXIFXXX

SEQ ID NO: 831 - protein, 6 aa, Artificial Sequence
  epitope
QMMSDQ

SEQ ID NO: 832 - protein, 6 aa, Artificial Sequence
  epitope
  misc_feature (4)..(4): Xaa can be any amino acid
  misc_feature (6)..(6): Xaa can be any amino acid
QMMXDX

SEQ ID NO: 833 - protein, 15 aa, Artificial Sequence
  epitope
GNMKFKQRGREEQAE

SEQ ID NO: 834 - protein, 6 aa, Artificial Sequence
  epitope
GNMKFK

SEQ ID NO: 835 - protein, 6 aa, Artificial Sequence
  epitope
  misc_feature (1)..(2): Xaa can be any amino acid
XXMKFK

SEQ ID NO: 836 - protein, 10 aa, Artificial Sequence
  epitope
MKFKQRGREE

SEQ ID NO: 837 - protein, 10 aa, Artificial Sequence
  epitope
  misc_feature (1)..(1): Xaa can be any amino acid
  misc_feature (5)..(5): Xaa can be any amino acid
  misc_feature (7)..(7): Xaa can be any amino acid
  misc_feature (9)..(10): Xaa can be any amino acid
XKFKXRXRXX

SEQ ID NO: 838 - protein, 5 aa, Artificial Sequence
  epitope
REEQA

SEQ ID NO: 839 - protein, 10 aa, Artificial Sequence
  epitope
  misc_feature (1)..(3): Xaa can be any amino acid
  misc_feature (5)..(5): Xaa can be any amino acid
  misc_feature (7)..(7): Xaa can be any amino acid
  misc_feature (10)..(10): Xaa can be any amino acid
XXXKXRXREX

SEQ ID NO: 840 - protein, 10 aa, Artificial Sequence
  epitope
FKQRGREEQA

SEQ ID NO: 841 - protein, 10 aa, Artificial Sequence
  epitope
  misc_feature (1)..(1): Xaa can be any amino acid
  misc_feature (3)..(3): Xaa can be any amino acid
  misc_feature (5)..(5): Xaa can be any amino acid
  misc_feature (8)..(10): Xaa can be any amino acid
XKXRXREXXX

SEQ ID NO: 842 - protein, 10 aa, Artificial Sequence
  epitope
KQRGREEQAE

SEQ ID NO: 843 - protein, 10 aa, Artificial Sequence
  epitope
  misc_feature (1)..(2): Xaa can be any amino acid
  misc_feature (4)..(5): Xaa can be any amino acid
  misc_feature (8)..(9): Xaa can be any amino acid
XXRXXEEXXE

SEQ ID NO: 844 - protein, 10 aa, Artificial Sequence
  epitope
  misc_feature (1)..(1): Xaa can be any amino acid
  misc_feature (3)..(3): Xaa can be any amino acid
  misc_feature (5)..(8): Xaa can be any amino acid
XKXKXXXXEE

SEQ ID NO: 845 - protein, 9 aa, Artificial Sequence
  epitope
KQRGREEQA

SEQ ID NO: 846 - protein, 9 aa, Artificial Sequence
  epitope
  misc_feature (2)..(5): Xaa can be any amino acid
  misc_feature (9)..(9): Xaa can be any amino acid
KXXXXEEQX

SEQ ID NO: 847 - protein, 15 aa, Artificial Sequence
  epitope
IMHQLTCNGVLEGIR

SEQ ID NO: 848 - protein, 8 aa, Artificial Sequence
  epitope
NGVLEGIR

SEQ ID NO: 849 - protein, 8 aa, Artificial Sequence
  epitope
  misc_feature (3)..(4): Xaa can be any amino acid
  misc_feature (6)..(7): Xaa can be any amino acid
NGXXEXXR

SEQ ID NO: 850 - protein, 5 aa, Artificial Sequence
  epitope
VLEGI

SEQ ID NO: 851 - protein, 4 aa, Artificial Sequence
  epitope
VLEG

SEQ ID NO: 852 - protein, 9 aa, Artificial Sequence
  epitope
QLTCNGVLE

SEQ ID NO: 853 - protein, 9 aa, Artificial Sequence
  epitope
  misc_feature (2)..(4): Xaa can be any amino acid
  misc_feature (6)..(6): Xaa can be any amino acid
  misc_feature (8)..(8): Xaa can be any amino acid
QXXXNXVXE

SEQ ID NO: 854 - protein, 10 aa, Artificial Sequence
  epitope
TCNGVLEGIR

SEQ ID NO: 855 - protein, 10 aa, Artificial Sequence
  epitope
  misc_feature (1)..(2): Xaa can be any amino acid
  misc_feature (4)..(4): Xaa can be any amino acid
  misc_feature (6)..(8): Xaa can be any amino acid
XXNXVXXXIR

SEQ ID NO: 856 - protein, 4 aa, Artificial Sequence
  epitope
HQLT

SEQ ID NO: 857 - protein, 8 aa, Artificial Sequence
  epitope
  misc_feature (2)..(3): Xaa can be any amino acid
  misc_feature (6)..(7): Xaa can be any amino acid
NXXLEXXR

SEQ ID NO: 858 - protein, 15 aa, Artificial Sequence
  epitope
LDKELYRCGKTKVFF

SEQ ID NO: 859 - protein, 8 aa, Artificial Sequence
  epitope
YRCGKTKV

SEQ ID NO: 860 - protein, 8 aa, Artificial Sequence
  epitope
  misc_feature (1)..(3): Xaa can be any amino acid
  misc_feature (8)..(8): Xaa can be any amino acid
XXXGKTKX

SEQ ID NO: 861 - protein, 10 aa, Artificial Sequence
  epitope
YRCGKTKVFF

SEQ ID NO: 862 - protein, 10 aa, Artificial Sequence
  epitope
  misc_feature (1)..(4): Xaa can be any amino acid
  misc_feature (8)..(9): Xaa can be any amino acid
XXXXKTKXXF

SEQ ID NO: 863 - protein, 10 aa, Artificial Sequence
  epitope
YRCGKTKVFF

SEQ ID NO: 864 - protein, 10 aa, Artificial Sequence
  epitope
  misc_feature (1)..(1): Xaa can be any amino acid
  misc_feature (3)..(4): Xaa can be any amino acid
  misc_feature (8)..(9): Xaa can be any amino acid
XRXXKTKXXF

SEQ ID NO: 865 - protein, 15 aa, Artificial Sequence
  epitope
VQKTNQDKATKDHQI

SEQ ID NO: 866 - protein, 8 aa, Artificial Sequence
  epitope
VQKTNQDK

SEQ ID NO: 867 - protein, 8 aa, Artificial Sequence
  epitope
  misc_feature (2)..(2): Xaa can be any amino acid
  misc_feature (4)..(6): Xaa can be any amino acid
VXKXXXDK

SEQ ID NO: 868 - protein, 6 aa, Artificial Sequence
  epitope
DKATKD

SEQ ID NO: 869 - protein, 6 aa, Artificial Sequence
  epitope
  misc_feature (6)..(6): Xaa can be any amino acid
DKATKX

SEQ ID NO: 870 - protein, 8 aa, Artificial Sequence
  epitope
VQKTNQDK

SEQ ID NO: 871 - protein, 8 aa, Artificial Sequence
  epitope
  misc_feature (1)..(1): Xaa can be any amino acid
  misc_feature (4)..(6): Xaa can be any amino acid
XQKXXXDK

SEQ ID NO: 872 - protein, 10 aa, Artificial Sequence
  epitope
VQKTNQDKAT

SEQ ID NO: 873 - protein, 10 aa, Artificial Sequence
  epitope
  misc_feature (1)..(2): Xaa can be any amino acid
  misc_feature (5)..(6): Xaa can be any amino acid
  misc_feature (8)..(8): Xaa can be any amino acid
  misc_feature (10)..(10): Xaa can be any amino acid
XXKTXXDXAX

SEQ ID NO: 874 - protein, 6 aa, Artificial Sequence
  epitope
  misc_feature (5)..(6): Xaa can be any amino acid
DKATXX

SEQ ID NO: 875 - protein, 10 aa, Artificial Sequence
  epitope
VQKTNQDKAT

SEQ ID NO: 876 - protein, 10 aa, Artificial Sequence
  epitope
  misc_feature (1)..(2): Xaa can be any amino acid
  misc_feature (4)..(6): Xaa can be any amino acid
  misc_feature (9)..(10): Xaa can be any amino acid
XXKXXXDKXX

SEQ ID NO: 877 - protein, 9 aa, Artificial Sequence
  epitope
TNQDKATKD

SEQ ID NO: 878 - protein, 9 aa, Artificial Sequence
  epitope
  misc_feature (1)..(3): Xaa can be any amino acid
  misc_feature (6)..(7): Xaa can be any amino acid
  misc_feature (9)..(9): Xaa can be any amino acid
XXXDKXXKX

SEQ ID NO: 879 - protein, 15 aa, Artificial Sequence
  epitope
EISHQDEIINKVNKE

SEQ ID NO: 880 - protein, 4 aa, Artificial Sequence
  epitope
EIIN

SEQ ID NO: 881 - protein, 15 aa, Artificial Sequence
  epitope
MTQETVADIERQHKD

SEQ ID NO: 882 - protein, 7 aa, Artificial Sequence
  epitope
ADIERQH

SEQ ID NO: 883 - protein, 7 aa, Artificial Sequence
  epitope
  misc_feature (3)..(4): Xaa can be any amino acid
ADXXRQH

SEQ ID NO: 884 - protein, 4 aa, Artificial Sequence
  epitope
RQHK

SEQ ID NO: 885 - protein, 10 aa, Artificial Sequence
  epitope
QETVADIERQ

SEQ ID NO: 886 - protein, 10 aa, Artificial Sequence
  epitope
  misc_feature (2)..(2): Xaa can be any amino acid
  misc_feature (4)..(4): Xaa can be any amino acid
  misc_feature (7)..(10): Xaa can be any amino acid
QXTXADXXXX

SEQ ID NO: 887 - protein, 10 aa, Artificial Sequence
  epitope
TQETVADIER

SEQ ID NO: 888 - protein, 10 aa, Artificial Sequence
  epitope
  misc_feature (1)..(3): Xaa can be any amino acid
  misc_feature (5)..(5): Xaa can be any amino acid
  misc_feature (9)..(10): Xaa can be any amino acid
XXXTXADIXX

SEQ ID NO: 889 - protein, 9 aa, Artificial Sequence
  epitope
VADIERQHK

SEQ ID NO: 890 - protein, 9 aa, Artificial Sequence
  epitope
  misc_feature (1)..(1): Xaa can be any amino acid
  misc_feature (5)..(7): Xaa can be any amino acid
  misc_feature (9)..(9): Xaa can be any amino acid
XADIXXXHX

SEQ ID NO: 891 - protein, 5 aa, Artificial Sequence
  epitope
ERQHK

SEQ ID NO: 892 - protein, 15 aa, Artificial Sequence
  epitope
QLEDTKKMVDDESRE

SEQ ID NO: 893 - protein, 7 aa, Artificial Sequence
  epitope
LEDTKKM

SEQ ID NO: 894 - protein, 7 aa, Artificial Sequence
  epitope
  misc_feature (2)..(4): Xaa can be any amino acid
LXXXKKM

SEQ ID NO: 895 - protein, 10 aa, Artificial Sequence
  epitope
EDTKKMVDDE

SEQ ID NO: 896 - protein, 10 aa, Artificial Sequence
  epitope
  misc_feature (1)..(3): Xaa can be any amino acid
  misc_feature (7)..(8): Xaa can be any amino acid
XXXKKMXXDE

SEQ ID NO: 897 - protein, 9 aa, Artificial Sequence
  epitope
KMVDDESRE

SEQ ID NO: 898 - protein, 9 aa, Artificial Sequence
  epitope
  misc_feature (2)..(4): Xaa can be any amino acid
  misc_feature (6)..(6): Xaa can be any amino acid
  misc_feature (8)..(8): Xaa can be any amino acid
KXXXDXSXE

SEQ ID NO: 899 - protein, 5 aa, Artificial Sequence
  epitope
LEDTK

SEQ ID NO: 900 - protein, 10 aa, Artificial Sequence
  epitope
KKMVDDESRE

SEQ ID NO: 901 - protein, 10 aa, Artificial Sequence
  epitope
  misc_feature (3)..(7): Xaa can be any amino acid
  misc_feature (10)..(10): Xaa can be any amino acid
KKXXXXXSRX

SEQ ID NO: 902 - protein, 7 aa, Artificial Sequence
  epitope
TKKMVDD

SEQ ID NO: 903 - protein, 7 aa, Artificial Sequence
  epitope
  misc_feature (1)..(1): Xaa can be any amino acid
  misc_feature (5)..(5): Xaa can be any amino acid
  misc_feature (7)..(7): Xaa can be any amino acid
XKKMXDX

SEQ ID NO: 904 - protein, 9 aa, Artificial Sequence
  epitope
QLEDTKKMV

SEQ ID NO: 905 - protein, 9 aa, Artificial Sequence
  epitope
  misc_feature (1)..(5): Xaa can be any amino acid
XXXXXKKMV

SEQ ID NO: 906 - protein, 9 aa, Artificial Sequence
  epitope
KKMVDDESR

SEQ ID NO: 907 - protein, 9 aa, Artificial Sequence
  epitope
  misc_feature (3)..(3): Xaa can be any amino acid
  misc_feature (5)..(5): Xaa can be any amino acid
  misc_feature (7)..(9): Xaa can be any amino acid
KKXVXDXXX

SEQ ID NO: 908 - protein, 15 aa, Artificial Sequence
  epitope
EIDKRIQEKEEEFDA

SEQ ID NO: 909 - protein, 4 aa, Artificial Sequence
  epitope
RIQE

SEQ ID NO: 910 - protein, 5 aa, Artificial Sequence
  epitope
KRIQE

SEQ ID NO: 911 - protein, 5 aa, Artificial Sequence
  epitope
  misc_feature (4)..(4): Xaa can be any amino acid
KRIXE

SEQ ID NO: 912 - protein, 15 aa, Artificial Sequence
  epitope
VRIFAWPHLDNNGIK

SEQ ID NO: 913 - protein, 5 aa, Artificial Sequence
  epitope
DNNGI

SEQ ID NO: 914 - protein, 5 aa, Artificial Sequence
  epitope
HLDNN

SEQ ID NO: 915 - protein, 15 aa, Artificial Sequence
  epitope
WHKQLFTELSQQVHL

SEQ ID NO: 916 - protein, 5 aa, Artificial Sequence
  epitope
TELSQ

SEQ ID NO: 917 - protein, 15 aa, Artificial Sequence
  epitope
TGVHEALEMRDGDKS

SEQ ID NO: 918 - protein, 6 aa, Artificial Sequence
  epitope
RDGDKS

SEQ ID NO: 919 - protein, 6 aa, Artificial Sequence
  epitope
  misc_feature (3)..(3): Xaa can be any amino acid
  misc_feature (6)..(6): Xaa can be any amino acid
RDXDKX

SEQ ID NO: 920 - protein, 5 aa, Artificial Sequence
  epitope
RDGDK

SEQ ID NO: 921 - protein, 8 aa, Artificial Sequence
  epitope
VHEALEMR

SEQ ID NO: 922 - protein, 8 aa, Artificial Sequence
  epitope
  misc_feature (2)..(2): Xaa can be any amino acid
  misc_feature (5)..(5): Xaa can be any amino acid
  misc_feature (7)..(7): Xaa can be any amino acid
VXEAXEXR

SEQ ID NO: 923 - protein, 7 aa, Artificial Sequence
  epitope
VHEALEM

SEQ ID NO: 924 - protein, 7 aa, Artificial Sequence
  epitope
  misc_feature (2)..(2): Xaa can be any amino acid
  misc_feature (6)..(7): Xaa can be any amino acid
VXEALXX

SEQ ID NO: 925 - protein, 5 aa, Artificial Sequence
  epitope
  misc_feature (1)..(1): Xaa can be any amino acid
XDGDK

SEQ ID NO: 926 - protein, 6 aa, Artificial Sequence
  epitope
RDGDKS

SEQ ID NO: 927 - protein, 6 aa, Artificial Sequence
  epitope
  misc_feature (6)..(6): Xaa can be any amino acid
RDGDKX

SEQ ID NO: 928 - protein, 15 aa, Artificial Sequence
  epitope
HLKAVIKGRFGLDAT

SEQ ID NO: 929 - protein, 6 aa, Artificial Sequence
  epitope
KGRFGL

SEQ ID NO: 930 - protein, 6 aa, Artificial Sequence
  epitope
  misc_feature (4)..(4): Xaa can be any amino acid
  misc_feature (6)..(6): Xaa can be any amino acid
KGRXGX

SEQ ID NO: 931 - protein, 8 aa, Artificial Sequence
  epitope
IKGRFGLD

SEQ ID NO: 932 - protein, 8 aa, Artificial Sequence
  epitope
  misc_feature (1)..(2): Xaa can be any amino acid
  misc_feature (5)..(5): Xaa can be any amino acid
  misc_feature (7)..(7): Xaa can be any amino acid
XXGRXGXD

SEQ ID NO: 933 - protein, 8 aa, Artificial Sequence
  epitope
KGRFGLDA

SEQ ID NO: 934 - protein, 8 aa, Artificial Sequence
  epitope
  misc_feature (2)..(2): Xaa can be any amino acid
  misc_feature (4)..(4): Xaa can be any amino acid
  misc_feature (6)..(6): Xaa can be any amino acid
  misc_feature (8)..(8): Xaa can be any amino acid
KXRXGXDX

SEQ ID NO: 935 - protein, 15 aa, Artificial Sequence
  epitope
EEIDRKKAEVRKRLE

SEQ ID NO: 936 - protein, 4 aa, Artificial Sequence
  epitope
EVRK

SEQ ID NO: 937 - protein, 6 aa, Artificial Sequence
  epitope
EEIDRK

SEQ ID NO: 938 - protein, 6 aa, Artificial Sequence
  epitope
  misc_feature (5)..(6): Xaa can be any amino acid
EEIDXX

SEQ ID NO: 939 - protein, 15 aa, Artificial Sequence
  epitope
RKKKLRLLLRKKAAE

SEQ ID NO: 940 - protein, 9 aa, Artificial Sequence
  epitope
KKLRLLLRK

SEQ ID NO: 941 - protein, 9 aa, Artificial Sequence
  epitope
  misc_feature (1)..(1): Xaa can be any amino acid
  misc_feature (4)..(5): Xaa can be any amino acid
  misc_feature (8)..(9): Xaa can be any amino acid
XKLXXLLXX

SEQ ID NO: 942 - protein, 6 aa, Artificial Sequence
  epitope
RKKAAE

SEQ ID NO: 943 - protein, 15 aa, Artificial Sequence
  epitope
AADNQPVGRIVMELR

SEQ ID NO: 944 - protein, 9 aa, Artificial Sequence
  epitope
DNQPVGRIV

SEQ ID NO: 945 - protein, 9 aa, Artificial Sequence
  epitope
  misc_feature (1)..(1): Xaa can be any amino acid
  misc_feature (6)..(6): Xaa can be any amino acid
  misc_feature (8)..(9): Xaa can be any amino acid
XNQPVXRXX

SEQ ID NO: 946 - protein, 5 aa, Artificial Sequence
  epitope
IVMEL

SEQ ID NO: 947 - protein, 9 aa, Artificial Sequence
  epitope
AADNQPVGR

SEQ ID NO: 948 - protein, 9 aa, Artificial Sequence
  epitope
  misc_feature (1)..(5): Xaa can be any amino acid
XXXXXPVGR

SEQ ID NO: 949 - protein, 10 aa, Artificial Sequence
  epitope
RCFQEWAERY

SEQ ID NO: 950 - protein, 10 aa, Artificial Sequence
  epitope
LANYLKGINA

SEQ ID NO: 951 - protein, 10 aa, Artificial Sequence
  epitope
ELEPIRTDYS

SEQ ID NO: 952 - protein, 7 aa, Artificial Sequence
  epitope
RDERLAK

SEQ ID NO: 953 - protein, 8 aa, Artificial Sequence
  epitope
KDHQIRNI

SEQ ID NO: 954 - protein, 6 aa, Artificial Sequence
  epitope
KDHQIR

SEQ ID NO: 955 - protein, 10 aa, Artificial Sequence
  epitope
AKSAMDSLAR

SEQ ID NO: 956 - protein, 7 aa, Artificial Sequence
  epitope
QKQVQEE

SEQ ID NO: 957 - protein, 10 aa, Artificial Sequence
  epitope
KVLIEELECL

SEQ ID NO: 958 - protein, 8 aa, Artificial Sequence
  epitope
DWFQKLKP

SEQ ID NO: 959 - protein, 7 aa, Artificial Sequence
  epitope
SMDIIGH

SEQ ID NO: 960 - protein, 10 aa, Artificial Sequence
  epitope
VREVNRKYFD

SEQ ID NO: 961 - protein, 7 aa, Artificial Sequence
  epitope
LDDALAS

SEQ ID NO: 962 - protein, 6 aa, Artificial Sequence
  epitope
VSDEEA

SEQ ID NO: 963 - protein, 10 aa, Artificial Sequence
  epitope
DEEASLDVEA

SEQ ID NO: 964 - protein, 6 aa, Artificial Sequence
  epitope
VCELRG

SEQ ID NO: 965 - protein, 9 aa, Artificial Sequence
  epitope
DPIIEDYHK

SEQ ID NO: 966 - protein, 10 aa, Artificial Sequence
  epitope
FDPIIEDYHK

SEQ ID NO: 967 - protein, 8 aa, Artificial Sequence
  epitope
EGKIEKSL

SEQ ID NO: 968 - protein, 10 aa, Artificial Sequence
  epitope
VDPDGKFVIS

SEQ ID NO: 969 - protein, 6 aa, Artificial Sequence
  epitope
KLIAVK

SEQ ID NO: 970 - protein, 9 aa, Artificial Sequence
  epitope
KGCRYFTKD

SEQ ID NO: 971 - protein, 10 aa, Artificial Sequence
  epitope
SGYNIVKRPE

SEQ ID NO: 972 - protein, 10 aa, Artificial Sequence
  epitope
YNIYNFVEYK

SEQ ID NO: 973 - protein, 9 aa, Artificial Sequence
  epitope
IFDKDGKKA

SEQ ID NO: 974 - protein, 8 aa, Artificial Sequence
  epitope
GRATLLGK

SEQ ID NO: 975 - protein, 9 aa, Artificial Sequence
  epitope
DISQDHAHK

SEQ ID NO: 976 - protein, 10 aa, Artificial Sequence
  epitope
NKQRYRESDM

SEQ ID NO: 977 - protein, 8 aa, Artificial Sequence
  epitope
NAALELLR

SEQ ID NO: 978 - protein, 8 aa, Artificial Sequence
  epitope
LQKFVFDK

SEQ ID NO: 979 - protein, 10 aa, Artificial Sequence
  epitope
QWTAADAVNS

SEQ ID NO: 980 - protein, 9 aa, Artificial Sequence
  epitope
PTKYNKKMV

SEQ ID NO: 981 - protein, 5 aa, Artificial Sequence
  epitope
KRIAE

SEQ ID NO: 982 - protein, 6 aa, Artificial Sequence
  epitope
RDKDKK

SEQ ID NO: 983 - protein, 7 aa, Artificial Sequence
  epitope
VYEALEL

SEQ ID NO: 984 - protein, 6 aa, Artificial Sequence
  epitope
  misc_feature (3)..(3): Xaa can be any amino acid
DKXTKD